European Patent Application EP 4 527 466 A2, published March 26, 2025. Title: ANTI-DLL3 CHIMERIC ANTIGEN RECEPTORS AND USES THEREOF. Applicant: Legend Biotech Ireland Limited. The sequence listing filed with the application follows.

SEQUENCE LISTING (529 sequences)

SEQ ID NO: 1 - protein, 10 aa, synthetic construct
  REGION 1..10: note = AS63930 CDR1
GYTYSGNYMA

SEQ ID NO: 2 - protein, 10 aa, synthetic construct
  REGION 1..10: note = AS63932 CDR1
GYTYGSTFMG

SEQ ID NO: 3 - protein, 10 aa, synthetic construct
  REGION 1..10: note = AS63951 CDR1
RDIYGNNCMA

SEQ ID NO: 4 - protein, 10 aa, synthetic construct
  REGION 1..10: note = AS63984 CDR1
GYTYSSNFMG

SEQ ID NO: 5 - protein, 7 aa, synthetic construct
  REGION 1..7: note = AS63987 CDR1
GYRNCMA

SEQ ID NO: 6 - protein, 10 aa, synthetic construct
  REGION 1..10: note = AS63997 CDR1
FSGYGVSTMA

SEQ ID NO: 7 - protein, 10 aa, synthetic construct
  REGION 1..10: note = AS64047 CDR1
QYVYRWDLMG

SEQ ID NO: 8 - protein, 10 aa, synthetic construct
  REGION 1..10: note = AS64052 CDR1
GYTYRSNFMG

SEQ ID NO: 9 - protein, 11 aa, synthetic construct
  REGION 1..11: note = AS64062 CDR1
RSPYSSSRCMG

SEQ ID NO: 10 - protein, 10 aa, synthetic construct
  REGION 1..10: note = AS64072 CDR1
GYSYYINLMA

SEQ ID NO: 11 - protein, 10 aa, synthetic construct
  REGION 1..10: note = AS64097 CDR1
GYTYSRNCMG

SEQ ID NO: 12 - protein, 10 aa, synthetic construct
  REGION 1..10: note = AS64114 CDR1
GNTYSTNYMG

SEQ ID NO: 13 - protein, 10 aa, synthetic construct
  REGION 1..10: note = AS64123 CDR1
GYTYTSNWLG

SEQ ID NO: 14 - protein, 10 aa, synthetic construct
  REGION 1..10: note = AS64130 CDR1
GYTYRSNFMG

SEQ ID NO: 15 - protein, 10 aa, synthetic construct
  REGION 1..10: note = AS64137 CDR1
GSTYSTNFMG

SEQ ID NO: 16 - protein, 10 aa, synthetic construct
  REGION 1..10: note = AS64142 CDR1
GFTFDRNAMR

SEQ ID NO: 17 - protein, 10 aa, synthetic construct
  REGION 1..10: note = AS64154 CDR1
GYTYRYLYMG

SEQ ID NO: 18 - protein, 10 aa, synthetic construct
  REGION 1..10: note = AS64160 CDR1
VYTSSSYCMG

SEQ ID NO: 19 - protein, 10 aa, synthetic construct
  REGION 1..10: note = AS64228 CDR1
GVSYNRCSMG

SEQ ID NO: 20 - protein, 10 aa, synthetic construct
  REGION 1..10: note = AS64300 CDR1
GDIYNLMSMA

SEQ ID NO: 21 - protein, 10 aa, synthetic construct
  REGION 1..10: note = AS64380 CDR1
GNTYSSNYMG

SEQ ID NO: 22 - protein, 10 aa, synthetic construct
  REGION 1..10: note = AS64395 CDR1
GSTYSTNFMG

SEQ ID NO: 23 - protein, 10 aa, synthetic construct
  REGION 1..10: note = AS64443 CDR1
GYTDSSVYIG

SEQ ID NO: 24 - protein, 10 aa, synthetic construct
  REGION 1..10: note = AS64511 CDR1
RATYSTNYIS

SEQ ID NO: 25 - protein, 10 aa, synthetic construct
  REGION 1..10: note = AS64536 CDR1
RYTDNFVYMG

SEQ ID NO: 26 - protein, 10 aa, synthetic construct
  REGION 1..10: note = AS64597 CDR1
GYTYRVNFMG

SEQ ID NO: 27 - protein, 9 aa, synthetic construct
  REGION 1..9: note = AS64617 CDR1
GYTDRCSMA

SEQ ID NO: 28 - protein, 12 aa, synthetic construct
  REGION 1..12: note = AS64634 CDR1
GYSFRGDFMCMG

SEQ ID NO: 29 - protein, 10 aa, synthetic construct
  REGION 1..10: note = AS69498 CDR1
GNTYSSNYMA

SEQ ID NO: 30 - protein, 10 aa, synthetic construct
  REGION 1..10: note = AS69500 CDR1
RYTYSSACMG

SEQ ID NO: 31 - protein, 10 aa, synthetic construct
  REGION 1..10: note = AS69527 CDR1
RYTFSSTCMA

SEQ ID NO: 32 - protein, 10 aa, synthetic construct
  REGION 1..10: note = AS68280 CDR1
GSTYSSNYLG

SEQ ID NO: 33 - protein, 10 aa, synthetic construct
  REGION 1..10: note = AS68355 CDR1
GYTYSGVCMG

SEQ ID NO: 34 - protein, 10 aa, synthetic construct
  REGION 1..10: note = AS69443 CDR1
GFTFDDSDMA

SEQ ID NO: 35 - protein, 10 aa, synthetic construct
  REGION 1..10: note = AS75376 CDR1
GYTYSSHSMG

SEQ ID NO: 36 - protein, 10 aa, synthetic construct
  REGION 1..10: note = AS75387 CDR1
GYPYSSPCMA

SEQ ID NO: 37 - protein, 10 aa, synthetic construct
  REGION 1..10: note = AS75695 CDR1
GYTVSAYCMG

SEQ ID NO: 38 - protein, 10 aa, synthetic construct
  REGION 1..10: note = AS76169 CDR1
GYIYSSFCMG

SEQ ID NO: 39 - protein, 10 aa, synthetic construct
  REGION 1..10: note = AS63931 CDR1
FSGYGVSTMA

SEQ ID NO: 40 - protein, 10 aa, synthetic construct
  REGION 1..10: note = AS63937 CDR1
GSTISSRPMA

SEQ ID NO: 41 - protein, 10 aa, synthetic construct
  REGION 1..10: note = AS63948 CDR1
GYTYRYLYMG

SEQ ID NO: 42 - protein, 10 aa, synthetic construct
  REGION 1..10: note = AS63956 CDR1
GFTYSNCCMR

SEQ ID NO: 43 - protein, 10 aa, synthetic construct
  REGION 1..10: note = AS63965 CDR1
GYSSGSCRMG

SEQ ID NO: 44 - protein, 10 aa, synthetic construct
  REGION 1..10: note = AS63993 CDR1
GFTFDDLVMA

SEQ ID NO: 45 - protein, 10 aa, synthetic construct
  REGION 1..10: note = AS63999 CDR1
GYTYSSNWMG

SEQ ID NO: 46 - protein, 10 aa, synthetic construct
  REGION 1..10: note = AS64006 CDR1
GYTGDTTYIG

SEQ ID NO: 47 - protein, 10 aa, synthetic construct
  REGION 1..10: note = AS64057 CDR1
GFTFDRNAMR

SEQ ID NO: 48 - protein, 10 aa, synthetic construct
  REGION 1..10: note = AS64060 CDR1
GSTYCTYRMS

SEQ ID NO: 49 - protein, 10 aa, synthetic construct
  REGION 1..10: note = AS64071 CDR1
GNTYRLNSMG

SEQ ID NO: 50 - protein, 10 aa, synthetic construct
  REGION 1..10: note = AS64093 CDR1
RYIYGNNCMA

SEQ ID NO: 51 - protein, 10 aa, synthetic construct
  REGION 1..10: note = AS64118 CDR1
GYTYSACRMA

SEQ ID NO: 52 - protein, 10 aa, synthetic construct
  REGION 1..10: note = AS64120 CDR1
RYIYGNNCMA

SEQ ID NO: 53 - protein, 10 aa, synthetic construct
  REGION 1..10: note = AS64124 CDR1
TYTPSNNYMG

SEQ ID NO: 54 - protein, 10 aa, synthetic construct
  REGION 1..10: note = AS64135 CDR1
TSTYCRYYMR

SEQ ID NO: 55 - protein, 10 aa, synthetic construct
  REGION 1..10: note = AS64163 CDR1
GYRYRWNCMA

SEQ ID NO: 56 - protein, 10 aa, synthetic construct
  REGION 1..10: note = AS64182 CDR1
GQTSRYLYMG

SEQ ID NO: 57 - protein, 10 aa, synthetic construct
  REGION 1..10: note = AS64183 CDR1
GHTYSANCMA

SEQ ID NO: 58 - protein, 10 aa, synthetic construct
  REGION 1..10: note = AS64207 CDR1
GYTYSSNFMG

SEQ ID NO: 59 - protein, 10 aa, synthetic construct
  REGION 1..10: note = AS64276 CDR1
GYTGSSRCMA

SEQ ID NO: 60 - protein, 10 aa, synthetic construct
  REGION 1..10: note = AS64336 CDR1
GRTYSSCSMG

SEQ ID NO: 61 - protein, 7 aa, synthetic construct
  REGION 1..7: note = AS64346 CDR1
GYTYFMG

SEQ ID NO: 62 - protein, 10 aa, synthetic construct
  REGION 1..10: note = AS64420 CDR1
GDTSRSVWMG

SEQ ID NO: 63 - protein, 10 aa, synthetic construct
  REGION 1..10: note = AS64473 CDR1
GYTYRYLYMA

SEQ ID NO: 64 - protein, 10 aa, synthetic construct
  REGION 1..10: note = AS64475 CDR1
GYTWSRNWMG

SEQ ID NO: 65 - protein, 10 aa, synthetic construct
  REGION 1..10: note = AS64513 CDR1
DYPYIDNCMG

SEQ ID NO: 66 - protein, 10 aa, synthetic construct
  REGION 1..10: note = AS64562 CDR1
GYTARRDFMA

SEQ ID NO: 67 - protein, 10 aa, synthetic construct
  REGION 1..10: note = AS64583 CDR1
GFTIAVYTMG

SEQ ID NO: 68 - protein, 10 aa, synthetic construct
  REGION 1..10: note = AS64594 CDR1
GYTYNSNYMG

SEQ ID NO: 69 - protein, 10 aa, synthetic construct
  REGION 1..10: note = AS64605 CDR1
RYPYSSICMG

SEQ ID NO: 70 - protein, 10 aa, synthetic construct
  REGION 1..10: note = AS64606 CDR1
GYTSRSNYMG

SEQ ID NO: 71 - protein, 10 aa, synthetic construct
  REGION 1..10: note = AS68121 CDR1
GYTYSRNCMG

SEQ ID NO: 72 - protein, 10 aa, synthetic construct
  REGION 1..10: note = AS68170 CDR1
GYTYRSNCMG

SEQ ID NO: 73 - protein, 10 aa, synthetic construct
  REGION 1..10: note = AS63964 CDR1
GYTYSYNNMG

SEQ ID NO: 74 - protein, 8 aa, synthetic construct
  REGION 1..8: note = AS64116 CDR1
GYIYSCVG

SEQ ID NO: 75 - protein, 13 aa, synthetic construct
  REGION 1..13: note = AS68270 CDR1
GYPSSTYYMLSMA

SEQ ID NO: 76 - protein, 10 aa, synthetic construct
  REGION 1..10: note = AS68320 CDR1
GYTYNTNYMG

SEQ ID NO: 77 - protein, 10 aa, synthetic construct
  REGION 1..10: note = AS68351 CDR1
GDTFRAYYMN

SEQ ID NO: 78 - protein, 10 aa, synthetic construct
  REGION 1..10: note = AS75378 CDR1
GNTRSTTYMG

SEQ ID NO: 79 - protein, 10 aa, synthetic construct
  REGION 1..10: note = AS75383 CDR1
GYTFSSYCLG

SEQ ID NO: 80 - protein, 11 aa, synthetic construct
  REGION 1..11: note = AS75751 CDR1
GYFYNTYYFMG

SEQ ID NO: 81 - protein, 10 aa, synthetic construct
  REGION 1..10: note = AS76422 CDR1
GYTFAGNCLG

SEQ ID NO: 82 - protein, 20 aa, synthetic construct
  REGION 1..20: note = AS63930 CDR2
VVYNIDGGGRFTTYADSVKG

SEQ ID NO: 83 - protein, 17 aa, synthetic construct
  REGION 1..17: note = AS63932 CDR2
VIYTGGGSTWYASSVKG

SEQ ID NO: 84 - protein, 17 aa, synthetic construct
  REGION 1..17: note = AS63951 CDR2
SIYPAGGRPYYADSVKG

SEQ ID NO: 85 - protein, 17 aa, synthetic construct
  REGION 1..17: note = AS63984 CDR2
TIVSGGGTTYYADSVRG

SEQ ID NO: 86 - protein, 17 aa, synthetic construct
  REGION 1..17: note = AS63987 CDR2
VIYTPSGITDYASSVKG

SEQ ID NO: 87 - protein, 17 aa, synthetic construct
  REGION 1..17: note = AS63997 CDR2
AITVGSGNTYYADSVKG

SEQ ID NO: 88 - protein, 17 aa, synthetic construct
  REGION 1..17: note = AS64047 CDR2
AVYTGDGITYYADSVKG

SEQ ID NO: 89 - protein, 17 aa, synthetic construct
  REGION 1..17: note = AS64052 CDR2
TIHSGVATTYYADSVKG

SEQ ID NO: 90 - protein, 17 aa, synthetic construct
  REGION 1..17: note = AS64062 CDR2
ALYTGGGSTSYADSVKG

SEQ ID NO: 91 - protein, 17 aa, synthetic construct
  REGION 1..17: note = AS64072 CDR2
AHGPVSGTAYYTDSVKG

SEQ ID NO: 92 - protein, 17 aa, synthetic construct
  REGION 1..17: note = AS64097 CDR2
AINTGGGSTYYADSLEG

SEQ ID NO: 93 - protein, 17 aa, synthetic construct
  REGION 1..17: note = AS64114 CDR2
VIYTRGGHTYYVDSVRG

SEQ ID NO: 94 - protein, 17 aa, synthetic construct
  REGION 1..17: note = AS64123 CDR2
IIYTGSGSTHYRSSVKG

SEQ ID NO: 95 - protein, 17 aa, synthetic construct
  REGION 1..17: note = AS64130 CDR2
TIDSRGTITYYADSVKG

SEQ ID NO: 96 - protein, 17 aa, synthetic construct
  REGION 1..17: note = AS64137 CDR2
TLVTWVERTAYADSVKG

SEQ ID NO: 97 - protein, 17 aa, synthetic construct
  REGION 1..17: note = AS64142 CDR2
CIDWTGANIAYADSVKG

SEQ ID NO: 98 - protein, 17 aa, synthetic construct
  REGION 1..17: note = AS64154 CDR2
CIYTGSGSTGYADSVKG

SEQ ID NO: 99 - protein, 17 aa, synthetic construct
  REGION 1..17: note = AS64160 CDR2
AMCFGGLVTHYADSVKG

SEQ ID NO: 100 - protein, 16 aa, synthetic construct
  REGION 1..16: note = AS64228 CDR2
RIQPGGNTYYADSVKG

SEQ ID NO: 101 - protein, 17 aa, synthetic construct
  REGION 1..17: note = AS64300 CDR2
YINTIIGNTYYTDSVKG

SEQ ID NO: 102 - protein, 17 aa, synthetic construct
  REGION 1..17: note = AS64380 CDR2
VIYTRGGHTYYVDSVRG

SEQ ID NO: 103 - protein, 17 aa, synthetic construct
  REGION 1..17: note = AS64395 CDR2
TLVTWAERTAYADSVKG

SEQ ID NO: 104 - protein, 17 aa, synthetic construct
  REGION 1..17: note = AS64443 CDR2
IIYTGGESTHYRSSVKG

SEQ ID NO: 105 - protein, 17 aa, synthetic construct
  REGION 1..17: note = AS64511 CDR2
TITTGDGETAYADSVKG

SEQ ID NO: 106 - protein, 17 aa, synthetic construct
  REGION 1..17: note = AS64536 CDR2
LIYPGGGSTYYASSVKG

SEQ ID NO: 107 - protein, 17 aa, synthetic construct
  REGION 1..17: note = AS64597 CDR2
TIDSGVGTTYYADSVKG

SEQ ID NO: 108 - protein, 16 aa, synthetic construct
  REGION 1..16: note = AS64617 CDR2
RISTSGFTNYAASVKG

SEQ ID NO: 109 - protein, 17 aa, synthetic construct
  REGION 1..17: note = AS64634 CDR2
VFYPGGGSTNYADSAKG

SEQ ID NO: 110 - protein, 17 aa, synthetic construct
  REGION 1..17: note = AS69498 CDR2
VIYTRGGHTYYIDSVRG

SEQ ID NO: 111 - protein, 18 aa, synthetic construct
  REGION 1..18: note = AS69500 CDR2
SIFTGTGGSTYYADSVKG

SEQ ID NO: 112 - protein, 17 aa, synthetic construct
  REGION 1..17: note = AS69527 CDR2
AIYTDDGSTWYADSVKG

SEQ ID NO: 113 - protein, 17 aa, synthetic construct
  REGION 1..17: note = AS68280 CDR2
AISTGDGATAYADSVKG

SEQ ID NO: 114 - protein, 16 aa, synthetic construct
  REGION 1..16: note = AS68355 CDR2
AIDSDGSTSYADSVKG

SEQ ID NO: 115 - protein, 16 aa, synthetic construct
  REGION 1..16: note = AS69443 CDR2
TISSDGSTYYADSVKG

SEQ ID NO: 116 - protein, 17 aa, synthetic construct
  REGION 1..17: note = AS75376 CDR2
VIYTGDGSTYYADSVKG

SEQ ID NO: 117 - protein, 17 aa, synthetic construct
  REGION 1..17: note = AS75387 CDR2
VAYTGGDIQYLTDSVKG

SEQ ID NO: 118 - protein, 16 aa, synthetic construct
  REGION 1..16: note = AS75695 CDR2
FIDAGGATIYADPVKG

SEQ ID NO: 119 - protein, 16 aa, synthetic construct
  REGION 1..16: note = AS76169 CDR2
YIRDNIMTSYTDSVKG

SEQ ID NO: 120 - protein, 17 aa, synthetic construct
  REGION 1..17: note = AS63931 CDR2
AITVGSGNTYYADSVTG

SEQ ID NO: 121 - protein, 17 aa, synthetic construct
  REGION 1..17: note = AS63937 CDR2
CIHTGLGRTYYADSVKG

SEQ ID NO: 122 - protein, 17 aa, synthetic construct
  REGION 1..17: note = AS63948 CDR2
CIYTGSGSTGYADSVKG

SEQ ID NO: 123 - protein, 16 aa, synthetic construct
  REGION 1..16: note = AS63956 CDR2
LINSSGGTYYADSVRG

SEQ ID NO: 124 - protein, 16 aa, synthetic construct
  REGION 1..16: note = AS63965 CDR2
KVISDGTTVYADSVKG

SEQ ID NO: 125 - protein, 16 aa, synthetic construct
  REGION 1..16: note = AS63993 CDR2
LVATAGNSVYADSVKG

SEQ ID NO: 126 - protein, 17 aa, synthetic construct
  REGION 1..17: note = AS63999 CDR2
IIYTGGISTHYRSSVKG

SEQ ID NO: 127 - protein, 17 aa, synthetic construct
  REGION 1..17: note = AS64006 CDR2
LIYTSGTSEYYADSVKG

SEQ ID NO: 128 - protein, 17 aa, synthetic construct
  REGION 1..17: note = AS64057 CDR2
CISWTGANIAYADSVKG

SEQ ID NO: 129 - protein, 16 aa, synthetic construct
  REGION 1..16: note = AS64060 CDR2
VIDSGGSTSYADSVKG

SEQ ID NO: 130 - protein, 17 aa, synthetic construct
  REGION 1..17: note = AS64071 CDR2
FIVMIRGTTYYGASVKG

SEQ ID NO: 131 - protein, 17 aa, synthetic construct
  REGION 1..17: note = AS64093 CDR2
SIYPAGGRTYYADSVKG

SEQ ID NO: 132 - protein, 16 aa, synthetic construct
  REGION 1..16: note = AS64118 CDR2
FINSAGSTYYADSVKG

SEQ ID NO: 133 - protein, 17 aa, synthetic construct
  REGION 1..17: note = AS64120 CDR2
SIYPAGGRPYYADSVKG

SEQ ID NO: 134 - protein, 17 aa, synthetic construct
  REGION 1..17: note = AS64124 CDR2
AIATIGGTTRYADSVKG

SEQ ID NO: 135 - protein, 16 aa, synthetic construct
  REGION 1..16: note = AS64135 CDR2
AMQPDGTTSYSDSVKG

SEQ ID NO: 136 - protein, 17 aa, synthetic construct
  REGION 1..17: note = AS64163 CDR2
AISTGSGSTYYAGSVKG

SEQ ID NO: 137 - protein, 17 aa, synthetic construct
  REGION 1..17: note = AS64182 CDR2
CIYTGSGSTGYADSVKG

SEQ ID NO: 138 - protein, 17 aa, synthetic construct
  REGION 1..17: note = AS64183 CDR2
SVYTDDDSTMYTDSVKG

SEQ ID NO: 139 - protein, 17 aa, synthetic construct
  REGION 1..17: note = AS64207 CDR2
TIVSGGGTTYYADSVRG

SEQ ID NO: 140 - protein, 17 aa, synthetic construct
  REGION 1..17: note = AS64276 CDR2
QIFTGRGTTGYADSVKG

SEQ ID NO: 141 - protein, 16 aa, synthetic construct
  REGION 1..16: note = AS64336 CDR2
HIFSDGSRYYADSVKG

SEQ ID NO: 142 - protein, 20 aa, synthetic construct
  REGION 1..20: note = AS64346 CDR2
TIGTGDIFNGAAYYVDSVKG

SEQ ID NO: 143 - protein, 17 aa, synthetic construct
  REGION 1..17: note = AS64420 CDR2
TISTAGGSTWYTDSVKG

SEQ ID NO: 144 - protein, 17 aa, synthetic construct
  REGION 1..17: note = AS64473 CDR2
CIYTGSGTTGYADSVKG

SEQ ID NO: 145 - protein, 17 aa, synthetic construct
  REGION 1..17: note = AS64475 CDR2
TITISGGSTWYADSVKG

SEQ ID NO: 146 - protein, 17 aa, synthetic construct
  REGION 1..17: note = AS64513 CDR2
AACTGGGSTYYADSVKG

SEQ ID NO: 147 - protein, 17 aa, synthetic construct
  REGION 1..17: note = AS64562 CDR2
VIHTGGDTTYYADSVKG

SEQ ID NO: 148 - protein, 17 aa, synthetic construct
  REGION 1..17: note = AS64583 CDR2
CTSWAGGRTYTADSVKG

SEQ ID NO: 149 - protein, 17 aa, synthetic construct
  REGION 1..17: note = AS64594 CDR2
LIYTGGGSTYYADSVKG

SEQ ID NO: 150 - protein, 17 aa, synthetic construct
  REGION 1..17: note = AS64605 CDR2
RIYTGTGSTWYTDSVKG

SEQ ID NO: 151 - protein, 20 aa, synthetic construct
  REGION 1..20: note = AS64606 CDR2
AFYLIYTRGGSTYYASSVKG

SEQ ID NO: 152 - protein, 17 aa, synthetic construct
  REGION 1..17: note = AS68121 CDR2
TDYIRFGRTYYADSVKG

SEQ ID NO: 153 - protein, 18 aa, synthetic construct
  REGION 1..18: note = AS68170 CDR2
TIYTGGGRNLYYADSVKG

SEQ ID NO: 154 - protein, 16 aa, synthetic construct
  REGION 1..16: note = AS63964 CDR2
AISGGRFTAYADSVKG

SEQ ID NO: 155 - protein, 17 aa, synthetic construct
  REGION 1..17: note = AS64116 CDR2
GISTGGGGTVYADSVKG

SEQ ID NO: 156 - protein, 17 aa, synthetic construct
  REGION 1..17: note = AS68270 CDR2
AITSGTGSTSYADSVKD

SEQ ID NO: 157 - protein, 17 aa, synthetic construct
  REGION 1..17: note = AS68320 CDR2
AIYRHSGNTAYADSVKG

SEQ ID NO: 158 - protein, 17 aa, synthetic construct
  REGION 1..17: note = AS68351 CDR2
GISASGGRTSYADSVKG

SEQ ID NO: 159 - protein, 17 aa, synthetic construct
  REGION 1..17: note = AS75378 CDR2
IVYTGGRDTYYAASVKG

SEQ ID NO: 160 - protein, 16 aa, synthetic construct
  REGION 1..16: note = AS75383 CDR2
TFNNRGVANYHDSVKG

SEQ ID NO: 161 - protein, 16 aa, synthetic construct
  REGION 1..16: note = AS75751 CDR2
AIDTDGRTSYADSVKG

SEQ ID NO: 162 - protein, 16 aa, synthetic construct
  REGION 1..16: note = AS76422 CDR2
TYNNFGVANYADSVKG

SEQ ID NO: 163 - protein, 17 aa, synthetic construct
  REGION 1..17: note = AS63930 CDR3
EVADPTWGSRDQRRYKY

SEQ ID NO: 164 - protein, 9 aa, synthetic construct
  REGION 1..9: note = AS63932 CDR3
RYGSGNVNY

SEQ ID NO: 165 - protein, 21 aa, synthetic construct
  REGION 1..21: note = AS63951 CDR3
RSFSIAVCATRSGITRSNFAY

SEQ ID NO: 166 - protein, 20 aa, synthetic construct
  REGION 1..20: note = AS63984 CDR3
GGPVTNAPRWYPLRPPGYNY

SEQ ID NO: 167 - protein, 16 aa, synthetic construct
  REGION 1..16: note = AS63987 CDR3
DRPFVCNIANMRRSSN

SEQ ID NO: 168 - protein, 16 aa, synthetic construct
  REGION 1..16: note = AS63997 CDR3
GYLSGGSWDVPGRYNY

SEQ ID NO: 169 - protein, 16 aa, synthetic construct
  REGION 1..16: note = AS64047 CDR3
GFVSGGRWNQSYRYKY

SEQ ID NO: 170 - protein, 20 aa, synthetic construct
  REGION 1..20: note = AS64052 CDR3
GGPPANADRWYPLRPPGYNY

SEQ ID NO: 171 - protein, 17 aa, synthetic construct
  REGION 1..17: note = AS64062 CDR3
VVPRGGSCRLDERGYYH

SEQ ID NO: 172 - protein, 14 aa, synthetic construct
  REGION 1..14: note = AS64072 CDR3
ETTMGWAHERGYRY

SEQ ID NO: 173 - protein, 18 aa, synthetic construct
  REGION 1..18: note = AS64097 CDR3
GPDLGGSWCRPVERAFTY

SEQ ID NO: 174 - protein, 16 aa, synthetic construct
  REGION 1..16: note = AS64114 CDR3
ASRHRLRLNNPRDYDY

SEQ ID NO: 175 - protein, 7 aa, synthetic construct
  REGION 1..7: note = AS64123 CDR3
RFSEYNY

SEQ ID NO: 176 - protein, 20 aa, synthetic construct
  REGION 1..20: note = AS64130 CDR3
GGPRTNDDRWYPLRPPGYNY

SEQ ID NO: 177 - protein, 17 aa, synthetic construct
  REGION 1..17: note = AS64137 CDR3
AAASTDVRLLDPGDFAY

SEQ ID NO: 178 - protein, 17 aa, synthetic construct
  REGION 1..17: note = AS64142 CDR3
DTTSGYCSGFWSTSRYS

SEQ ID NO: 179 - protein, 17 aa, synthetic construct
  REGION 1..17: note = AS64154 CDR3
SSPRWGGTCRRWSQYNY

SEQ ID NO: 180 - protein, 19 aa, synthetic construct
  REGION 1..19: note = AS64160 CDR3
DFGRDKNYLRPLLPHAYNY

SEQ ID NO: 181 - protein, 9 aa, synthetic construct
  REGION 1..9: note = AS64228 CDR3
LCWRENVNY

SEQ ID NO: 182 - protein, 15 aa, synthetic construct
  REGION 1..15: note = AS64300 CDR3
FNYGGAWYEERSYKY

SEQ ID NO: 183 - protein, 16 aa, synthetic construct
  REGION 1..16: note = AS64380 CDR3
SSRHRLGLNNPRDYDY

SEQ ID NO: 184 - protein, 16 aa, synthetic construct
  REGION 1..16: note = AS64395 CDR3
AASTAVRLLDPGDFAY

SEQ ID NO: 185 - protein, 7 aa, synthetic construct
  REGION 1..7: note = AS64443 CDR3
RFPAVTY

SEQ ID NO: 186 - protein, 16 aa, synthetic construct
  REGION 1..16: note = AS64511 CDR3
NLRIGGDWFDGRDFRA

SEQ ID NO: 187 - protein, 16 aa, synthetic construct
  REGION 1..16: note = AS64536 CDR3
KWGLGGGGLKSDTYMY

SEQ ID NO: 188 - protein, 20 aa, synthetic construct
  REGION 1..20: note = AS64597 CDR3
GGPPTDGDRWYPLRPPGYNY

SEQ ID NO: 189 - protein, 10 aa, synthetic construct
  REGION 1..10: note = AS64617 CDR3
IVGRTCSLNY

SEQ ID NO: 190 - protein, 16 aa, synthetic construct
  REGION 1..16: note = AS64634 CDR3
RRWVSGTCYWDSDFHY

SEQ ID NO: 191 - protein, 16 aa, synthetic construct
  REGION 1..16: note = AS69498 CDR3
SSRHRLRLSDPRDYDY

SEQ ID NO: 192 - protein, 17 aa, synthetic construct
  REGION 1..17: note = AS69500 CDR3
RAFQVGYCYLRTDVYNY

SEQ ID NO: 193 - protein, 16 aa, synthetic construct
  REGION 1..16: note = AS69527 CDR3
RRWACPRVGSWHEFAY

SEQ ID NO: 194 - protein, 16 aa, synthetic construct
  REGION 1..16: note = AS68280 CDR3
ARGRFIDWTKATQYDY

SEQ ID NO: 195 - protein, 20 aa, synthetic construct
  REGION 1..20: note = AS68355 CDR3
AIVGGFNAYCSGGYVLDFGA

SEQ ID NO: 196 - protein, 24 aa, synthetic construct
  REGION 1..24: note = AS69443 CDR3
DFLTGFYYSDSPHPAPCSASDFGY

SEQ ID NO: 197 - protein, 17 aa, synthetic construct
  REGION 1..17: note = AS75376 CDR3
DPNPDYMLPFRPSRRSW

SEQ ID NO: 198 - protein, 14 aa, synthetic construct
  REGION 1..14: note = AS75387 CDR3
DLRLPRAGGCAYSY

SEQ ID NO: 199 - protein, 13 aa, synthetic construct
  REGION 1..13: note = AS75695 CDR3
DRRGRVRRCEYNA

SEQ ID NO: 200 - protein, 17 aa, synthetic construct
  REGION 1..17: note = AS76169 CDR3
DRGGYANSCAVAARYDY

SEQ ID NO: 201 - protein, 16 aa, synthetic construct
  REGION 1..16: note = AS63931 CDR3
GWLSGGSWHVPGRYNY

SEQ ID NO: 202 - protein, 14 aa, synthetic construct
  REGION 1..14: note = AS63937 CDR3
DSRRPCMVAAGYTY

SEQ ID NO: 203 - protein, 17 aa, synthetic construct
  REGION 1..17: note = AS63948 CDR3
ASPRWGGTCRRWSEYNY

SEQ ID NO: 204 - protein, 15 aa, synthetic construct
  REGION 1..15: note = AS63956 CDR3
YQAKYCSGPCAPPTD

SEQ ID NO: 205 - protein, 13 aa, synthetic construct
  REGION 1..13: note = AS63965 CDR3
WCREYPGGILNNG

SEQ ID NO: 206 - protein, 10 aa, synthetic construct
  REGION 1..10: note = AS63993 CDR3
RTDSEHAFKF

SEQ ID NO: 207 - protein, 7 aa, synthetic construct
  REGION 1..7: note = AS63999 CDR3
RYTDYNY

SEQ ID NO: 208 - protein, 7 aa, synthetic construct
  REGION 1..7: note = AS64006 CDR3
RSRTMMY

SEQ ID NO: 209 - protein, 17 aa, synthetic construct
  REGION 1..17: note = AS64057 CDR3
DTTSGSCSGFWSTSRYY

SEQ ID NO: 210 - protein, 14 aa, synthetic construct
  REGION 1..14: note = AS64060 CDR3
DPTIGCPQTYRYNY

SEQ ID NO: 211 - protein, 16 aa, synthetic construct
  REGION 1..16: note = AS64071 CDR3
STKDQFYVFNPIGYDS

SEQ ID NO: 212 - protein, 21 aa, synthetic construct
  REGION 1..21: note = AS64093 CDR3
RSFSIGVCATQSGITWSNFAY

SEQ ID NO: 213 - protein, 10 aa, synthetic construct
  REGION 1..10: note = AS64118 CDR3
TWDSSCRFQY

SEQ ID NO: 214 - protein, 21 aa, synthetic construct
  REGION 1..21: note = AS64120 CDR3
RSFSIADCATQSGITRSNFAY

SEQ ID NO: 215 - protein, 19 aa, synthetic construct
  REGION 1..19: note = AS64124 CDR3
GRPYSLPLPLPLESGAYRY

SEQ ID NO: 216 - protein, 13 aa, synthetic construct
  REGION 1..13: note = AS64135 CDR3
DPMGGSRTPCTSA

SEQ ID NO: 217 - protein, 17 aa, synthetic construct
  REGION 1..17: note = AS64163 CDR3
DPSVCPGGMWYSKEYRY

SEQ ID NO: 218 - protein, 17 aa, synthetic construct
  REGION 1..17: note = AS64182 CDR3
SSPHWGGTCRRWSEYKY

SEQ ID NO: 219 - protein, 13 aa, synthetic construct
  REGION 1..13: note = AS64183 CDR3
DLSGGPAGCGYTH

SEQ ID NO: 220 - protein, 20 aa, synthetic construct
  REGION 1..20: note = AS64207 CDR3
GGPPTNGAKWYPLRPPGYNY

SEQ ID NO: 221 - protein, 13 aa, synthetic construct
  REGION 1..13: note = AS64276 CDR3
SLGPGRGACGYNY

SEQ ID NO: 222 - protein, 13 aa, synthetic construct
  REGION 1..13: note = AS64336 CDR3
RTGWAPRCAVPGY

SEQ ID NO: 223 - protein, 18 aa, synthetic construct
  REGION 1..18: note = AS64346 CDR3
VQSKSSNYVLRDASTYNY

SEQ ID NO: 224 - protein, 7 aa, synthetic construct
  REGION 1..7: note = AS64420 CDR3
RSRYATY

SEQ ID NO: 225 - protein, 17 aa, synthetic construct
  REGION 1..17: note = AS64473 CDR3
SSPQWGGTCRRWSEYNY

SEQ ID NO: 226 - protein, 7 aa, synthetic construct
  REGION 1..7: note = AS64475 CDR3
RDTARTY

SEQ ID NO: 227 - protein, 18 aa, synthetic construct
  REGION 1..18: note = AS64513 CDR3
GYYSGSGPGYLLPWRYNY

SEQ ID NO: 228 - protein, 22 aa, synthetic construct
  REGION 1..22: note = AS64562 CDR3
GFRPRGGGYTGDVLAQAAAYNY

SEQ ID NO: 229 - protein, 17 aa, synthetic construct
  REGION 1..17: note = AS64583 CDR3
KAHPDCSGDWSPSGYEY

SEQ ID NO: 230 - protein, 7 aa, synthetic construct
  REGION 1..7: note = AS64594 CDR3
RTQTRNY

SEQ ID NO: 231 - protein, 22 aa, synthetic construct
  REGION 1..22: note = AS64605 CDR3
RSNSYSYSSCDYGPLTRGGYNF

SEQ ID NO: 232 - protein, 7 aa, synthetic construct
  REGION 1..7: note = AS64606 CDR3
RLDEKMY

SEQ ID NO: 233 - protein, 21 aa, synthetic construct
  REGION 1..21: note = AS68121 CDR3
DPGSRTDDSCGTSYNKGNFGY

SEQ ID NO: 234 - protein, 20 aa, synthetic construct
  REGION 1..20: note = AS68170 CDR3
ASDVAVGVNSCGGRTAGFDA

SEQ ID NO: 235 - protein, 17 aa, synthetic construct
  REGION 1..17: note = AS63964 CDR3
EVVDPTWGSRDQRRYKY

SEQ ID NO: 236 - protein, 17 aa, synthetic construct
  REGION 1..17: note = AS64116 CDR3
DRWNSFANCGAWGRYTY

SEQ ID NO: 237 - protein, 18 aa, synthetic construct
  REGION 1..18: note = AS68270 CDR3
ASGWIVPSRSLTANLYRY

SEQ ID NO: 238 - protein, 16 aa, synthetic construct
  REGION 1..16: note = AS68320 CDR3
GRAGPWALMRPTEFGY

SEQ ID NO: 239 - protein, 14 aa, synthetic construct
  REGION 1..14: note = AS68351 CDR3
GAVRLSTSSVRDSS

SEQ ID NO: 240 - protein, 7 aa, synthetic construct
  REGION 1..7: note = AS75378 CDR3
RSYEYTY

SEQ ID NO: 241 - protein, 16 aa, synthetic construct
  REGION 1..16: note = AS75383 CDR3
DRRYGRQWYQPCEWNT

SEQ ID NO: 242 - protein, 20 aa, synthetic construct
  REGION 1..20: note = AS75751 CDR3
GFGYMNVIQALNGMRQNPDY

SEQ ID NO: 243 - protein, 16 aa, synthetic construct
  REGION 1..16: note = AS76422 CDR3
DRRDGRRWSQPCEWNT

SEQ ID NO: 244 - protein, 10 aa, synthetic construct
  REGION 1..10: note = AS64380VH4 CDR1
GNTYSSNYMG

SEQ ID NO: 245 - protein, 10 aa, synthetic construct
  REGION 1..10: note = AS64380VH5 CDR1
GNTYSSNYMG

SEQ ID NO: 246 - protein, 10 aa, synthetic construct
  REGION 1..10: note = AS64380VH6 CDR1
GNTYSSNYMG

SEQ ID NO: 247 - protein, 10 aa, synthetic construct
  REGION 1..10: note = AS64380VH7 CDR1
GNTYSSNYMG

SEQ ID NO: 248 - protein, 10 aa, synthetic construct
  REGION 1..10: note = AS64511VH4 CDR1
RATYSTNYIS

SEQ ID NO: 249 - protein, 10 aa, synthetic construct
  REGION 1..10: note = AS64511VH5 CDR1
RATYSTNYIS

SEQ ID NO: 250 - protein, 10 aa, synthetic construct
  REGION 1..10: note = AS64511VH6 CDR1
RATYSTNYIS

SEQ ID NO: 251 - protein, 10 aa, synthetic construct
  REGION 1..10: note = AS63997VH4 CDR1
FSGYGVSTMA

SEQ ID NO: 252 - protein, 10 aa, synthetic construct
  REGION 1..10: note = AS63997VH5 CDR1
FSGYGVSTMA

SEQ ID NO: 253 - protein, 10 aa, synthetic construct
  REGION 1..10: note = AS63997VH6 CDR1
FSGYGVSTMA

SEQ ID NO: 254 - protein, 17 aa, synthetic construct
  REGION 1..17: note = AS64380VH4 CDR2
VIYTRGGHTYYVDSVRG

SEQ ID NO: 255 - protein, 17 aa, synthetic construct
  REGION 1..17: note = AS64380VH5 CDR2
VIYTRGGHTYYVDSVRG

SEQ ID NO: 256 - protein, 17 aa, synthetic construct
  REGION 1..17: note = AS64380VH6 CDR2
VIYTRGGHTYYVDSVRG

SEQ ID NO: 257 - protein, 17 aa, synthetic construct
  REGION 1..17: note = AS64380VH7 CDR2
VIYTRGGHTYYVDSVRG

SEQ ID NO: 258 - protein, 17 aa, synthetic construct
  REGION 1..17: note = AS64511VH4 CDR2
TITTGDGETAYADSVKG

SEQ ID NO: 259 - protein, 17 aa, synthetic construct
  REGION 1..17: note = AS64511VH5 CDR2
TITTGDGETAYADSVKG

SEQ ID NO: 260 - protein, 17 aa, synthetic construct
  REGION 1..17: note = AS64511VH6 CDR2
TITTGDGETAYADSVKG

SEQ ID NO: 261 - protein, 17 aa, synthetic construct
  REGION 1..17: note = AS63997VH4 CDR2
AITVGSGNTYYADSVKG

SEQ ID NO: 262 - protein, 17 aa, synthetic construct
  REGION 1..17: note = AS63997VH5 CDR2
AITVGSGNTYYADSVKG

SEQ ID NO: 263 - protein, 17 aa, synthetic construct
  REGION 1..17: note = AS63997VH6 CDR2
AITVGSGNTYYADSVKG

SEQ ID NO: 264 - protein, 16 aa, synthetic construct
  REGION 1..16: note = AS64380VH4 CDR3
SSRHRLGLNNPRDYDY

SEQ ID NO: 265 - protein, 16 aa, synthetic construct
  REGION 1..16: note = AS64380VH5 CDR3
SSRHRLGLNNPRDYDY

SEQ ID NO: 266 - protein, 16 aa, synthetic construct
  REGION 1..16: note = AS64380VH6 CDR3
SSRHRLGLNNPRDYDY

SEQ ID NO: 267 - protein, 16 aa, synthetic construct
  REGION 1..16: note = AS64380VH7 CDR3
SSRHRLGLNNPRDYDY

SEQ ID NO: 268 - protein, 16 aa, synthetic construct
  REGION 1..16: note = AS64511VH4 CDR3
NLRIGGDWFDGRDFRA

SEQ ID NO: 269 - protein, 16 aa, synthetic construct
  REGION 1..16: note = AS64511VH5 CDR3
NLRIGGDWFDGRDFRA

SEQ ID NO: 270 - protein, 16 aa, synthetic construct
  REGION 1..16: note = AS64511VH6 CDR3
NLRIGGDWFDGRDFRA

SEQ ID NO: 271 - protein, 16 aa, synthetic construct
  REGION 1..16: note = AS63997VH4 CDR3
GYLSGGSWDVPGRYNY

SEQ ID NO: 272 - protein, 16 aa, synthetic construct
  REGION 1..16: note = AS63997VH5 CDR3
GYLSGGSWDVPGRYNY

SEQ ID NO: 273 - protein, 16 aa, synthetic construct
  REGION 1..16: note = AS63997VH6 CDR3
GYLSGGSWDVPGRYNY

SEQ ID NO: 274 - protein, 129 aa, synthetic construct
  REGION 1..129: note = Anti-DLL3 camel sdAb amino acid sequence AS63930
EVQLAESGGGSVQAGGSLRLSCAASGYTYSGNYMAWFRQAPGNEREGVAVVYNIDGGGRFTTYADSVKGRFTISRGNDKNTVYLQMNSLKPEDSGMYYCAAEVADPTWGSRDQRRYKYWGQGTQVTVSS

SEQ ID NO: 275 - protein, 118 aa, synthetic construct
  REGION 1..118: note = Anti-DLL3 camel sdAb amino acid sequence AS63932
QVQLEESGGGSVQAGGSLRLSCVASGYTYGSTFMGWFRQNPGKEREGVAVIYTGGGSTWYASSVKGRFTISQDNAKNTVYLQMNSLKPEDTAMYYCAARYGSGNVNYWGQGTQVTVSS

SEQ ID NO: 276 - protein, 130 aa, synthetic construct
  REGION 1..130: note = Anti-DLL3 camel sdAb amino acid sequence AS63951
QVHLMESGGGSVQAGGSLRLACETSRDIYGNNCMAWFRQAPGKEREGVASIYPAGGRPYYADSVKGRFTISQDNAKNTVYLQMDSLKPEDTAMYYCAARSFSIAVCATRSGITRSNFAYWGQGTQVTVSS

SEQ ID NO: 277 - protein, 129 aa, synthetic construct
  REGION 1..129: note = Anti-DLL3 camel sdAb amino acid sequence AS63984
QVKLVESGGGSVQAGGSLRLSCAASGYTYSSNFMGWFRQAPGKEREGVATIVSGGGTTYYADSVRGRFTISQDNAKNTVYLQMNSLKPEDTAMYYCAAGGPVTNAPRWYPLRPPGYNYWGQGTQVTVSS

SEQ ID NO: 278 - protein, 122 aa, synthetic construct
  REGION 1..122: note = Anti-DLL3 camel sdAb amino acid sequence AS63987
QVRLVESGGGSVQAGGSLRLSCEATGYRNCMAWFRQAPGKEREGVAVIYTPSGITDYASSVKGRFTISQNNARNTQYLQMNSLKPEDTAMYYCAADRPFVCNIANMRRSSNWGRGTQVTVSS

SEQ ID NO: 279 - protein, 125 aa, synthetic construct
  REGION 1..125: note = Anti-DLL3 camel sdAb amino acid sequence AS63997
QVRLVESGGGSVQAGGSLRLSCAGSFSGYGVSTMAWFRQAPGKEREGVAAITVGSGNTYYADSVKGRFTISRDNAKRTVFLQMNSLKPEDTAMYYCAVGYLSGGSWDVPGRYNYWGQGTQVTVSS

SEQ ID NO: 280 - protein, 125 aa, synthetic construct
  REGION 1..125: note = Anti-DLL3 camel sdAb amino acid sequence AS64047
QVHLVESGGGSVQAGGSLRLSCAASQYVYRWDLMGWFRQAPGKEREAVAAVYTGDGITYYADSVKGRFSISQDNAKNTVYLQMNSLKPEDTGMYFCAAGFVSGGRWNQSYRYKYWGQGTQVTVSS

SEQ ID NO: 281 - protein, 129 aa, synthetic construct
  REGION 1..129: note = Anti-DLL3 camel sdAb amino acid sequence AS64052
QVHLMESGGGSVQAGGSLRLSCAASGYTYRSNFMGWFRQAPGKEREGIATIHSGVATTYYADSVKGRFTISQDNAKNTVYLQMNSLKPEDTAMYYCAAGGPPANADRWYPLRPPGYNYWGQGTQVTVSS

SEQ ID NO: 282 - protein, 127 aa, synthetic construct
  REGION 1..127: note = Anti-DLL3 camel sdAb amino acid sequence AS64062
QVRLVESGGGSVQVGGSLRLSCAASRSPYSSSRCMGWFRQAPGKEREGVAALYTGGGSTSYADSVKGRFTISQDNAKNTVYLQMNSLKPEDTAMYYCAAVVPRGGSCRLDERGYYHWGQGTQVTVSS

SEQ ID NO: 283 - protein, 123 aa, synthetic construct
  REGION 1..123: note = Anti-DLL3 camel sdAb amino acid sequence AS64072
QVQLVESGGGSVQAGGFLRLSCALSGYSYYINLMAWFRQAPGKEREAVAAHGPVSGTAYYTDSVKGRFTISRDPGKNTMYLQMFSLQPEDTALYYCAAETTMGWAHERGYRYWGQGTQVTVSS

SEQ ID NO: 284 - protein, 127 aa, synthetic construct
  REGION 1..127: note = Anti-DLL3 camel sdAb amino acid sequence AS64097
QVHLMESGGGSVQAGGSLRLSCEASGYTYSRNCMGWFRQAPGKEREGVAAINTGGGSTYYADSLEGRFTISQDNAKNTMYLQMNSLKPEDTAMYYCAAGPDLGGSWCRPVERAFTYWGQGTQVTVSS

SEQ ID NO: 285 - protein, 125 aa, synthetic construct
  REGION 1..125: note = Anti-DLL3 camel sdAb amino acid sequence AS64114
QVQLQESGGGSVQAGGSLTLSCEASGNTYSTNYMGWFRQAPGKEREEVAVIYTRGGHTYYVDSVRGRFTISQDNAKNTVYLQMNSLKPEDTAMYYCAAASRHRLRLNNPRDYDYWGQGTQVTVSS

SEQ ID NO: 286 - protein, 116 aa, synthetic construct
  REGION 1..116: note = Anti-DLL3 camel sdAb amino acid sequence AS64123
QVQLAESGGGSVQAGGSLRLSCAASGYTYTSNWLGWFRQAPGKEREEVAIIYTGSGSTHYRSSVKGRFTISQDNAKNTVYLQMNSLKPEDTAMYYCAARFSEYNYWGQGTQVTVSS

SEQ ID NO: 287 - protein, 129 aa, synthetic construct
  REGION 1..129: note = Anti-DLL3 camel sdAb amino acid sequence AS64130
EVQLAESGGGSVQAGGSLRLSCAASGYTYRSNFMGWFRQAPAKEREGVATIDSRGTITYYADSVKGRFTISQDNEKNTVYLQMNSLKPEDTAMYYCAAGGPRTNDDRWYPLRPPGYNYWGQGTQVTVSS

SEQ ID NO: 288 - protein, 126 aa, synthetic construct
  REGION 1..126: note = Anti-DLL3 camel sdAb amino acid sequence AS64137
QVRLVESGGGSVQAGGSLRLSCAASGSTYSTNFMGWFRQAPGKEREGVATLVTWVERTAYADSVKGRFTISQDRAKNTVYLQMNSLKPEDTAMYYCAAAAASTDVRLLDPGDFAYWGQGTQVTVSS

SEQ ID NO: 289 - protein, 126 aa, synthetic construct
  REGION 1..126: note = Anti-DLL3 camel sdAb amino acid sequence AS64142
QVHLMESGGGLVQTGGSLRLSCTASGFTFDRNAMRWYRQAPGKEREGVSCIDWTGANIAYADSVKGRFTISRDNAKNTLYLQMNSLKPEDTGMYYCAADTTSGYCSGFWSTSRYSWGQGTQVTVSS

SEQ ID NO: 290 - protein, 126 aa, synthetic construct
  REGION 1..126: note = Anti-DLL3 camel sdAb amino acid sequence AS64154
QVQLKESGGGSVQAGGSLRLSCTASGYTYRYLYMGWFRQTPGKEREGVACIYTGSGSTGYADSVKGRFTISQDNAKNTVYLQMNNLKPEDTAMYYCAASSPRWGGTCRRWSQYNYWGQGTQVTVSS

SEQ ID NO: 291 - protein, 128 aa, synthetic construct
  REGION 1..128: note = Anti-DLL3 camel sdAb amino acid sequence AS64160
EVQLVESGGGSVQAGGSLRLSCAASVYTSSSYCMGWFRQAPGKEREGVAAMCFGGLVTHYADSVKGRFTISQDNAKNTVYLQMNSLKPEDTAMYYCAADFGRDKNYLRPLLPHAYNYWGQGTQVTVSS

SEQ ID NO: 292 - protein, 117 aa, synthetic construct
  REGION 1..117: note = Anti-DLL3 camel sdAb amino acid sequence AS64228
QVQLKESGGGSIQAGGSLRLSCAASGVSYNRCSMGWYRQAPGKGRELVSRIQPGGNTYYADSVKGRFTVSQDNAKNTVSLQMNSLKPEDTAMYYCNALCWRENVNYWGQGTQVTVSS

SEQ ID NO: 293 - protein, 124 aa, synthetic construct
  REGION 1..124: note = Anti-DLL3 camel sdAb amino acid sequence AS64300
QVHLVESGGGSVQTGGSLRLSCAVSGDIYNLMSMAWFRRAPGKEREGVAYINTIIGNTYYTDSVKGRFTISRDNSKNTLYLQMNNLKPEDTAMYYCAAFNYGGAWYEERSYKYWGQGTQVTVSS

SEQ ID NO: 294 - protein, 125 aa, synthetic construct
  REGION 1..125: note = Anti-DLL3 camel sdAb amino acid sequence AS64380
EVQLVESGGGSVQAGGSLTLSCEASGNTYSSNYMGWFRQAPGKEREEVAVIYTRGGHTYYVDSVRGRFTISQDNAKNTVYLQMNSLKPEDTAMYYCAASSRHRLGLNNPRDYDYWGQGTQVTVSS

SEQ ID NO: 295 - protein, 125 aa, synthetic construct
  REGION 1..125: note = Anti-DLL3 camel sdAb amino acid sequence AS64395
QVRLVESGGGSVQAGGSLRLSCAASGSTYSTNFMGWFRQAPGKEREGVATLVTWAERTAYADSVKGRFTISQDRAKNTVYLQMNGLKPEDTAMYYCAAAASTAVRLLDPGDFAYWGQGTQVTVSS

SEQ ID NO: 296 - protein, 116 aa, synthetic construct
  REGION 1..116: note = Anti-DLL3 camel sdAb amino acid sequence AS64443
QVHLVESGGGSVQAGGSLRLSCAASGYTDSSVYIGWFRQAPGKEREEVAIIYTGGESTHYRSSVKGRFTVSQDNAKNTLYLQMNSLKPEDTAMYYCAARFPAVTYWGQGTQVTVSS

SEQ ID NO: 297 - protein, 125 aa, synthetic construct
  REGION 1..125: note = Anti-DLL3 camel sdAb amino acid sequence AS64511
QVQLVESGGGSVQAGGSLRLSCAASRATYSTNYISWFRQAPGKEREAVATITTGDGETAYADSVKGRFTISRDNAKNTVYLQMNSLKPEDTAMYYCAANLRIGGDWFDGRDFRAWGQGTQVTVSS

SEQ ID NO: 298 - protein, 125 aa, synthetic construct
  REGION 1..125: note = Anti-DLL3 camel sdAb amino acid sequence AS64536
QVKLVESGGGSVQAGGSLRLSCAASRYTDNFVYMGWFRQAPGKEREGVALIYPGGGSTYYASSVKGRFTISQDNAKGTVHLQMNNLKPEDTAMYYCAAKWGLGGGGLKSDTYMYWGQGTQVTVSS

SEQ ID NO: 299 - protein, 129 aa, synthetic construct
  REGION 1..129: note = Anti-DLL3 camel sdAb amino acid sequence AS64597
QVHLVESGGGSVQAGGSLRLSCAASGYTYRVNFMGWFRQTPGKEREGVATIDSGVGTTYYADSVKGRFTISHNNAKNTIYLQMNSLKPEDTAMYYCAAGGPPTDGDRWYPLRPPGYNYWGQGTQVTVSS

SEQ ID NO: 300 - protein, 117 aa, synthetic construct
  REGION 1..117: note = Anti-DLL3 camel sdAb amino acid sequence AS64617
QVQLVESGGGSVQAGGSLRLSCAASGYTDRCSMAWYRQAPGKERELVSRISTSGFTNYAASVKGRFTISQDNAKNTVYLQMNSLNPGDTGMYYCAIIVGRTCSLNYWGNGILVTVSS

SEQ ID NO: 301 - protein, 127 aa, synthetic construct
  REGION 1..127: note = Anti-DLL3 camel sdAb amino acid sequence AS64634
QVRLVESGGGSVQAGGSLRLSCAASGYSFRGDFMCMGWFRQTPGKGREGVAVFYPGGGSTNYADSAKGRFTISQDNAKNTMYLQMNTLKPEDTAMYYCAARRWVSGTCYWDSDFHYWGQGTQVTVSS

SEQ ID NO: 302 - protein, 125 aa, synthetic construct
  REGION 1..125: note = Anti-DLL3 camel sdAb amino acid sequence AS69498
QVQLQESGGGSVQAGGSLRLSCEASGNTYSSNYMAWFRQAPGKEREEVAVIYTRGGHTYYIDSVRGRFTISQDNAKNTVYLQMNSLKPEDTAMYYCAASSRHRLRLSDPRDYDYWGQGTQVTVSS

SEQ ID NO: 303 - protein, 127 aa, synthetic construct
  REGION 1..127: note = Anti-DLL3 camel sdAb amino acid sequence AS69500
QVRLVESGGGSVQAGGSLRLSCAADRYTYSSACMGWFRQAPGKEREGVASIFTGTGGSTYYADSVKGRFTISQDNAKNTVYLQMNSLKPEDTAIYYCAARAFQVGYCYLRTDVYNYWGQGTQVTVSS

SEQ ID NO: 304 - protein, 125 aa, synthetic construct
  REGION 1..125: note = Anti-DLL3 camel sdAb amino acid sequence AS69527
EVQLAESGGGSVQAGGSLRLSCVASRYTFSSTCMAWFRQAPGKEREEVAAIYTDDGSTWYADSVKGRFTISRDNAKNTVYLQMNSLKPEDTAMYYCAARRWACPRVGSWHEFAYWGQGTQVTVSS

SEQ ID NO: 305 - protein, 125 aa, synthetic construct
  REGION 1..125: note = Anti-DLL3 camel sdAb amino acid sequence AS68280
QVQLVESGGGSVHPGGSLRLSCAASGSTYSSNYLGWFRQAPGKGRDWVAAISTGDGATAYADSVKGRFTISQDNAKNTVYLQMNSLKLEDSAMYYCAAARGRFIDWTKATQYDYWGQGTQVTVSS

SEQ ID NO: 306 - protein, 128 aa, synthetic construct
  REGION 1..128: note = Anti-DLL3 camel sdAb amino acid sequence AS68355
QMQLVESGGDSVQAGGSLRLSCAASGYTYSGVCMGWFRQAPGKEREGVAAIDSDGSTSYADSVKGRFTISKDNAKNTLYLQMNSLKPEDTAMYYCAAAIVGGFNAYCSGGYVLDFGAWGQGTQVTVSS

SEQ ID NO: 307 - protein, 132 aa, synthetic construct
  REGION 1..132: note = Anti-DLL3 camel sdAb amino acid sequence AS69443
EVQLAESGGGSVQAGGSLRLSCSASGFTFDDSDMAWYRQAPGDGCDLVSTISSDGSTYYADSVKGRFTISQDNAKNTVYLQMHSLKPEDTAVYYCAADFLTGFYYSDSPHPAPCSASDFGYWGQGTQVTVSS

SEQ ID NO: 308 - protein, 126 aa, synthetic construct
  REGION 1..126: note = Anti-DLL3 camel sdAb amino acid sequence AS75376
QVQLKESGGGSVQAGGSLRLSCAASGYTYSSHSMGWFRQAPGKEREGVAVIYTGDGSTYYADSVKGRFTISQDNAKNTVYLQMNSLKPEDTAMYYCAADPNPDYMLPFRPSRRSWWGQGTQVTVSS

SEQ ID NO: 309 - protein, 123 aa, synthetic construct
  REGION 1..123: note = Anti-DLL3 camel sdAb amino acid sequence AS75387
QVHLVESGGGSVQAGGSLRLSCAASGYPYSSPCMAWFRQAPGKEREGVLVAYTGGDIQYLTDSVKGRFTISRDNAKNTVYLQMNSLKPEDTAMYYCAADLRLPRAGGCAYSYWGQGTQVTVSS

SEQ ID NO: 310 - protein, 121 aa, synthetic construct
  REGION 1..121: note = Anti-DLL3 camel sdAb amino acid sequence AS75695
QVRLVESGGGSVQAGGSLRLSCVASGYTVSAYCMGWFRQVLGKGRERIAFIDAGGATIYADPVKGRFTISKDNAKNTLYLQMNSLKPEDTAMYYCVADRRGRVRRCEYNAWGQGTQVTVSS

SEQ ID NO: 311 - protein, 125 aa, synthetic construct
  REGION 1..125: note = Anti-DLL3 camel sdAb amino acid sequence AS76169
QVHLMESGGGSVQAGGSLRLSCAASGYIYSSFCMGWFRQAPGKEREVVAYIRDNIMTSYTDSVKGRFTISKDNAKRTLYLQMNGLKPEDTGMYYCAVDRGGYANSCAVAARYDYWGRGTQVTVSS

SEQ ID NO: 312 - protein, 125 aa, synthetic construct
  REGION 1..125: note = Anti-DLL3 camel sdAb amino acid sequence AS63931
EVQLAESGGGSVQAGGSLRLSCAGSFSGYGVSTMAWFRQAPGKEREGVAAITVGSGNTYYADSVTGRFTISRDNAKRTVYLQMNSLKPEDTAMYYCAAGWLSGGSWHVPGRYNYWGQGTQVTVSS

SEQ ID NO: 313 - protein, 123 aa, synthetic construct
  REGION 1..123: note = Anti-DLL3 camel sdAb amino acid sequence AS63937
QVKLVESGGGSVQAGGSLRLSCAASGSTISSRPMAWFRQAPGKEREGVACIHTGLGRTYYADSVKGRFTISQDNAKNTVYLQVNSLKPEDTAMYYCAADSRRPCMVAAGYTYWGQGTQVTVSS

SEQ ID NO: 314 - protein, 126 aa, synthetic construct
  REGION 1..126: note = Anti-DLL3 camel sdAb amino acid sequence AS63948
QVQLVESGGGSVQAGGSLRLSCTASGYTYRYLYMGWFRQTPGKEREGVACIYTGSGSTGYADSVKGRFTISQDNAENTVYLQMNSLKPEDTAMYYCAAASPRWGGTCRRWSEYNYWGQGTQVTVSS

SEQ ID NO: 315 - protein, 123 aa, synthetic construct
  REGION 1..123: note = Anti-DLL3 camel sdAb amino acid sequence AS63956
QVHLVESGGGLVQAGGSLRLSCAASGFTYSNCCMRWYRQAPGKARELVSLINSSGGTYYADSVRGRFTISKDNAKNTLYLQMNSLKPEDTAMYYCAAYQAKYCSGPCAPPTDWGQGTQVTVSS

SEQ ID NO: 316 - protein, 121 aa, synthetic construct
  REGION 1..121: note = Anti-DLL3 camel sdAb amino acid sequence AS63965
QVQLVESGGGSVQAGGSLRLSCVASGYSSGSCRMGWYRQAPGKERELVSKVISDGTTVYADSVKGRFTLSQGNAKNTVYLQMSSLLPEDTAMYYCNAWCREYPGGILNNGWGQGTQVTVSS

SEQ ID NO: 317 - protein, 118 aa, synthetic construct
  REGION 1..118: note = Anti-DLL3 camel sdAb amino acid sequence AS63993
QVKLVESGGGLVQAGGSLRLSCTVSGFTFDDLVMAWFRQAPGKERQLVSLVATAGNSVYADSVKGRFTLSRDNAHSTAYLQMNGLKPEDTAMYYCAARTDSEHAFKFWGQGTQVTVSS

SEQ ID NO: 318 - protein, 116 aa, synthetic construct
  REGION 1..116: note = Anti-DLL3 camel sdAb amino acid sequence AS63999
EVQLVESGGGSVQAGGSLRLSCAASGYTYSSNWMGWFRQAPGKEREEVAIIYTGGISTHYRSSVKGRFTISQDNAKNTVYLQMNSLKPEDTAMYYCAARYTDYNYWGQGTQVTVSS

SEQ ID NO: 319 - protein, 116 aa, synthetic construct
  REGION 1..116: note = Anti-DLL3 camel sdAb amino acid sequence AS64006
QVHLVESGGGSVQAGGSLRLSCEVSGYTGDTTYIGWFRQAPGKEREGVALIYTSGTSEYYADSVKGRFIISRDNAKNTVYLQMNSLKPEDTAMYYCGARSRTMMYWGQGTQVTVSS

SEQ ID NO: 320 - protein, 126 aa, synthetic construct
  REGION 1..126: note = Anti-DLL3 camel sdAb amino acid sequence AS64057
QVQLEESGGGLVQTGGSLRLSCTASGFTFDRNAMRWYRQAPGKEREGVSCISWTGANIAYADSVKGRFTISRDNAKNTLYLQMNSLKPEDTGMYYCAADTTSGSCSGFWSTSRYYWGQGTQVTVSS

SEQ ID NO: 321 - protein, 122 aa, synthetic construct
  REGION 1..122: note = Anti-DLL3 camel sdAb amino acid sequence AS64060
QVKLVESGGGSVQAGGSLRLSCAASGSTYCTYRMSWFRQAPGKEREFVAVIDSGGSTSYADSVKGRFTISRDNAKNTVYLQMNSLKPEDTAMYYCKTDPTIGCPQTYRYNYWGQGTQVTVSS

SEQ ID NO: 322 - protein, 125 aa, synthetic construct
  REGION 1..125: note = Anti-DLL3 camel sdAb amino acid sequence AS64071
QVHLMESGGGSVQAGGSLRLSCVASGNTYRLNSMGWFRQAPGKEREGVAFIVMIRGTTYYGASVKGRFTISQDNAQTTVYLQMSSLKPEDTAMYYCAASTKDQFYVFNPIGYDSWGQGTQVTVSS

SEQ ID NO: 323 - protein, 130 aa, synthetic construct
  REGION 1..130: note = Anti-DLL3 camel sdAb amino acid sequence AS64093
QVHLVESGGGSVQAGGSLRLSCATSRYIYGNNCMAWFRQAPGKEREGVASIYPAGGRTYYADSVKGRFTISQDNAKNTVYLQIDSLKPEDTAMYYCAARSFSIGVCATQSGITWSNFAYWGQGTQVTVSS

SEQ ID NO: 324 - protein, 117 aa, synthetic construct
  REGION 1..117: note = Anti-DLL3 camel sdAb amino acid sequence AS64118
QVQLAESGGGSVQAGGSLRLSCAASGYTYSACRMAWYRQAPGKERELVSFINSAGSTYYADSVKGRFAISRDNAKTTVYLQMNALKAEDTAIYYCNTWDSSCRFQYWGQGTQVTVSS

SEQ ID NO: 325 - protein, 130 aa, synthetic construct
  REGION 1..130: note = Anti-DLL3 camel sdAb amino acid sequence AS64120
QVRLVESGGGSVQAGGSLRLSCETSRYIYGNNCMAWFRQAPGKEREGVASIYPAGGRPYYADSVKGRFTISQDNAKNTVYLQMDSLKPEDTAMYYCAARSFSIADCATQSGITRSNFAYWGQGTQVTVSS

SEQ ID NO: 326 - protein, 128 aa, synthetic construct
  REGION 1..128: note = Anti-DLL3 camel sdAb amino acid sequence AS64124
QVKLVESGGGSVQTGGSLRLSCAVSTYTPSNNYMGWFRQAPGKEREGVAAIATIGGTTRYADSVKGRFTISQDGAKNTIYLQMNGLKPEDTAMYYCAAGRPYSLPLPLPLESGAYRYWGQGTQVTVSS

SEQ ID NO: 327 - protein, 121 aa, synthetic construct
  REGION 1..121: note = Anti-DLL3 camel sdAb amino acid sequence AS64135
QVKLVESGGGSVQAGGSLRLSCVASTSTYCRYYMRWYRQAPGKEREFVSAMQPDGTTSYSDSVKGRFTMSQDRANNMLYLQMNSLRPEDTAMYYCKRDPMGGSRTPCTSAWGQGTQVTVSS

SEQ ID NO: 328 - protein, 125 aa, synthetic construct
  REGION 1..125: note = Anti-DLL3 camel sdAb amino acid sequence AS64163
QVRLVESGGGSVQAGGSLRLSCAVSGYRYRWNCMAWFRQAPGKEREGVAAISTGSGSTYYAGSVKGRFTISQDNAKNMYLQMNSLKPEDTAMYYCAADPSVCPGGMWYSKEYRYWGQGTQVTVSS

SEQ ID NO: 329 - protein, 126 aa, synthetic construct
  REGION 1..126: note = Anti-DLL3 camel sdAb amino acid sequence AS64182
QVHLMESGGGSVQAGGSLRLSCTASGQTSRYLYMGWFRQTPGKEREGVACIYTGSGSTGYADSVKGRFTISQDNAKNTVYLQTNSLKPEDTAMYYCAASSPHWGGTCRRWSEYKYWGQGTQVTVSS

SEQ ID NO: 330 - protein, 122 aa, synthetic construct
  REGION 1..122: note = Anti-DLL3 camel sdAb amino acid sequence AS64183
QVHLVESGGGSVQAGGSLRLSCAASGHTYSANCMAWFRRAPGKEREWVASVYTDDDSTMYTDSVKGRFTIFQDNAKNTVYLQMNSLKPEDTGMYICAADLSGGPAGCGYTHWGQGTQVTVSS

SEQ ID NO: 331 - protein, 129 aa, synthetic construct
  REGION 1..129: note = Anti-DLL3 camel sdAb amino acid sequence AS64207
EVQLVESGGGSVQAGGSLRLSCAASGYTYSSNFMGWFRQAPGKEREGVATIVSGGGTTYYADSVRGRFTISQDNAKNTVYLQMNSLKPEDTAMYYCAAGGPPTNGAKWYPLRPPGYNYWGQGTQVTVSS

SEQ ID NO: 332 - protein, 122 aa, synthetic construct
  REGION 1..122: note = Anti-DLL3 camel sdAb amino acid sequence AS64276
QVHLMESGGGSVQAGGSLSLSCVVSGYTGSSRCMAWFRQAPGKEREAVAQIFTGRGTTGYADSVKGRFTISQDNAKNTVYLRMNSLRPEDTAIYYCAASLGPGRGACGYNYWGQGTQVTVSS

SEQ ID NO: 333 - protein, 121 aa, synthetic construct
  REGION 1..121: note = Anti-DLL3 camel sdAb amino acid sequence AS64336
QVQLVESGGGSVQAGGSLRLSCTTSGRTYSSCSMGWYRQAPGKERELVSHIFSDGSRYYADSVKGRFTISQDNAKNTVYLQMNSLKPEDTAMYYCNRRTGWAPRCAVPGYWGQGTQVTVSS

SEQ ID NO: 334 - protein, 127 aa, synthetic construct
  REGION 1..127: note = Anti-DLL3 camel sdAb amino acid sequence AS64346
QVHLVESGGGSVQAGGSLRLSCAASGYTYFMGWFRQAPQKEREWVATIGTGDIFNGAAYYVDSVKGRFAISQDNAKNTVYLQMNSLKPEDTAVYVCAAVQSKSSNYVLRDASTYNYWGQGTQVTVSS

SEQ ID NO: 335 - protein, 116 aa, synthetic construct
  REGION 1..116: note = Anti-DLL3 camel sdAb amino acid sequence AS64420
EVQLVESGGGSVQAEGSLRLSCAASGDTSRSVWMGWARQVPGKEREVVATISTAGGSTWYTDSVKGRFTISQDNAKNTVYLQMNSLKPEDTAIYYCAARSRYATYWGQGTQVTVSS

SEQ ID NO: 336 - protein, 126 aa, synthetic construct
  REGION 1..126: note = Anti-DLL3 camel sdAb amino acid sequence AS64473
QVRLVESGGGSVQAGGSLRLSCTASGYTYRYLYMAWFRQTPGKEREGVACIYTGSGTTGYADSVKGRFTISQDNAKNTVYLQMNSLNAEDTAMYYCAASSPQWGGTCRRWSEYNYWGQGTQVTVSS

SEQ ID NO: 337 - protein, 116 aa, synthetic construct
  REGION 1..116: note = Anti-DLL3 camel sdAb amino acid sequence AS64475
QVQLQESGGGSVQAGGSLRLSCAASGYTWSRNWMGWFRQAPGKEREGFATITISGGSTWYADSVKGRFTISLDNAGNTVYLQMNSLKPEDTAMYYCAARDTARTYWGQGTQVTVSS

SEQ ID NO: 338 - protein, 127 aa, synthetic construct
  REGION 1..127: note = Anti-DLL3 camel sdAb amino acid sequence AS64513
EVQLVESGGGSVQAGGSLRLSCVASDYPYIDNCMGWFRQGPGKEREGVAAACTGGGSTYYADSVKGRFTISRDNAKNTVYLQMNSLKPEDTDVYYCATGYYSGSGPGYLLPWRYNYWGQGTQVTVSS

SEQ ID NO: 339 - protein, 131 aa, synthetic construct
  REGION 1..131: note = Anti-DLL3 camel sdAb amino acid sequence AS64562
EVQLVESGGGSVQAGGSLRLSCAASGYTARRDFMAWFRQVPGKEREGVAVIHTGGDTTYYADSVKGRFTISRDNAQNIMNLQMNSLKPEDTAMYYCAAGFRPRGGGYTGDVLAQAAAYNYWGQGTQVTVSS

SEQ ID NO: 340 - protein, 126 aa, synthetic construct
  REGION 1..126: note = Anti-DLL3 camel sdAb amino acid sequence AS64583
EVQLAESGGGLVQAGGSLRLSCTASGFTIAVYTMGWFRQAPGKEREGISCTSWAGGRTYTADSVKGRFTISRDNAKNTLYLQMNSLKPEDTAMYYCAAKAHPDCSGDWSPSGYEYWGQGTQVTVSS

SEQ ID NO: 341 - protein, 116 aa, synthetic construct
  REGION 1..116: note = Anti-DLL3 camel sdAb amino acid sequence AS64594
QVHLVESGGGSVQAGGSLRLSCAASGYTYNSNYMGWFRQAPGKEREGVALIYTGGGSTYYADSVKGRFTISRDNAKNTVYLQMNSLKPEDTAMYYCSVRTQTRNYWGQGTQVTVSS

SEQ ID NO: 342 - protein, 131 aa, synthetic construct
  REGION 1..131: note = Anti-DLL3 camel sdAb amino acid sequence AS64605
QVKLVESGGGSVQAGGSLRLSCAVSRYPYSSICMGWFRQAPGKESEGVARIYTGTGSTWYTDSVKGRFTIARDNAQNTVYLQMNSLKPEDTAMYYCAARSNSYSYSSCDYGPLTRGGYNFWGQGTQVTVSS

SEQ ID NO: 343 - protein, 115 aa, synthetic construct
  REGION 1..115: note = Anti-DLL3 camel sdAb amino acid sequence AS64606
EVQLAESGGGSVQAGGSLRLSCAVSGYTSRSNYMGWFRQAPGKEREGVALIYTRGGSTYYASSVKGRFTISQDSAKKTYLQMNSVKPEDTAMYYCALRLDEKMYWGQGTQVTVSS

SEQ ID NO: 344 - protein, 133 aa, synthetic construct
  REGION 1..133: note = Anti-DLL3 camel sdAb amino acid sequence AS68121
EVQLAESGGGSVQAGGSLRLSCDASGYTYSRNCMGWFRQAPGKEREGVAAFYTDYIRFGRTYYADSVKGRFTIFQDNAKNTVYLQMNSLKPEDTAMYYCAADPGSRTDDSCGTSYNKGNFGYWGQGTQVTVSS

SEQ ID NO: 345 - protein, 130 aa, synthetic construct
  REGION 1..130: note = Anti-DLL3 camel sdAb amino acid sequence AS68170
QVQLVESGGGSVQAGGSLRLSCTASGYTYRSNCMGWFRQAPGKEREGVATIYTGGGRNLYYADSVKGRFTISRDNAKNTLYLQMNSLKPEDSARYYCAAASDVAVGVNSCGGRTAGFDAWGQGTQVTVSS

SEQ ID NO: 346 - protein, 125 aa, synthetic construct
  REGION 1..125: note = Anti-DLL3 camel sdAb amino acid sequence AS63964
QVRLVESGGGSVQAGGSLRLSCSASGYTYSYNNMGWFRQAPGNEREGVAAISGGRFTAYADSVKGRFTISRDNAENTLYLQMNNLKPEDTGMYYCAAEVVDPTWGSRDQRRYKYWGQGTQVTVSS

SEQ ID NO: 347 - protein, 124 aa, synthetic construct
  REGION 1..124: note = Anti-DLL3 camel sdAb amino acid sequence AS64116
QVKLVESGGGSVQAGGSLRLSCAASGYIYSCVGWFRQAPGKEREGVAGISTGGGGTVYADSVKGQFTISRDNAKNTVYLQMDSLKPEDTAMYYCAADRWNSFANCGAWGRYTYWGQGTQVTVSS

SEQ ID NO: 348 - protein, 130 aa, synthetic construct
  REGION 1..130: note = Anti-DLL3 camel sdAb amino acid sequence AS68270
QVQLAESGGGSVQAGGSLRLSCVASGYPSSTYYMLSMAWFRQAPGKEREGVAAITSGTGSTSYADSVKDRFTISKDYANNTLYLHINNLKPEDTAMYYCAAASGWIVPSRSLTANLYRYWGQGTQVTVSS

SEQ ID NO: 349 - protein, 125 aa, synthetic construct
  REGION 1..125: note = Anti-DLL3 camel sdAb amino acid sequence AS68320
QVHLVESGGDSVQAGGSLRLSCAASGYTYNTNYMGWFRQAPGKEREGVAAIYRHSGNTAYADSVKGRFTISQDYAKNTVYLQMNSLKPEDTAMYYCAAGRAGPWALMRPTEFGYWGQGTQVTVSS

SEQ ID NO: 350 - protein, 123 aa, synthetic construct
  REGION 1..123: note = Anti-DLL3 camel sdAb amino acid sequence AS68351
QVQLEESGGGLVQPGGSLRLSCAASGDTFRAYYMNWVRQAPGKGFEWVSGISASGGRTSYADSVKGRFTISRDNAKNTLYLQLNSLSTEDTGMYYCVKGAVRLSTSSVRDSSWGQGTQVTVSS

SEQ ID NO: 351 - protein, 116 aa, synthetic construct
  REGION 1..116: note = Anti-DLL3 camel sdAb amino acid sequence AS75378
QVQLEESGGGSVQAGGSLRLSCVVSGNTRSTTYMGWFRQAPGKEREGVAIVYTGGRDTYYAASVKGRFTISQDNAKTTIYLQMNSLEPEDTAMYYCAARSYEYTYWGRGTQVTVSS

SEQ ID NO: 352 - protein, 124 aa, synthetic construct
  REGION 1..124: note = Anti-DLL3 camel sdAb amino acid sequence AS75383
EVQLAESGGGSVQAGGSLRLSCVASGYTFSSYCLGWFRQAPGKQRQGVATFNNRGVANYHDSVKGRFTASVDNAKNTLLLQMNSLEPDDTAMYYCAADRRYGRQWYQPCEWNTWGQGTQVTVSS

SEQ ID NO: 353 - protein, 129 aa, synthetic construct
  REGION 1..129: note = Anti-DLL3 camel sdAb amino acid sequence AS75751
QVRLVESGGGSVQAGGSLRLSCVASGYFYNTYYFMGWFRQAPGKEREGVAAIDTDGRTSYADSVKGRFTISKDNAKNTLYLQMNSLKPEDTAMYYCAAGFGYMNVIQALNGMRQNPDYWGQGTQVTVSS

SEQ ID NO: 354 - protein, 124 aa, synthetic construct
  REGION 1..124: note = Anti-DLL3 camel sdAb amino acid sequence AS76422
QVKLVESGGGSVQAGGSLRLSCAASGYTFAGNCLGWFRQAPGKGREGVVTYNNFGVANYADSVKGRFTVSQDNAKNTLLLQMNSLEPEDTAMYYCAADRRDGRRWSQPCEWNTWGQGTQVTVSS

SEQ ID NO: 355 - protein, 125 aa, synthetic construct
  REGION 1..125: note = Anti-DLL3 humanized sdAb amino acid sequence AS64380VH4
EVQLVESGGGLVQPGGSLRLSCAASGNTYSSNYMGWFRQAPGKGLEEVAVIYTRGGHTYYVDSVRGRFTISRDNAKNSLYLQMNSLRAEDTAVYYCAASSRHRLGLNNPRDYDYWGQGTLVTVSS

SEQ ID NO: 356 - protein, 125 aa, synthetic construct
  REGION 1..125: note = Anti-DLL3 humanized sdAb amino acid sequence AS64380VH5
EVQLVESGGGLVQPGGSLRLSCAASGNTYSSNYMGWFRQAPGKGLEEVAVIYTRGGHTYYVDSVRGRFTISQDNAKNSLYLQMNSLRAEDTAVYYCAASSRHRLGLNNPRDYDYWGQGTLVTVSS

SEQ ID NO: 357 - protein, 125 aa, synthetic construct
  REGION 1..125: note = Anti-DLL3 humanized sdAb amino acid sequence AS64380VH6
EVQLVESGGGLVQPGGSLRLSCAASGNTYSSNYMGWFRQAPGKGLEEVAVIYTRGGHTYYVDSVRGRFTISQDNAKNSVYLQMNSLRAEDTAMYYCAASSRHRLGLNNPRDYDYWGQGTLVTVSS

SEQ ID NO: 358 - protein, 125 aa, synthetic construct
  REGION 1..125: note = Anti-DLL3 humanized sdAb amino acid sequence AS64380VH7
EVQLVESGGGLVQPGGSLRLSCAASGNTYSSNYMGWFRQAPGKGREEVAVIYTRGGHTYYVDSVRGRFTISQDNAKNSVYLQMNSLRAEDTAMYYCAASSRHRLGLNNPRDYDYWGQGTLVTVSS

SEQ ID NO: 359 - protein, 125 aa, synthetic construct
  REGION 1..125: note = Anti-DLL3 humanized sdAb amino acid sequence AS64511VH4
EVQLVESGGGLVQPGGSLRLSCAASRATYSTNYISWFRQAPGKGLEAVATITTGDGETAYADSVKGRFTISRDNAKNSLYLQMNSLRAEDTAVYYCAANLRIGGDWFDGRDFRAWGQGTLVTVSS

SEQ ID NO: 360 - protein, 125 aa, synthetic construct
  REGION 1..125: note = Anti-DLL3 humanized sdAb amino acid sequence AS64511VH5
EVQLVESGGGLVQPGGSLRLSCAASRATYSTNYISWFRQAPGKGLEAVATITTGDGETAYADSVKGRFTISRDNAKNSVYLQMNSLRAEDTAMYYCAANLRIGGDWFDGRDFRAWGQGTLVTVSS

SEQ ID NO: 361 - protein, 125 aa, synthetic construct
  REGION 1..125: note = Anti-DLL3 humanized sdAb amino acid sequence AS64511VH6
EVQLVESGGGLVQPGGSLRLSCAASRATYSTNYISWFRQAPGKGREAVATITTGDGETAYADSVKGRFTISRDNAKNSVYLQMNSLRAEDTAMYYCAANLRIGGDWFDGRDFRAWGQGTLVTVSS

SEQ ID NO: 362 - protein, 125 aa, synthetic construct
  REGION 1..125: note = Anti-DLL3 humanized sdAb amino acid sequence AS63931VH4
QVQLVESGGGVVQPGGSLRLSCAGSFSGYGVSTMAWFRQAPGKGLEGVAAITVGSGNTYYADSVTGRFTISRDNSKNTLYLQMNSLRAEDTAVYYCAAGWLSGGSWHVPGRYNYWGQGTLVTVSS

SEQ ID NO: 363 - protein, 125 aa, synthetic construct
  REGION 1..125: note = Anti-DLL3 humanized sdAb amino acid sequence AS63931VH5
QVQLVESGGGVVQPGGSLRLSCAGSFSGYGVSTMAWFRQAPGKGLEGVAAITVGSGNTYYADSVTGRFTISRDNSKNTVYLQMNSLRAEDTAMYYCAAGWLSGGSWHVPGRYNYWGQGTLVTVSS

SEQ ID NO: 364 - protein, 125 aa, synthetic construct
  REGION 1..125: note = Anti-DLL3 humanized sdAb amino acid sequence AS63931VH6
QVQLVESGGGVVQPGGSLRLSCAGSFSGYGVSTMAWFRQAPGKGREGVAAITVGSGNTYYADSVTGRFTISRDNSKNTVYLQMNSLRAEDTAMYYCAAGWLSGGSWHVPGRYNYWGQGTLVTVSS

SEQ ID NO: 365 - protein, 125 aa, synthetic construct
  REGION 1..125: note = Anti-DLL3 humanized sdAb amino acid sequence AS63997VH4
QVQLVESGGGVVQPGGSLRLSCAASFSGYGVSTMAWFRQAPGKGLEGVAAITVGSGNTYYADSVKGRFTISRDNSKNTLYLQMNSLRAEDTAVYYCAVGYLSGGSWDVPGRYNYWGQGTLVTVSS

SEQ ID NO: 366 - protein, 125 aa, synthetic construct
  REGION 1..125: note = Anti-DLL3 humanized sdAb amino acid sequence AS63997VH5
QVQLVESGGGVVQPGGSLRLSCAASFSGYGVSTMAWFRQAPGKGLEGVAAITVGSGNTYYADSVKGRFTISRDNSKNTVYLQMNSLRAEDTAMYYCAVGYLSGGSWDVPGRYNYWGQGTLVTVSS

SEQ ID NO: 367 - protein, 125 aa, synthetic construct
  REGION 1..125: note = Anti-DLL3 humanized sdAb amino acid sequence AS63997VH6
QVQLVESGGGVVQPGGSLRLSCAASFSGYGVSTMAWFRQAPGKGREGVAAITVGSGNTYYADSVKGRFTISRDNSKNTVYLQMNSLRAEDTAMYYCAVGYLSGGSWDVPGRYNYWGQGTLVTVSS

SEQ ID NO: 368 - DNA, 387 bp, synthetic construct
  misc_feature 1..387: note = Camel sdAb AS63930 Nucleic Acid Sequence
  source 1..387: mol_type = other DNA
gaggtgcaactggcggagtctgggggaggatcggtgcaggctggagggtctctgagactctcctgtgcagcctctggatacacctacagtggcaactatatggcctggttccgccaggctccagggaacgagcgcgagggggtcgcagttgtttataatattgacggtggcggtcgtttcactacctatgccgactccgtgaagggccgattcaccatctcccgaggcaacgacaagaacacggtgtatctgcaaatgaacagcctgaaacctgaggatagtggcatgtactactgtgcggcagaggtagctgatccgacctgggggtcgcgtgaccaaagacgatataagtactggggccaggggacccaggtcaccgtctcctca

SEQ ID NO: 369 - DNA, 354 bp, synthetic construct
  misc_feature 1..354: note = Camel sdAb AS63932 Nucleic Acid Sequence
  source 1..354: mol_type = other DNA
caggtgcaattggaggagtctgggggaggctcggtgcaggctggagggtctctgagactctcctgtgtagcctctggatacacctacggtagcaccttcatgggctggttccgccagaatccagggaaggagcgcgagggggtcgcagttatttatactggtggtggtagtacatggtatgccagctccgtgaagggccgattcaccatctcccaggacaacgccaagaacacggtgtatctgcaaatgaacagcctgaaacctgaggacactgccatgtactactgtgcggcgcgttacgggtcgggaaacgttaactactggggccaggggacccaggtcaccgtctcctca

SEQ ID NO: 370 - DNA, 390 bp, synthetic construct
  misc_feature 1..390: note = Camel sdAb AS63951 Nucleic Acid Sequence
  source 1..390: mol_type = other DNA
caggtgcacctgatggagtctgggggaggctcggtgcaggctggagggtctctgagactcgcctgtgaaacctctagagacatctacggtaacaactgcatggcctggttccgccaggctccagggaaggagcgcgagggagtcgcgtctatttatcctgctggtggtcgcccgtactatgccgactccgtgaagggccgattcaccatctcccaagacaacgccaagaacacggtgtatctgcaaatggacagcctgaaacctgaggacacggccatgtactactgcgcggcacgctctttttcgatagcagtttgcgcgacgcgctctggtattaccaggtctaattttgcttactggggccaggggacccaggtcaccgtctcctca

SEQ ID NO: 371 - DNA, 387 bp, synthetic construct
  misc_feature 1..387: note = Camel sdAb AS63984 Nucleic Acid Sequence
  source 1..387: mol_type = other DNA
caggtgaagttggtggagtctgggggaggctcggtgcaggctggagggtctctgagactctcctgtgcagcctctggatacacctacagtagcaacttcatgggctggttccgccaggctccagggaaggagcgcgagggggtcgcaactattgtttctggtggtggtaccacatactatgccgactccgtgaggggccgattcaccatctcccaagacaacgccaagaacacggtgtatctgcaaatgaacagcctgaaacctgaggacactgccatgtactactgtgcggcagggggccccgttacgaacgcacctagatggtaccccctccgacctcctggttataactactggggccaggggacccaggtcaccgtctcctca

SEQ ID NO: 372 - DNA, 366 bp, synthetic construct
  misc_feature 1..366: note = Camel sdAb AS63987 Nucleic Acid Sequence
  source 1..366: mol_type = other DNA
caggtgaggttggtggagtctgggggaggctcggtgcaggctggagggtctctgagactctcctgtgaagccactggatatagaaactgcatggcctggttccgccaagctccagggaaggaacgcgagggggtcgcagttatttatactcctagtggtatcacggactatgcaagctccgtgaagggccgattcaccatctcccaaaacaacgccaggaacacgcagtatctgcaaatgaacagcctgaaacctgaggacactgccatgtactactgtgcggcagatcgaccctttgtttgtaatatagcgaatatgagaaggtcctccaactggggccgggggacccaggtcaccgtctcctca

SEQ ID NO: 373 - DNA, 375 bp, synthetic construct
  misc_feature 1..375: note = Camel sdAb AS63997 Nucleic Acid Sequence
  source 1..375: mol_type = other DNA
caggtgaggttggtggagtctgggggaggctcggtgcaggctggagggtctctgagactctcctgtgcaggctctttctctggatacggcgtcagtaccatggcctggttccgccaggctccagggaaggagcgcgagggggtcgcagctattacagttggtagtggaaacacatactatgccgactccgtgaagggccgattcaccatctcccgagacaacgccaagaggacggtgtttttgcaaatgaacagcctgaaacctgaggacactgccatgtactactgtgcggtcggatacttgtcgggtggtagttgggacgttcccggaaggtataactactggggccaggggacccaggtcaccgtctcctca

SEQ ID NO: 374 - DNA, 375 bp, synthetic construct
  misc_feature 1..375: note = Camel sdAb AS64047 Nucleic Acid Sequence
  source 1..375: mol_type = other DNA
caggtgcacctggtggagtctgggggaggctcggtgcaggctggagggtctctgagactctcctgtgcagcctctcagtacgtttacaggtgggacctcatgggctggttccgccaggctccagggaaggagcgcgaggcggtcgctgctgtttatactggtgatggtattacatactatgccgactccgtgaagggccgattcagcatttcccaagacaacgccaagaacacggtgtatctgcaaatgaacagcctgaaacctgaggacactggcatgtacttctgtgcggcaggcttcgtctctggtggtagatggaaccagtcatatcgttataaatactggggccaggggacccaggtcaccgtctcctca

SEQ ID NO: 375 - DNA, 387 bp, synthetic construct
  misc_feature 1..387: note = Camel sdAb AS64052 Nucleic Acid Sequence
  source 1..387: mol_type = other DNA
caggtgcacctgatggagtctgggggaggctcggtgcaggctggagggtctctgagactctcctgtgcagcctctggatacacctaccgcagcaacttcatgggctggttccgccaggctccagggaaggagcgcgaggggatcgcaactattcattctggtgtggctaccacatactatgccgactccgtgaagggccgattcaccatctcccaagacaacgccaagaacacggtgtatctgcaaatgaacagcctgaaacctgaggacactgccatgtactactgtgcggcagggggcccccctgcgaacgctgatagatggtaccccctccgacctcctggttataactactggggccaggggacccaggtcaccgtctcctca

SEQ ID NO: 376 - DNA, 381 bp, synthetic construct
  misc_feature 1..381: note = Camel sdAb AS64062 Nucleic Acid Sequence
  source 1..381: mol_type = other DNA
caggtgaggttggtggagtctgggggaggctcggtgcaggttggagggtctctgagactctcctgtgcagcctctagatctccctacagtagcagtaggtgcatggggtggttccgccaggctccagggaaggagcgcgagggggtcgcagctctttatactggtggtggtagcacatcctatgccgactccgtgaagggccgattcaccatctcccaagacaacgccaagaatacggtgtatctgcaaatgaacagcctgaaacctgaggacactgccatgtactactgtgcggcagttgtccctaggggtggtagctgccgtcttgatgaaagagggtattaccactggggccaggggacccaggtcaccgtctcctca

SEQ ID NO: 377 - DNA, 369 bp, synthetic construct
  misc_feature 1..369: note = Camel sdAb AS64072 Nucleic Acid Sequence
  source 1..369: mol_type = other DNA
caggtgcagctggtggagtctgggggaggctcggtgcaggccggagggtttctgagactctcctgtgcactctctggatacagctactatattaacttgatggcgtggttccgtcaggctccagggaaggagcgcgaggcagtcgcagctcatggtcctgtgagtgggacagcatactataccgactccgtgaagggccgattcaccatctcccgagaccccggcaagaacacgatgtatcttcaaatgtttagcctgcaaccggaggacactgccctctactactgtgcggcggaaacgactatgggttgggcccacgaacgcgggtataggtactggggccaggggacccaggtcaccgtctcctca

SEQ ID NO: 378 - DNA, 381 bp, synthetic construct
  misc_feature 1..381: note = Camel sdAb AS64097 Nucleic Acid Sequence
  source 1..381: mol_type = other DNA
caggtgcacctgatggagtctgggggaggctcggtgcaggctggagggtctctgagactctcctgtgaagcctctggatacacctacagtcgcaactgcatgggctggttccgccaggctccagggaaggagcgcgagggggtcgcagctattaacactggtggtggtagcacatattatgccgactcccttgagggccgattcaccatctcccaagacaacgccaagaatactatgtatctgcaaatgaacagcctgaaacctgaggacactgccatgtactactgtgcggcaggtcccgatctcggtggtagctggtgtcggcccgttgagcgggcttttacgtactggggccaggggacccaggtcaccgtctcctca

SEQ ID NO: 379 - DNA, 375 bp, synthetic construct
  misc_feature 1..375: note = Camel sdAb AS64114 Nucleic Acid Sequence
  source 1..375: mol_type = other DNA
caggtgcaactgcaggagtctggggggggctcggtgcaggctggagggtctctgacactctcctgtgaagcctctggaaacacctacagtactaattacatgggctggttccgccaggctccagggaaggagcgcgaagaggtcgcggttatttacactcgtggtggtcacacatactatgtcgactccgtgaggggccgattcaccatctcccaagacaacgccaagaacacggtgtatctgcaaatgaacagcctgaaacctgaggacactgccatgtactactgtgcggcagcttcacgacatagactccgtttaaataacccacgggactatgactactggggccaggggacccaggtcaccgtctcctca

SEQ ID NO: 380 - DNA, 348 bp, synthetic construct
  misc_feature 1..348: note = Camel sdAb AS64123 Nucleic Acid Sequence
  source 1..348: mol_type = other DNA
caggtgcaactggcggagtctgggggaggctcggtgcaggctggagggtctctgagactctcctgtgcagcctctggatacacttatacgagcaactggctgggctggttccgccaggctccagggaaggagcgcgaggaggtcgcaattatttatactggtagtggtagtacacactatcgcagctccgtgaagggccgattcaccatctcccaagacaacgccaagaacacggtgtatctgcaaatgaacagcctgaaacctgaggacactgccatgtactactgtgcggcgcgtttctcagagtataattactggggccaggggacccaggtcaccgtctcctca

SEQ ID NO: 381 - DNA, 387 bp, synthetic construct
  misc_feature 1..387: note = Camel sdAb AS64130 Nucleic Acid Sequence
  source 1..387: mol_type = other DNA
gaggtgcaactggcggagtctgggggaggctcggtgcaggctggagggtctctgagactctcctgtgcagcctctggatacacctaccgtagcaacttcatgggctggttccgccaggctccggcgaaggagcgcgagggggtcgcaactattgattctcgtggtactatcacatactatgccgactccgtgaagggccgattcaccatctcccaagacaacgagaagaacacggtgtatctgcaaatgaacagcctgaaacctgaggacactgccatgtactactgtgcggcagggggcccccgcacgaacgatgatagatggtaccccctccgacctcctggttataactactggggccaggggacccaggtcaccgtctcctca

SEQ ID NO: 382 - DNA, 378 bp, synthetic construct
  misc_feature 1..378: note = Camel sdAb AS64137 Nucleic Acid Sequence
  source 1..378: mol_type = other DNA
caggtgaggttagtggagtctgggggaggctcggtgcaggctggagggtctctgagactctcctgtgctgcctctggatccacctacagtacaaacttcatgggctggttccgccaggctccagggaaggagcgcgagggggtcgcaacgctggttacttgggttgaacgcacagcctatgccgactccgtgaagggccgattcaccatctcccaagaccgcgccaagaacacggtgtatctacaaatgaacagcctgaaacctgaggacactgccatgtactactgtgcggcagccgccgcttccactgatgtacgtctcctcgacccgggggactttgcttactggggccaggggacccaggtcaccgtctcctca

SEQ ID NO: 383 - DNA, 378 bp, synthetic construct
  misc_feature 1..378: note = Camel sdAb AS64142 Nucleic Acid Sequence
  source 1..378: mol_type = other DNA
caggtgcacctgatggagtctgggggaggcttggtgcagacaggggggtctctgagactctcctgtacagcctctggattcacttttgatcgtaatgccatgcgctggtaccgccaggctccagggaaggagcgcgagggggtctcatgtattgattggacgggtgcaaatattgcctatgcagactccgtgaagggccgattcaccatctccagagacaacgccaagaacacgctgtatctgcaaatgaacagcctgaaacctgaggacacgggcatgtattactgtgcggcagatacgacgtcggggtattgttcaggcttttggtctacgagccggtactcatggggccaggggacccaggtcaccgtctcctca

SEQ ID NO: 384 - DNA, 378 bp, synthetic construct
  misc_feature 1..378: note = Camel sdAb AS64154 Nucleic Acid Sequence
  source 1..378: mol_type = other DNA
caggtgcaattgaaggagtctgggggaggctcggtgcaggctggagggtctctgagactctcctgtacagcctctggatacacctacagatacctctacatgggctggttccgccagactccagggaaggagcgcgagggggtcgcatgtatttatactggtagtggtagcacagggtatgccgactccgtgaagggccgattcaccatctcccaagacaacgccaagaacacggtgtatctgcaaatgaacaacctgaaacctgaggacactgccatgtactactgtgcggcaagttcgccccggtggggcggtacctgtcgacgctggtctcagtataactactggggccaggggacccaggtcaccgtctcctca

SEQ ID NO: 385 - DNA, 384 bp, synthetic construct
  misc_feature 1..384: note = Camel sdAb AS64160 Nucleic Acid Sequence
  source 1..384: mol_type = other DNA
gaggtgcagctggtggagtctgggggaggctcggtgcaggctggagggtctctgagactctcctgtgcggcctctgtatacaccagcagtagctactgcatgggctggttccgccaggctccagggaaggagcgcgagggggtcgcagctatgtgttttggtggtcttgtcacacactatgccgactccgtgaagggccgattcaccatctcccaagacaatgccaagaacacggtgtatctgcaaatgaacagcctgaaacctgaggacactgccatgtactactgtgcggcagatttcggcagggataaaaactatttacgaccgttactgccccatgcatataactactggggccaagggacccaggtcaccgtctcctca

SEQ ID NO: 386 - DNA, 351 bp, synthetic construct
  misc_feature 1..351: note = Camel sdAb AS64228 Nucleic Acid Sequence
  source 1..351: mol_type = other DNA
caggtgcaattgaaggagtctgggggaggttcgatccaggctggagggtctctgagactctcctgtgcagcctctggagtctcctacaataggtgcagtatgggctggtaccgccaggctccagggaaggggcgcgagttggtctcacgtattcagccgggtggtaatacatactatgcagactccgtgaagggccgattcaccgtctcccaagacaacgccaagaacacagtatctctacaaatgaacagcctgaaacctgaggacacggccatgtattactgtaacgcactgtgctggcgggagaatgttaactactggggccaggggacccaggtcaccgtctcctca

SEQ ID NO: 387 - DNA, 372 bp, synthetic construct
  misc_feature 1..372: note = Camel sdAb AS64300 Nucleic Acid Sequence
  source 1..372: mol_type = other DNA
caggtgcacctggtggagtctgggggaggctcggtgcagactggaggatctctgagactctcctgtgcagtctctggagacatctataacctcatgtcgatggcctggttccgccgggctccagggaaggagcgcgagggggtcgcatatattaatactattattggtaacacatactatactgactccgtgaagggccgattcaccatctcccgcgataactccaagaacactttgtatctgcaaatgaacaacctgaaacctgaggacacagccatgtactactgtgcggcgttcaattacggaggtgcctggtacgaggaacgcagctataaatactggggccaggggacccaggtcaccgtctcctca

SEQ ID NO: 388 - DNA, 375 bp, synthetic construct
  misc_feature 1..375: note = Camel sdAb AS64380 Nucleic Acid Sequence
  source 1..375: mol_type = other DNA
gaggtgcagctggtggagtctggggggggctcggtgcaggctggagggtctctgacactctcctgtgaagcctctggaaacacctacagtagtaattacatgggctggttccgccaggctccagggaaggagcgcgaggaggtcgcggttatttacactcgtggtggtcacacatactatgtcgactccgtgaggggccgattcaccatctcccaagacaacgccaagaacacggtgtatctgcaaatgaacagcctgaaacctgaggacactgccatgtactactgtgcggcgtcttcacgacatagactcggtttaaataacccacgggactatgactactggggccaggggacccaggtcaccgtctcctca

SEQ ID NO: 389 - DNA, 375 bp, synthetic construct
  misc_feature 1..375: note = Camel sdAb AS64395 Nucleic Acid Sequence
  source 1..375: mol_type = other DNA
caggtgaggttggtggagtctgggggaggctcggtgcaggctggagggtctctgagactctcctgtgctgcctctggatccacctacagtacaaacttcatgggctggttccgccaggctccagggaaggagcgcgagggggtcgcaacgcttgttacttgggctgaacgcacagcctatgccgactccgtgaagggccgattcaccatctcccaagaccgcgccaagaacacggtgtatctacaaatgaacggcctgaaacctgaggacactgccatgtactactgtgcggcagccgcttccactgctgtacgtctcctcgacccgggggactttgcttactggggccaggggacccaggtcaccgtctcctca

SEQ ID NO: 390 - DNA, 348 bp, synthetic construct
  misc_feature 1..348: note = Camel sdAb AS64443 Nucleic Acid Sequence
  source 1..348: mol_type = other DNA
caggtgcacctggtggagtctgggggaggctcggtgcaggctggagggtctctgagactctcctgtgcagcctctggatataccgacagtagcgtctacataggctggttccgccaggctccagggaaggagcgcgaggaggtcgcgattatttatactggtggtgaaagcacacactatcgcagctccgtgaagggccgattcaccgtctcccaagacaacgccaagaacacgctgtatctgcaaatgaacagcctgaaacctgaggacacggccatgtattactgtgcagcacgattcccagctgttacctactggggccaggggacccaggtcaccgtctcctca

SEQ ID NO: 391 - DNA, 375 bp, synthetic construct
  misc_feature 1..375: note = Camel sdAb AS64511 Nucleic Acid Sequence
  source 1..375: mol_type = other DNA
caggtgcagctggtggagtctgggggaggctcggtgcaggctggagggtctctgagactctcctgtgcagcctctagagccacctacagtaccaactacataagctggttccgccaggctccagggaaggagcgcgaggcggtcgcaacaattactactggtgatggtgagacagcgtatgccgactccgtgaagggccgattcaccatctcccgagacaacgccaagaacacggtctatctgcaaatgaacagcctgaaacctgaggacactgccatgtactactgtgcggcgaacttgcgaatcggtggcgactggttcgacggacgcgattttcgtgcctggggccaggggacccaggtcaccgtctcctca

SEQ ID NO: 392 - DNA, 375 bp, synthetic construct
  misc_feature 1..375: note = Camel sdAb AS64536 Nucleic Acid Sequence
  source 1..375: mol_type = other DNA
caggtgaagttggtggagtctgggggaggctcggtgcaggctggagggtctctgagactctcctgtgcagcctctagatacaccgacaatttcgtgtacatgggctggttccgccaggctccagggaaggagcgcgagggggtcgcactgatttatcctggtggtggtagcacctactatgcctcctccgtgaagggccgattcaccatctcccaagacaacgccaagggcacggtgcatctgcaaatgaacaacctgaaacctgaggacactgccatgtactactgtgcggcaaaatgggggctgggcggggggggcctgaaatcagatacgtatatgtactggggccaggggacccaggtcaccgtctcctca

SEQ ID NO: 393 - DNA, 387 bp, synthetic construct
  misc_feature 1..387: note = Camel sdAb AS64597 Nucleic Acid Sequence
  source 1..387: mol_type = other DNA
caggtgcacctggtggagtctgggggaggctcggtgcaggctggagggtctctgagactctcctgtgcagcctctggatacacctaccgtgtcaacttcatgggctggttccgccagactccagggaaggagcgcgagggggtcgcaactattgattctggtgtgggtaccacatactatgccgactccgtgaagggccgattcaccatctcccataacaacgccaagaacacgatttatctgcaaatgaacagcctgaaacctgaggacactgccatgtactactgtgcggcagggggcccccctacggacggtgatagatggtaccccctccgacctcctggttataactattggggccaggggacccaggtcaccgtctcctca

SEQ ID NO: 394 - DNA, 351 bp, synthetic construct
  misc_feature 1..351: note = Camel sdAb AS64617 Nucleic Acid Sequence
  source 1..351: mol_type = other DNA
caggtgcagctggtggagtctgggggaggctcggtgcaggctggagggtctctgagactctcctgtgcagcctctggatacactgatagatgcagcatggcctggtaccgccaggctccagggaaggagcgcgagttggtctcgcgtattagcacgagcggtttcacaaactacgcagcctccgtgaagggccgattcaccatctcccaagacaacgccaagaacacggtgtatctgcaaatgaacagcctgaaccccggggacacgggcatgtattactgtgccataatcgtaggacgtacttgtagtttgaactactggggcaacggcatcctggtcaccgtctcctca

SEQ ID NO: 395 - DNA, 381 bp, synthetic construct
  misc_feature 1..381: note = Camel sdAb AS64634 Nucleic Acid Sequence
  source 1..381: mol_type = other DNA
caggtgaggttggtggagtctgggggaggctcggtgcaggctggagggtctctgagactctcctgtgcagcctccggatacagttttagaggcgactttatgtgtatgggctggttccgccagactccagggaaggggcgcgagggggtcgcagttttttatcctggtggcggcagcacaaactatgccgactccgcgaagggccgattcaccatctcccaagacaacgccaagaacacgatgtatctgcaaatgaacaccctgaaacctgaggacactgccatgtactactgtgcggctcgacggtgggtcagtggtacctgctactgggatagtgactttcattactggggccaggggacccaggtcaccgtctcctca

SEQ ID NO: 396 - DNA, 375 bp, synthetic construct
  misc_feature 1..375: note = Camel sdAb AS69498 Nucleic Acid Sequence
  source 1..375: mol_type = other DNA
cagatgcagctggtggagtctgggggaggctcggtgcaggctggagggtctctgagactctcctgtgcagcctctggaaacacctacagtaccaattacatggcgtggttccgccaggctccagggaaggagcgcgaggaggtcgcggttatttacactcgtggtggtcacacctactatatcgactccgtgaggggccgattcaccatctcccaagacaacgccaagaacacggtgtatctgcaaataaacagcctgaaacctgaggacactgccatgtactactgtgcggcgtcttcacgaattagactccattgaatcgacccacgggactatcacgactggggccaggggacccaggtcaccgtctcctca

SEQ ID NO: 397 - DNA, 381 bp, synthetic construct
  misc_feature 1..381: note = Camel sdAb AS69500 Nucleic Acid Sequence
  source 1..381: mol_type = other DNA
caggtgaggttagtggagtctgggggaggctcggtgcaggctggagggtctctgagactctcctgtgcagccgacagatacacctacagtagcgcctgcatgggctggttccgccaggctccagggaaggagcgcgagggggtcgcctctatttttactggtactggtggtagcacatactatgccgactccgtgaagggccgattcaccatctcccaagacaacgccaagaacacggtgtatctgcaaatgaacagcctgaaacctgaggacactgccatatactactgtgcggcaagggccttccaggtcggttactgctacctgcgaaccgatgtgtataactactggggccaggggacccaggtcaccgtctcctca

SEQ ID NO: 398 - DNA, 375 bp, synthetic construct
  misc_feature 1..375: note = Camel sdAb AS69527 Nucleic Acid Sequence
  source 1..375: mol_type = other DNA
gaggtgcagctggcggagtctgggggaggctcggtccaggctggagggtctctgagactctcctgtgtagcctctagatacaccttcagtagcacctgcatggcctggttccgccaggctccagggaaggagcgcgaggaggtcgcagctatttatactgatgatggtagcacatggtatgccgactccgtgaagggccgattcaccatctccagagacaacgccaagaacacggtgtatctgcaaatgaacagcctgaaacctgaggacactgctatgtactactgtgcggcacgtaggtgggcgtgccccagggttggtagctggcatgagttcgcctactggggccaggggacccaggtcaccgtctcctca

SEQ ID NO: 399 - DNA, 375 bp, synthetic construct
  misc_feature 1..375: note = Camel sdAb AS68280 Nucleic Acid Sequence
  source 1..375: mol_type = other DNA
caggtgcaactggtggagtctgggggaggctcggtgcaccctggagggtctctgagactctcctgtgcagcctctggatccacctacagttccaactacctcggctggttccgccaggctccaggaaaggggcgcgactgggttgcggctattagcactggtgacggtgccacagcctatgccgactccgtgaagggccgattcaccatctcccaagacaacgccaagaacacggtgtatctgcaaatgaacagcttgaaacttgaggacagtgccatgtactactgtgcggcggctcgcggcagatttatcgattggacaaaggcaacccagtatgactactggggccaggggacccaggtcaccgtctcctca

SEQ ID NO: 400 - DNA, 384 bp, synthetic construct
  misc_feature 1..384: note = Camel sdAb AS68355 Nucleic Acid Sequence
  source 1..384: mol_type = other DNA
cagatgcagctggtggagtctgggggagactcggtgcaggctggagggtctctgagactctcctgtgcagcctctggatacacctacagcggcgtctgcatgggctggttccgccaggctccagggaaggagcgcgagggggtcgcagctattgatagtgatggtagcacaagctacgcagactccgtgaagggccgattcaccatctccaaagacaacgccaagaacactctgtatctgcaaatgaacagcctgaaacctgaggacactgccatgtactactgtgcggcagccattgtcgggggttttaatgcatattgtagtggtggttatgttctggactttggtgcctggggccaggggacccaggtcaccgtctcctca

SEQ ID NO: 401 - DNA, 396 bp, synthetic construct
  misc_feature 1..396: note = Camel sdAb AS69443 Nucleic Acid Sequence
  source 1..396: mol_type = other DNA
gaggtgcagctggcggagtctgggggaggctcggtgcaggctggagggtctctgagactctcctgttcagcctctggtttcacttttgatgattctgacatggcctggtaccgccaggctccaggggatgggtgcgacttggtctcaactattagtagtgatggtagcacatactatgcagactccgtgaagggccgattcaccatctcccaagacaacgccaagaacacggtgtatctgcaaatgcacagcctgaaacctgaggacacggccgtgtattactgtgcggcagatttcctcaccggcttttactatagcgactccccccatccggccccttgttctgcatccgactttggttactggggccaggggacccaggtcaccgtctcctca

SEQ ID NO: 402 - DNA, 378 bp, synthetic construct
  misc_feature 1..378: note = Camel sdAb AS75376 Nucleic Acid Sequence
  source 1..378: mol_type = other DNA
caggtgcaattgaaggagtctgggggaggctcggtgcaggctggagggtctctgagactctcctgtgcagcctctggatacacctacagtagccactccatgggctggttccgccaggctccagggaaggagcgcgagggggtcgcagttatttatactggtgatggtagcacatactatgccgactccgtgaagggccgattcaccatctcccaagacaacgccaagaacacggtgtatctgcaaatgaacagcctgaaacctgaggacactgccatgtactactgtgcggcagatccgaaccccgattatatgcttccgtttcggccgtcccgtaggtcgtggtggggccaggggacccaggtcaccgtctcctca

SEQ ID NO: 403 - DNA, 369 bp, synthetic construct
  misc_feature 1..369: note = Camel sdAb AS75387 Nucleic Acid Sequence
  source 1..369: mol_type = other DNA
caggtgcacctggtggagtctgggggaggctcggtgcaggctggagggtctctgagactctcctgtgcagcctctggatacccctacagtagcccctgcatggcctggtttcgccaggctccagggaaggagcgcgagggggttttagttgcttatactggtggggacattcaataccttaccgactccgtgaagggccgattcaccatctcccgagacaacgccaagaacacggtgtatctgcaaatgaacagcctgaaacctgaggacactgccatgtactactgtgcggcggatctgcgattacctcgtgccggcggttgtgcgtatagctactggggccaggggacccaggtcaccgtctcctca

SEQ ID NO: 404 - DNA, 363 bp, synthetic construct
  misc_feature 1..363: note = Camel sdAb AS75695 Nucleic Acid Sequence
  source 1..363: mol_type = other DNA
caggtgaggttggtggagtctgggggaggctcggtgcaggctggagggtctctgagactctcctgtgtagcctctggatacaccgtcagtgcctactgtatgggctggttccgccaggttctagggaaggggcgcgagaggatcgcatttatcgatgccgggggtgctacgatttacgcagaccccgtgaagggccgattcaccatctccaaagacaacgccaagaacactctgtatctgcaaatgaacagcctgaaacctgaggacactgccatgtactactgtgttgcagatcgccgggggcgggtacgtcggtgcgagtataacgcctggggccaggggacccaggtcaccgtctcctca

SEQ ID NO: 405 - DNA, 375 bp, synthetic construct
  misc_feature 1..375: note = Camel sdAb AS76169 Nucleic Acid Sequence
  source 1..375: mol_type = other DNA
caggtgcacctgatggagtctgggggaggctcggtgcaggctggagggtctctgagactctcctgtgcagcctctggatacatttacagtagcttctgcatgggctggttccgccaggctccagggaaggagcgcgaggtggtcgcgtatattcgcgataatattatgacaagttacacagactccgtgaagggccgattcaccatctccaaagacaacgccaagagaactctgtatctacaaatgaacggcctgaaacctgaagatactggcatgtactactgtgcggtagaccgggggggatacgctaatagttgcgcggtagcggcccggtatgattactggggccgggggacccaggtcaccgtctcctca

SEQ ID NO: 406 - DNA, 375 bp, synthetic construct
  misc_feature 1..375: note = Camel sdAb AS63931 Nucleic Acid Sequence
  source 1..375: mol_type = other DNA
gaggtgcagctggcggagtctgggggaggctcggtgcaggctggggggtctctgagactctcctgtgcaggctctttctctggatacggcgtcagtaccatggcctggttccgccaggctccagggaaggagcgcgagggggtcgcagctattactgttggtagtggaaacacatactatgccgactccgtgacgggccgattcaccatctcccgagacaacgccaagaggacggtgtatttgcaaatgaacagcctgaaacctgaggacactgccatgtactactgtgcggccggatggttgtcgggtggtagttggcacgttcccggcaggtataactactggggccaggggacccaggtcaccgtctcctca

SEQ ID NO: 407 - DNA, 369 bp, synthetic construct
  misc_feature 1..369: note = Camel sdAb AS63937 Nucleic Acid Sequence
  source 1..369: mol_type = other DNA
caggtgaagttagtggagtctgggggaggctcggtgcaggctggagggtctctgagactctcctgtgcagcctctggatccaccatcagtagtcgcccgatggcctggttccgccaggctccagggaaggagcgcgagggggtcgcgtgtatacatactggtcttggtagaacatactatgccgactccgtgaagggccgattcaccatctcccaagacaacgccaagaacacggtgtatctgcaagtgaacagcctgaaacctgaggacactgccatgtactactgtgcggcagactcgcggcggccgtgtatggtagccgcagggtatacctactggggccaggggacccaggtcaccgtctcctca

SEQ ID NO: 408 - DNA, 378 bp, synthetic construct
  misc_feature 1..378: note = Camel sdAb AS63948 Nucleic Acid Sequence
  source 1..378: mol_type = other DNA
caggtgcagctggtggagtctgggggaggctcggtgcaggctggagggtctctgagactctcctgtacagcctctggatacacctatagatacctctacatgggctggttccgccagactccagggaaggagcgcgagggggtcgcatgtatttatactggtagtggtagcacagggtatgccgactccgtgaagggccgattcaccatctcccaagacaacgccgagaacacggtgtatctgcaaatgaacagcctgaaacctgaggacactgccatgtactactgtgcggcagcttcgccccggtggggtggtacctgtcgacggtggtccgagtataactactggggccaggggacccaggtcaccgtctcctca

SEQ ID NO: 409 - DNA, 369 bp, synthetic construct
  misc_feature 1..369: note = Camel sdAb AS63956 Nucleic Acid Sequence
  source 1..369: mol_type = other DNA
caggtgcacctggtggagtctgggggaggcttggtgcaggctggagggtctctgagactctcctgtgcagcctccggattcacctacagtaactgctgcatgaggtggtaccgccaggctccagggaaggcgcgcgagttggtctcattaattaatagtagtggtggcacatactatgcagactctgtgaggggccgattcaccatctccaaagacaacgccaagaacacgctgtatctgcaaatgaacagcctgaaacctgaggacacggccatgtattactgtgcggcttaccaagccaagtactgttcaggcccttgcgcccccccaactgactggggccaggggacccaggtcaccgtctcctca

SEQ ID NO: 410 - DNA, 363 bp, synthetic construct
  misc_feature 1..363: note = Camel sdAb AS63965 Nucleic Acid Sequence
  source 1..363: mol_type = other DNA
caggtgcagctggtggagtctgggggaggctcggtgcaggctggagggtctctgagactctcctgtgtagcctctggatacagcagcggtagttgtcgcatgggctggtaccgccaggctccagggaaggagcgcgagttggtttcaaaggttattagtgatggtactacagtctatgcagactccgtgaagggccgattcaccctctcccaaggaaacgccaagaacacggtgtatctgcaaatgagtagcctgttacctgaggacacggccatgtattactgtaatgcatggtgtagggagtatcccggggggatcctgaataacggctggggccaggggacccaggtcaccgtctcctca

SEQ ID NO: 411 - DNA, 354 bp, synthetic construct
  misc_feature 1..354: note = Camel sdAb AS63993 Nucleic Acid Sequence
  source 1..354: mol_type = other DNA
caggtgaagttggtggagtctggggggggcttggtgcaggcaggggggtctctgagactctcctgtacagtttctggattcactttcgatgacctcgtcatggcctggttccgccaggctccagggaaggagcgccaacttgtctcgttggttgcgactgctggtaatagcgtctatgcagactccgtgaagggccgattcacactctccagagacaacgcccacagcacggcgtatctgcaaatgaacggcctgaaacctgaggacacggccatgtattactgtgcggcacgtaccgattctgagcatgcgtttaagttctggggtcaggggacccaggtcaccgtctcctca

SEQ ID NO: 412 - DNA, 348 bp, synthetic construct
  misc_feature 1..348: note = Camel sdAb AS63999 Nucleic Acid Sequence
  source 1..348: mol_type = other DNA
gaggtgcaactggtggagtctgggggaggctcggtgcaggctggagggtctctgagactctcctgtgcagcctctggatacacttacagtagcaactggatgggctggttccgccaggctccagggaaggagcgcgaggaggtcgcaattatttatactggtggtattagtacacactatcgcagctccgtgaagggccgattcaccatctcccaagacaacgccaagaacacggtgtatctgcaaatgaacagcctgaaacctgaggacactgccatgtactactgtgcggcgcgttatacagactataactactggggccaggggacccaggtcaccgtctcctca

SEQ ID NO: 413 - DNA, 348 bp, synthetic construct
  misc_feature 1..348: note = Camel sdAb AS64006 Nucleic Acid Sequence
  source 1..348: mol_type = other DNA
caggtgcacctggtggagtctgggggaggctcggtgcaggctggagggtctctgagactctcctgtgaagtctctggatacaccggcgatacgacttacataggctggttccgccaggctccagggaaggagcgcgagggggtcgcacttatttatactagtggtactagcgagtactacgccgactccgtgaagggccgattcatcatctcccgagacaacgccaagaacacggtgtatttacaaatgaacagcctgaaacctgaggacactgccatgtactactgtggcgcacggagccgcacgatgatgtactggggccaggggacccaggtcaccgtctcctca

SEQ ID NO: 414 - DNA, 378 bp, synthetic construct
  misc_feature 1..378: note = Camel sdAb AS64057 Nucleic Acid Sequence
  source 1..378: mol_type = other DNA
caggtgcaattggaggagtctgggggaggcttggtgcagacaggggggtctctgagactctcctgtacagcctctggattcacttttgatcgtaatgccatgcgctggtaccgccaggctccagggaaggagcgcgagggggtctcatgtattagttggacgggtgcaaatattgcctatgcagactccgtgaagggccgattcaccatctccagagacaacgccaagaacacgctgtatctgcaaatgaacagcctgaaacctgaggacacgggcatgtattactgtgcggcagatacgacgtcggggtcttgttcaggcttttggtctacgagccggtactactggggccaggggacccaggtcaccgtctcctca

SEQ ID NO: 415 - DNA, 366 bp, synthetic construct
  misc_feature 1..366: note = Camel sdAb AS64060 Nucleic Acid Sequence
  source 1..366: mol_type = other DNA
caggtgaagttagtggagtctgggggaggctcggtgcaggctggagggtctctgagactctcctgtgcagcctctggatccacctactgtacctaccgtatgagctggttccgccaggctccagggaaggagcgcgagttcgtcgcagttattgatagtggcggtagcacaagctacgcagactccgtgaagggccgattcaccatctcccgagacaacgccaagaacacggtgtatctgcaaatgaacagcctgaaacctgaggacacggccatgtattactgtaaaacagatccaaccatcggctgcccccagacatataggtataactactggggccaggggacccaggtcaccgtctcctca

SEQ ID NO: 416 - DNA, 375 bp, synthetic construct
  misc_feature 1..375: note = Camel sdAb AS64071 Nucleic Acid Sequence
  source 1..375: mol_type = other DNA
caggtgcacctgatggagtctgggggaggctcggtgcaggctggagggtctctgagactctcctgtgtagcctctggaaacacttacaggctcaactctatgggctggttccgccaggctccagggaaggagcgcgagggggtcgcatttattgttatgattagaggtaccacatactatggcgcctccgtaaagggccgattcaccatctcccaagacaacgcccagaccacggtgtatctgcaaatgagcagcctgaaaccggaggacactgccatgtactactgtgcggcatccactaaggaccagttttatgtatttaatcctattgggtatgactcttggggccaggggacccaggtcaccgtctcctca

SEQ ID NO: 417 - DNA, 390 bp, synthetic construct
  misc_feature 1..390: note = Camel sdAb AS64093 Nucleic Acid Sequence
  source 1..390: mol_type = other DNA
caggtgcacctggtggagtctgggggaggctcggtgcaggctggagggtctctgagactctcctgtgcaacctctagatacatctacggtaacaactgcatggcctggttccgccaggctccagggaaggagcgcgagggagtcgcgtctatttatcctgctggtggtcgcacgtactatgccgactccgtgaagggccgattcaccatctcccaagacaacgccaagaacacggtgtatctgcaaattgacagcctgaaacctgaggacacggccatgtactactgcgcggcacgctctttttcgataggagtttgcgcgacgcagtctggtattacctggtctaattttgcttactggggccaggggacccaggtcaccgtctcctca

SEQ ID NO: 418 - DNA, 351 bp, synthetic construct
  misc_feature 1..351: note = Camel sdAb AS64118 Nucleic Acid Sequence
  source 1..351: mol_type = other DNA
caggtgcaactggcggagtctgggggaggctcggtgcaggctggagggtctctgagactctcctgtgcagcctctggatacacctacagtgcctgtagaatggcctggtaccgccaggctcccgggaaggagcgcgagttggtttcatttattaatagtgctggtagcacatactatgccgactccgtgaagggccgattcgccatctcccgagacaacgccaagacaacggtgtatctacaaatgaacgccctgaaagctgaggacacggccatatattactgtaacacatgggatagtagctgccgctttcagtactggggccaggggacccaggtcaccgtctcctca

SEQ ID NO: 419 - DNA, 404 bp, synthetic construct
  misc_feature 1..404: note = Camel sdAb AS64120 Nucleic Acid Sequence
  source 1..404: mol_type = other DNA
caggtgaggttggtggagtctgggggaggctcggtgcaggctggagggtctctgagactctcctgtgaaacctctagatacatctacggtaacaactgcatggcctggttccgccaggctccagggaaggagcgcgagggagtcgcgtctatttatcctgctggtggtcgcccgtactatgccgactccgtgaagggccgattcaccatctcccaaagacaacgccaagaacacggtgtatctgcaaaatggacagccctgaaaacctgaggacacggcccatgtactactgcgcgggcacgcttcttttttcgatagcaaattgcgccaacgcaatcctggtattaaccagggccaaattttggcttacgggggccaggggacccaggtcacccttctcctca

SEQ ID NO: 420 - DNA, 384 bp, synthetic construct
  misc_feature 1..384: note = Camel sdAb AS64124 Nucleic Acid Sequence
  source 1..384: mol_type = other DNA
caggtgaagttggtggagtctgggggaggctcggtgcagactggagggtctctgagactctcctgtgcagtctctacgtacacccccagtaacaactacatgggctggttccgccaggctccagggaaggagcgcgagggcgtcgcggctatcgctactattggtggtaccacacgttatgccgactccgtgaagggccgattcaccatctcccaagacggcgccaagaacacgatatatctgcaaatgaacggcctgaaaccggaggacactgccatgtactactgtgcggccgggcggccatactcattacccttacccttacccttggaaagcggtgcgtatcgctactggggccaggggacccaggtcaccgtctcctca

SEQ ID NO: 421 - DNA, 363 bp, synthetic construct
  misc_feature 1..363: note = Camel sdAb AS64135 Nucleic Acid Sequence
  source 1..363: mol_type = other DNA
caggtgaagttggtggagtctgggggaggctcggtgcaggctggagggtctctgagactctcctgtgtagcctctacatcaacctactgtaggtactacatgcgctggtaccggcaggctccagggaaagagcgcgagttcgtctcagcgatgcaacccgatggtacgacaagctactcagactccgtgaagggccgattcaccatgtcccaagacagagccaacaatatgttgtatctgcaaatgaacagcctgaggcctgaggacacggccatgtattactgtaaaagagatccaatggggggttcaaggaccccgtgcacctccgcctggggccaggggacccaggtcaccgtctcctca

SEQ ID NO: 422 - DNA, 375 bp, synthetic construct
  misc_feature 1..375: note = Camel sdAb AS64163 Nucleic Acid Sequence
  source 1..375: mol_type = other DNA
caggtgaggttggtggagtctgggggaggctcggtgcaggctggagggtctctgagactctcctgtgcagtctctggatacagatatagatggaactgcatggcctggttccgccaggctccagggaaggagcgcgagggggtcgcagctatttctactggaagcggaagcacatactatgccggctccgtgaagggccgattcaccatctcccaagacaacgccaagaacatgtatctgcaaatgaacagcctgaaacctgaggacactgccatgtactactgtgcggcagatccttcggtttgccccggtggtatgtggtactccaaagagtataggtactggggccaggggacccaggtcaccgtctcctca

SEQ ID NO: 423 - DNA, 378 bp, synthetic construct
  misc_feature 1..378: note = Camel sdAb AS64182 Nucleic Acid Sequence
  source 1..378: mol_type = other DNA
caggtgcacctgatggagtctgggggaggctcggtgcaggctggagggtctctgagactctcctgcacagcctctggacagacctccagatacctctacatgggctggtttcgccagactccagggaaggagcgcgagggggtcgcatgtatttatactggtagtggtagcacagggtatgccgactccgtgaagggccgattcaccatctcccaagacaacgccaagaacacggtgtatctgcaaacgaatagcctgaaacctgaggacactgccatgtactactgtgcggcaagttcgccccattggggcggtacctgtcgacgctggtccgagtataagtactggggccaggggacccaggtcaccgtctcctca

SEQ ID NO: 424 - DNA, 366 bp, synthetic construct
  misc_feature 1..366: note = Camel sdAb AS64183 Nucleic Acid Sequence
  source 1..366: mol_type = other DNA
caggtgcacctggtggagtctgggggaggctcggtgcaggctggagggtctctgagactctcctgtgcagcctctggacacacctacagtgccaactgcatggcctggttccgccgggccccagggaaggagcgcgagtgggtcgcgtcggtttatactgatgatgatagcacaatgtataccgactccgtgaagggccgattcaccatcttccaagacaacgccaagaacacggtgtatctgcaaatgaacagcctgaaacctgaggacactggcatgtacatctgtgcggcagatttaagcggaggaccggccggttgtgggtatacccactggggccaggggacccaggtcaccgtctcctca

SEQ ID NO: 425 - DNA, 387 bp, synthetic construct
  misc_feature 1..387: note = Camel sdAb AS64207 Nucleic Acid Sequence
  source 1..387: mol_type = other DNA
gaggtgcagctggtggagtctgggggaggctcggtgcaggctggagggtctctgagactctcctgtgcagcctctggatacacctacagtagcaacttcatgggctggttccgccaggctccagggaaggagcgcgagggggtcgcaactattgtttctggtggtggtaccacatactatgccgactccgtgaggggccgattcaccatctcccaagacaacgccaagaacacggtgtatctgcaaatgaacagcctgaaacctgaggacactgccatgtactactgtgcggcagggggcccccctacgaacggtgctaagtggtaccccctccgacctcctggttataactactggggccaggggacccaggtcaccgtctcctca

SEQ ID NO: 426 - DNA, 366 bp, synthetic construct
  misc_feature 1..366: note = Camel sdAb AS64276 Nucleic Acid Sequence
  source 1..366: mol_type = other DNA
caggtgcacctgatggagtctgggggaggctcggtgcaggctggagggtctctgagcctctcctgtgtagtctctggatacaccggcagtagccgctgtatggcctggttccgccaggctccagggaaggagcgcgaggcggtcgcacaaatttttactggtcgtggtaccacaggctatgccgactccgtgaagggccgattcactatttcccaagacaacgccaagaacacggtgtatctgcgaatgaacagtctgagacctgaggacactgccatttactactgtgcggcgagtctcggcccgggacgcggagcctgtgggtataactactggggccaggggacccaggtcaccgtctcctca

SEQ ID NO: 427 - DNA, 363 bp, synthetic construct
  misc_feature 1..363: note = Camel sdAb AS64336 Nucleic Acid Sequence
  source 1..363: mol_type = other DNA
caggtgcagctggtggagtctgggggaggctcggtgcaggctggagggtctctaagactctcctgtacaacctctggacgcacctacagtagctgcagcatgggctggtaccgccaggctccagggaaggagcgcgagttggtctcacatatttttagtgatggtagcagatactatgcagactccgtgaagggccgattcaccatctcccaagacaacgccaagaacacggtgtatctgcaaatgaacagcctgaaacctgaggacacggccatgtattactgtaaccgccgtacgggttgggcaccaaggtgcgctgttcccggttactggggccaggggacccaggtcaccgtctcctca

SEQ ID NO: 428 - DNA, 381 bp, synthetic construct
  misc_feature 1..381: note = Camel sdAb AS64346 Nucleic Acid Sequence
  source 1..381: mol_type = other DNA
caggtgcacctggtggagtctgggggaggctcggtgcaggctggagggtctctgagactctcctgtgcagcctctggatacacctatttcatgggctggttccgccaggctccacagaaggagcgcgaatgggtcgcgactattggtactggtgatattttcaatggcgctgcttactatgtcgactccgtgaagggccgattcgccatctcccaagacaacgccaagaacacggtgtatctgcaaatgaacagcctgaaacctgaagacactgccgtgtacgtctgtgcggcagttcaatcgaaatcctcaaactacgtgttgagagacgcatctacctacaactactggggccaggggacccaggtcaccgtctcctca

SEQ ID NO: 429 - DNA, 348 bp, synthetic construct
  misc_feature 1..348: note = Camel sdAb AS64420 Nucleic Acid Sequence
  source 1..348: mol_type = other DNA
gaggtgcagctggtggagtctgggggaggctcggtgcaggctgaagggtctctgagactctcctgtgcagcctctggagacaccagtagaagcgtctggatgggctgggcccgccaggttccagggaaagagcgcgaggtggtcgcaaccattagtactgccggtggtagtacatggtataccgactccgtgaagggccgattcaccatctcccaagacaacgccaagaacacggtgtacctgcaaatgaacagcctgaaacctgaggacactgccatatactattgtgcggccagaagcagatatgctacctactggggccaggggacccaggtcaccgtctcctca

SEQ ID NO: 430 - DNA, 378 bp, synthetic construct
  misc_feature 1..378: note = Camel sdAb AS64473 Nucleic Acid Sequence
  source 1..378: mol_type = other DNA
caggtgaggttggtggagtctgggggaggctcggtgcaggctggagggtctctgagactctcctgtacagcctctggatacacctacagatacctctacatggcctggttccgccagactccagggaaggagcgcgagggggtcgcatgtatttatactggtagtggtaccacagggtatgccgactccgtgaagggccgattcaccatctcccaagacaacgccaagaatacggtgtatctgcaaatgaacagcctgaacgctgaggacactgccatgtactactgtgcggcaagttcgccccagtggggcggtacctgtcgacgctggtccgagtataactactggggccaggggacccaggtcaccgtctcctca

SEQ ID NO: 431 - DNA, 348 bp, synthetic construct
  misc_feature 1..348: note = Camel sdAb AS64475 Nucleic Acid Sequence
  source 1..348: mol_type = other DNA
caggtgcaactgcaggagtctgggggaggctcggtgcaggctggagggtctctgagactctcctgtgcagcctctggatacacctggagtcgcaactggatgggctggttccgccaggctccagggaaggagcgcgaggggttcgcaactattacaattagtggtggtagcacatggtatgccgactccgtgaagggccgattcaccatctccctagacaacgccgggaacacggtgtatctgcaaatgaacagcctgaaacctgaggacactgccatgtactactgtgcggcgcgggataccgcgcggacctactggggccagggtacccaggtcaccgtctcctca

SEQ ID NO: 432 - DNA, 381 bp, synthetic construct
  misc_feature 1..381: note = Camel sdAb AS64513 Nucleic Acid Sequence
  source 1..381: mol_type = other DNA
gaggtgcagctggtggaatctgggggaggctcggtgcaggctggagggtctctgagactctcctgtgtagcctctgactacccctacatagacaactgcatgggctggttccgccagggtccagggaaggagcgcgagggggtcgcagctgcgtgtactggtggtggtagcacatattatgccgactccgtgaagggccgattcaccatctcccgagacaacgccaagaacacggtgtatctgcaaatgaacagcctgaaacctgaggacactgacgtgtactactgtgcgacaggctactatagcggctctggtccggggtatttactcccatggaggtataactactggggccaggggacccaggtcaccgtctcctca

SEQ ID NO: 433 - DNA, 393 bp, synthetic construct
  misc_feature 1..393: note = Camel sdAb AS64562 Nucleic Acid Sequence
  source 1..393: mol_type = other DNA
gaggtgcaactggtggaatctgggggaggctcggtgcaggctggagggtctctgagactctcctgtgcagcctctggatacaccgctaggcgcgacttcatggcctggttccgccaggttccagggaaggagcgcgagggggtcgcagtcattcatactggtggtgacaccacatactatgccgactccgtgaagggccgattcaccatctcccgcgacaacgcccagaacataatgaatctgcaaatgaacagccttaaacctgaggacactgccatgtactactgtgcggcaggtttccgtccgcgtggtggaggatacacgggtgacgtcttggcccaggctgcggcatacaactactggggccaggggacccaggtcaccgtctcctca

SEQ ID NO: 434 - DNA, 378 bp, synthetic construct
  misc_feature 1..378: note = Camel sdAb AS64583 Nucleic Acid Sequence
  source 1..378: mol_type = other DNA
gaggtgcagctggcggagtctgggggaggcttggtgcaggcaggggggtctctgagactctcctgtacagcctctggattcactattgctgtttataccatgggctggttccgccaggctccagggaaggagcgcgagggaatctcatgtactagctgggctggtggtcgcacatacactgcagactccgtgaagggccgattcaccatctccagagacaacgccaagaacacgctgtatctgcaaatgaacagcctgaaacctgaggacacggccatgtattactgtgcggcaaaggcacatcccgactgttcaggggattggtccccatctgggtatgaatactggggccaggggacccaggtcaccgtctcctca

SEQ ID NO: 435 - DNA, 348 bp, synthetic construct
  misc_feature 1..348: note = Camel sdAb AS64594 Nucleic Acid Sequence
  source 1..348: mol_type = other DNA
caggtgcacctggtggagtctgggggaggctcggtgcaggctggagggtctctgagactctcctgtgcagcctctggatacacctacaatagcaactacatgggctggttccgccaggctccagggaaggagcgcgagggggtcgcacttatttatactggtggtggtagcacatattatgccgactccgtgaagggccgattcaccatctcccgagacaacgccaaaaacacggtgtatctgcaaatgaacagcctgaaacctgaggacactgccatgtactactgttcggtaagaacgcagacgcgtaactactggggccaggggacccaggtcaccgtctcctca

SEQ ID NO: 436 - DNA, 393 bp, synthetic construct
  misc_feature 1..393: note = Camel sdAb AS64605 Nucleic Acid Sequence
  source 1..393: mol_type = other DNA
caggtgaagttggtggagtctgggggaggctcggtgcaggctggagggtctctgagactctcctgtgcagtttctagatatccctacagcagcatctgcatgggctggttccgccaggctccagggaaggagagcgagggtgtcgcacgtatttatactggtactggtagtacatggtataccgactccgtgaagggccgattcaccatcgcccgagacaacgcccagaacacggtgtatctgcaaatgaacagcctgaaacctgaggacactgccatgtactactgtgcggcgcgtagcaattcatattcatattcaagttgtgattacggccccctcacgaggggggggtataacttctggggccaggggacccaggtcaccgtctcctca

SEQ ID NO: 437 - DNA, 345 bp, synthetic construct
  misc_feature 1..345: note = Camel sdAb AS64606 Nucleic Acid Sequence
  source 1..345: mol_type = other DNA
gaggtgcagctggcggagtctgggggaggatcggtgcaggctggagggtctctgagactctcctgtgcagtctctggatacaccagccgtagcaattacatgggctggttccgccaggctccagggaaggagcgcgagggggtcgcgctaatttatactcgtggtggtagcacatactatgcctcctccgtgaagggccggttcaccatctcccaagacagtgccaagaaaacgtatctgcaaatgaacagtgtgaaaccggaggacactgccatgtactactgtgctttgcgccttgatgagaagatgtactggggccaggggacccaggtcaccgtctcctca

SEQ ID NO: 438 - DNA, 399 bp, synthetic construct
  misc_feature 1..399: note = Camel sdAb AS68121 Nucleic Acid Sequence
  source 1..399: mol_type = other DNA
gaggtgcagctggcggagtctgggggaggctcggtgcaggctggagggtctctgagactctcctgtgatgcctctggatacacctacagccgcaactgcatgggctggttccgccaggctccagggaaggagcgcgagggggtcgcagcgttctatactgattatattcgttttgggcgcacatattatgccgactccgtgaagggccgattcaccatcttccaagacaacgccaagaacacggtgtatctgcaaatgaacagcctgaaacctgaggacactgccatgtactactgtgcggcagatcctgggagtcgtacagacgatagttgtggtacctcatacaacaaagggaattttggttactggggccaggggacccaggtcaccgtctcctca

SEQ ID NO: 439 - DNA, 390 bp, synthetic construct
  misc_feature 1..390: note = Camel sdAb AS68170 Nucleic Acid Sequence
  source 1..390: mol_type = other DNA
caggtgcagctggtggagtctgggggaggctcggtgcaggctggagggtcgctgagactctcctgtacagcctctggatacacctacagaagcaactgtatgggctggttccgccaggctccagggaaggagcgcgagggggtcgcaacaatctatactggtggtggtcgtaatctatactatgccgactccgtgaagggccgattcaccatctcccgagacaacgccaagaacaccctgtacctgcaaatgaacagcctgaagcctgaggactctgccaggtactactgtgcggccgcgagtgacgtggcagttggtgttaattcctgcgggggaaggactgcggggtttgacgcctggggccaggggacccaggtcaccgtctcctca

SEQ ID NO: 440 - DNA, 375 bp, synthetic construct
  misc_feature 1..375: note = Camel sdAb AS63964 Nucleic Acid Sequence
  source 1..375: mol_type = other DNA
caggtgaggttagtggagtctgggggaggatcggtacaggctggagggtctctgagactctcctgctcagcctctggatacacctacagttacaacaatatgggctggttccgccaggctccagggaacgagcgcgagggggtcgcagctattagtggtggtcgtttcaccgcctatgccgactccgtgaagggccgattcaccatctcccgagacaacgccgagaacacgctgtatctgcaaatgaacaacctgaaacctgaggacactgggatgtactactgtgcggcagaggtagttgatccgacctgggggtcgcgtgaccaaagacgatataagtactggggccaggggacccaggtcaccgtctcctca

SEQ ID NO: 441 - DNA, 372 bp, synthetic construct
  misc_feature 1..372: note = Camel sdAb AS64116 Nucleic Acid Sequence
  source 1..372: mol_type = other DNA
caggtgaagttggtggagtctgggggaggctcggtgcaggctggagggtctctgagactctcgtgtgcagcctctggatacatctacagttgcgtgggctggttccgccaggctccagggaaggagcgcgagggggtcgcaggtattagtactggtggtggtggcacagtctatgccgactccgtgaagggccaattcaccatctcccgagacaacgccaagaacacggtgtacctgcaaatggacagcctgaaacctgaggacactgccatgtactactgtgcggcagatcgatggaattcattcgctaattgcggtgcctggggaaggtatacctactggggccaggggacccaggtcaccgtctcctca

SEQ ID NO: 442 - DNA, 390 bp, synthetic construct
  misc_feature 1..390: note = Camel sdAb AS68270 Nucleic Acid Sequence
  source 1..390: mol_type = other DNA
caggtgcaactggcggagtctgggggaggctcggtgcaggctggagggtctctgagactctcctgtgtagcctctggatacccctcttccacctactacatgctcagcatggcgtggttccgccaggctccagggaaggagcgcgagggggtcgccgctattactagcggtactgggagcacaagctacgcagactccgtgaaggaccgattcaccatctccaaagactacgccaacaacactctgtatctgcacataaacaacctgaaacctgaggacactgccatgtactactgtgcggcagcctcaggttggatcgttcctagtaggtccctgaccgccaacctatataggtattggggccaggggacccaggtcaccgtctcctca

SEQ ID NO: 443 - DNA, 375 bp, synthetic construct
  misc_feature 1..375: note = Camel sdAb AS68320 Nucleic Acid Sequence
  source 1..375: mol_type = other DNA
caggtgcacctggtggagtctgggggagactcggtgcaggctggagggtccctgagactctcctgtgcagcctctggatacacctacaataccaactacatgggctggttccgccaggctccagggaaggagcgcgagggggtcgcagctatttatagacatagtggtaacacagcctatgccgactccgtgaagggccgattcaccatctcccaagactacgccaagaacaccgtgtatctgcaaatgaacagcctgaaacctgaggacactgccatgtactactgtgcggcagggcgcgctggtccctgggccctgatgcgcccgactgagtttggttactggggccaggggacccaggtcaccgtctcctca

SEQ ID NO: 444 - DNA, 369 bp, synthetic construct
  misc_feature 1..369: note = Camel sdAb AS68351 Nucleic Acid Sequence
  source 1..369: mol_type = other DNA
caggtgcaattggaggagtctgggggaggcttggtgcagcctggggggtctctgagactctcctgtgcggcctctggagacacatttcgtgcctattacatgaactgggtccgccaggctccagggaagggattcgagtgggtctcaggtattagcgccagtggcggccgtacgtcatacgcagactccgtgaagggccgattcaccatctccagagacaacgccaaaaacacgctgtatctgcaattgaacagcctgagcactgaggacacgggcatgtattattgtgtaaagggagctgtccgtctctcgacatcgtcagtacgggattcgtcctggggccaggggacccaggtcaccgtctcctca

SEQ ID NO: 445 - DNA, 348 bp, synthetic construct
  misc_feature 1..348: note = Camel sdAb AS75378 Nucleic Acid Sequence
  source 1..348: mol_type = other DNA
caggtgcaattggaggagtctgggggaggctcggtgcaggctggagggtctctgagactctcctgtgtagtctctggaaacacccgcagtaccacgtacatgggctggttccgccaggctccagggaaggagcgcgagggggtcgcaatagtttatactggtggtcgtgacacatactatgccgcctccgtgaagggccgattcaccatctcccaagacaacgccaagacaacgatctatctgcaaatgaacagtctggaacctgaggacactgccatgtactactgtgcggcacgctcatatgagtatacctactggggtcgggggacccaggtcaccgtctcctca

SEQ ID NO: 446 - DNA, 372 bp, synthetic construct
  misc_feature 1..372: note = Camel sdAb AS75383 Nucleic Acid Sequence
  source 1..372: mol_type = other DNA
gaggtgcaactggcggagtctgggggaggctcggtgcaggctggagggtctctgagactctcctgtgtagcctctggatacaccttcagtagctactgcttgggctggttccgccaggctccagggaagcagcgccagggggtcgcaacgtttaataatagaggtgtcgcaaactaccacgattccgtgaagggccgattcaccgcctccgtagacaacgccaagaacactctgcttctgcaaatgaacagcctggaacctgacgacacggccatgtactactgtgcggcggatcgccggtacggtcgtcagtggtatcagccttgcgagtggaacacctggggccaggggacccaggtcaccgtctcctca

SEQ ID NO: 447 - DNA, 387 bp, synthetic construct
  misc_feature 1..387: note = Camel sdAb AS75751 Nucleic Acid Sequence
  source 1..387: mol_type = other DNA
caggtgaggttggtggagtctgggggaggctcggtgcaggctggagggtctctgagactctcctgtgtagcctctggatacttctacaatacctactactttatgggctggttccgccaggctccagggaaggagcgcgagggggtcgcagctattgatactgatggtagaacaagttacgcagactccgtgaagggccgattcaccatctccaaagacaacgccaagaacactctgtatctgcaaatgaacagcctgaaacctgaggacactgccatgtactactgtgcggcaggttttggctatatgaatgttattcaggctcttaatggcatgagacagaatcccgactactggggccaggggacccaggtcaccgtctcctca

SEQ ID NO: 448 - DNA, 372 bp, synthetic construct
  misc_feature 1..372: note = Camel sdAb AS76422 Nucleic Acid Sequence
  source 1..372: mol_type = other DNA
caggtgaagttggtggagtctgggggaggctcggtgcaggctggagggtctctgagactctcctgtgcagcctctggatacaccttcgctggcaactgcttgggctggtttcgccaggctccagggaaggggcgcgagggggtcgtaacgtacaataacttcggtgtcgccaactacgccgattccgtgaagggccgattcaccgtctcccaagacaacgccaagaacactctgcttctgcaaatgaacagcctggaacctgaggacactgccatgtactactgtgcggcggaccgccgggacggtcgtcgctggtctcagccttgcgagtggaatacctggggccaggggacccaggtcaccgtctcctca

SEQ ID NO: 449 - DNA, 375 bp, synthetic construct
  misc_feature 1..375: note = Humanized sdAb AS64380VH4 Nucleic Acid Sequence
  source 1..375: mol_type = other DNA
gaggtgcagctggtggagagcggaggaggactggtgcagccaggaggcagcctgaggctgtcctgcgcagcatctggaaacacctacagctccaattatatgggatggttcaggcaggcacctggcaagggactggaggaggtggccgtgatctacaccaggggaggacacacatactatgtggactccgtgcggggacggttcaccatcagcagggataacgccaagaacagcctgtatctgcagatgaactctctgagagccgaggacacagccgtgtactattgtgcagcatctagcaggcacaggctgggcctgaacaatccaagggactacgattattggggccagggcaccctggtgacagtgtcctct

SEQ ID NO: 450 - DNA, 375 bp, synthetic construct
  misc_feature 1..375: note = Humanized sdAb AS64380VH5 Nucleic Acid Sequence
  source 1..375: mol_type = other DNA
gaggtgcagctggtggagagcggaggaggactggtgcagccaggaggcagcctgaggctgtcctgcgcagcatctggaaacacctacagctccaattatatgggatggttcaggcaggcacctggcaagggcctggaggaggtggccgtgatctacaccagaggcggccacacatactatgtggactccgtgcggggacggttcaccatcagccaggataacgccaagaacagcctgtatctgcagatgaactctctgagggccgaggacacagccgtgtactattgtgcagcatctagcaggcacaggctgggcctgaacaatccaagggactacgattattggggccagggcaccctggtgacagtgtcctct

SEQ ID NO: 451 - DNA, 375 bp, synthetic construct
  misc_feature 1..375: note = Humanized sdAb AS64380VH6 Nucleic Acid Sequence
  source 1..375: mol_type = other DNA
gaggtgcagctggtggagagcggaggaggactggtgcagccaggaggcagcctgaggctgtcctgcgcagcatctggaaacacctacagctccaattatatgggatggttcaggcaggcacctggcaagggcctggaggaggtggccgtgatctacaccagaggcggccacacatactatgtggactccgtgcggggacggttcaccatcagccaggataacgccaagaacagcgtgtatctgcagatgaactctctgagggccgaggacacagccatgtactattgtgcagcatctagcaggcacaggctgggcctgaacaatccaagggactacgattattggggccagggcaccctggtgacagtgtcctct

SEQ ID NO: 452 - DNA, 375 bp, synthetic construct
  misc_feature 1..375: note = Humanized sdAb AS64380VH7 Nucleic Acid Sequence
  source 1..375: mol_type = other DNA
gaggtgcagctggtggagagcggaggaggactggtgcagccaggaggcagcctgaggctgtcctgcgcagcatctggaaacacctacagctccaattatatgggatggttcaggcaggcacctggcaagggaagagaggaggtggccgtgatctacaccaggggaggacacacatactatgtggactccgtgcggggacggttcaccatcagccaggataacgccaagaacagcgtgtatctgcagatgaactctctgagggccgaggacacagccatgtactattgtgcagcatctagcaggcacaggctgggcctgaacaatccaagggactacgattattggggccagggcaccctggtgacagtgtcctct

SEQ ID NO: 453 - DNA, 375 bp, synthetic construct
  misc_feature 1..375: note = Humanized sdAb AS64511VH4 Nucleic Acid Sequence
  source 1..375: mol_type = other DNA
gaggtgcagctggtggagtccggaggaggactggtgcagccaggaggctctctgaggctgagctgcgcagcatccagagcaacctactctacaaactatatcagctggttcaggcaggcacctggcaagggactggaggcagtggcaaccatcaccacaggcgatggcgagacagcctacgccgactctgtgaagggcaggtttaccatctcccgcgataacgccaagaacagcctgtatctgcagatgaacagcctgagggccgaggacacagccgtgtactattgtgcagcaaatctgaggatcggaggcgactggttcgatggaagggactttagagcatggggacagggaaccctggtgacagtgagctcc

SEQ ID NO: 454 - DNA, 375 bp, synthetic construct
  misc_feature 1..375: note = Humanized sdAb AS64511VH5 Nucleic Acid Sequence
  source 1..375: mol_type = other DNA
gaggtgcagctggtggagtccggaggaggactggtgcagccaggaggctctctgaggctgagctgcgcagcatccagagcaacctactctacaaactatatcagctggttcaggcaggcacctggcaagggactggaggcagtggcaaccatcaccacaggcgatggcgagacagcctacgccgactctgtgaagggcaggtttaccatctcccgcgataacgccaagaacagcgtgtatctgcagatgaacagcctgagggccgaggacacagccatgtactattgtgcagcaaatctgaggatcggaggcgactggttcgatggaagggactttagagcatggggacagggaaccctggtgacagtgagctcc

SEQ ID NO: 455 - DNA, 375 bp, synthetic construct
  misc_feature 1..375: note = Humanized sdAb AS64511VH6 Nucleic Acid Sequence
  source 1..375: mol_type = other DNA
gaggtgcagctggtggagtccggaggaggactggtgcagccaggaggctctctgaggctgagctgcgcagcatccagagcaacctactctacaaactatatcagctggttcaggcaggcacctggcaagggaagggaggcagtggccaccatcaccacaggcgatggcgagacagcctacgccgactctgtgaagggcaggtttaccatctcccgcgataacgccaagaacagcgtgtatctgcagatgaacagcctgcgggccgaggacacagccatgtactattgtgcagcaaatctgaggatcggaggcgactggttcgatggaagggactttagagcatggggacagggaaccctggtgacagtgagctcc

SEQ ID NO: 456 - DNA, 375 bp, synthetic construct
  misc_feature 1..375: note = Humanized sdAb AS63931VH4 Nucleic Acid Sequence
  source 1..375: mol_type = other DNA
caggtgcagctggtggagagcggaggaggagtggtgcagccaggaggcagcctgaggctgtcctgcgcaggctctttcagcggatacggcgtgtccaccatggcatggtttaggcaggcacctggcaagggactggagggagtggcagcaatcaccgtgggatccggaaacacatactatgccgactctgtgaccggccggttcacaatctctagagataacagcaagaataccctgtatctgcagatgaacagcctgcgggccgaggacacagccgtgtactattgtgcagcaggatggctgtccggaggatcttggcacgtgcccggcaggtacaactattggggccagggcaccctggtgacagtgagctcc

SEQ ID NO: 457 - DNA, 375 bp, synthetic construct
  misc_feature 1..375: note = Humanized sdAb AS63931VH5 Nucleic Acid Sequence
  source 1..375: mol_type = other DNA
caggtgcagctggtggagagcggaggaggagtggtgcagccaggaggcagcctgaggctgtcctgcgcaggctctttcagcggatacggcgtgtccaccatggcatggtttaggcaggcacctggcaagggactggagggagtggcagcaatcaccgtgggatccggaaacacatactatgccgactctgtgaccggccggttcacaatctctagagataacagcaagaataccgtgtatctgcagatgaacagcctgcgggccgaggacacagccatgtactattgtgcagcaggatggctgtccggaggatcttggcacgtgcccggcaggtacaactattggggccagggcaccctggtgacagtgagctcc

SEQ ID NO: 458 - DNA, 375 bp, synthetic construct
  misc_feature 1..375: note = Humanized sdAb AS63931VH6 Nucleic Acid Sequence
  source 1..375: mol_type = other DNA
caggtgcagctggtggagagcggaggaggagtggtgcagccaggaggcagcctgaggctgtcctgcgcaggctctttcagcggatacggcgtgtccaccatggcctggtttaggcaggcacctggcaagggaagggagggagtggcagcaatcaccgtgggatccggaaacacatactatgccgactctgtgaccggccggttcacaatctctagagataacagcaagaataccgtgtatctgcagatgaacagcctgcgggccgaggacacagccatgtactattgtgcagcaggatggctgtccggaggatcttggcacgtgcccggcaggtacaactattggggccagggcaccctggtgacagtgagctcc

SEQ ID NO: 459 - DNA, 375 bp, synthetic construct
  misc_feature 1..375: note = Humanized sdAb AS63997VH4 Nucleic Acid Sequence
  source 1..375: mol_type = other DNA
caggtgcagctggtggagagcggaggaggagtggtgcagccaggaggcagcctgaggctgtcctgcgcagcctctttcagcggatacggcgtgtccaccatggcatggtttaggcaggcacctggcaagggactggagggagtggcagcaatcaccgtgggatccggaaacacatactatgccgactctgtgaagggccggttcaccatctctagagataacagcaagaatacactgtacctgcagatgaacagcctgcgggccgaggacacagccgtgtactattgtgccgtgggctatctgtccggaggatcttgggatgtgccaggaaggtacaactattggggccagggcaccctggtgacagtgagctcc

SEQ ID NO: 460 - DNA, 375 bp, synthetic construct
  misc_feature 1..375: note = Humanized sdAb AS63997VH5 Nucleic Acid Sequence
  source 1..375: mol_type = other DNA
caggtgcagctggtggagagcggaggaggagtggtgcagccaggaggcagcctgaggctgtcctgcgcagcctctttcagcggatacggcgtgtccaccatggcatggtttaggcaggcacctggcaagggactggagggagtggcagcaatcaccgtgggatccggaaacacatactatgccgactctgtgaagggccggttcaccatctctagagataacagcaagaatacagtgtacctgcagatgaacagcctgcgggccgaggacacagccatgtactattgtgccgtgggctatctgtccggaggatcttgggatgtgccaggaaggtacaactattggggccagggcaccctggtgacagtgagctcc

SEQ ID NO: 461 - DNA, 375 bp, synthetic construct
  misc_feature 1..375: note = Humanized sdAb AS63997VH6 Nucleic Acid Sequence
  source 1..375: mol_type = other DNA
caggtgcagctggtggagagcggaggaggagtggtgcagccaggaggcagcctgaggctgtcctgcgcagcctctttcagcggatacggcgtgtccaccatggcctggtttaggcaggcacctggcaagggaagggagggagtggcagcaatcaccgtgggatccggaaacacatactatgccgactctgtgaagggccggttcaccatctctagagataacagcaagaatacagtgtacctgcagatgaacagcctgcgggccgaggacacagccatgtactattgtgccgtgggctatctgtccggaggatcttgggatgtgccaggaaggtacaactattggggccagggcaccctggtgacagtgagctcc

SEQ ID NO: 462 - protein, 15 aa, synthetic construct
  REGION 1..15: note = Linker amino acid sequence
GGGGSGGGGSGGGGS

SEQ ID NO: 463 - protein, 10 aa, synthetic construct
  REGION 1..10: note = Linker amino acid sequence
GGGGSGGGGS

SEQ ID NO: 464 - protein, 5 aa, synthetic construct
  REGION 1..5: note = Linker amino acid sequence
GGGGS

SEQ ID NO: 465 - protein, 21 aa, synthetic construct
  REGION 1..21: note = CD8 signal peptide amino acid sequence
MALPVTALLLPLALLLHAARP

SEQ ID NO: 466 - protein, 69 aa, synthetic construct
  REGION 1..69: note = CD8 hinge amino acid sequence
TTTPAPRPPTPAPTIASQPLSLRPEACRPAAGGAVHTRGLDFACDIYIWAPLAGTCGVLLLSLVITLYC

SEQ ID NO: 467 - protein, 24 aa, synthetic construct
  REGION 1..24: note = CD8 transmembrane domain amino acid sequence
IYIWAPLAGTCGVLLLSLVITLYC

SEQ ID NO: 468 - protein, 42 aa, synthetic construct
  REGION 1..42: note = 4-1BB intracellular domain amino acid sequence
KRGRKKLLYIFKQPFMRPVQTTQEEDGCSCRFPEEEEGGCEL

SEQ ID NO: 469 - protein, 41 aa, synthetic construct
  REGION 1..41: note = CD28 intracellular domain amino acid sequence
RSKRSRLLHSDYMNMTPRRPGPTRKHYQPYAPPRDFAAYRS

SEQ ID NO: 470 - protein, 112 aa, synthetic construct
  REGION 1..112: note = CD3 intracellular domain amino acid sequence
RVKFSRSADAPAYKQGQNQLYNELNLGRREEYDVLDKRRGRDPEMGGKPRRKNPQEGLYNELQKDKMAEAYSEIGMKGERRRGKGHDGLYQGLSTATKDTYDALHMQALPPR

SEQ ID NO: 471 - protein, 25 aa, synthetic construct
  REGION 1..25: note = F2A element amino acid sequence
GSGVKQTLNFDLLKLAGDVESNPGP

SEQ ID NO: 472 - protein, 22 aa, synthetic construct
  REGION 1..22: note = P2A element amino acid sequence
GSGATNFSLLKQAGDVEENPGP

SEQ ID NO: 473 - protein, 257 aa, synthetic construct
  REGION 1..257: note = CAR3 anti-DLL3 scFv amino acid sequence
MALPVTALLLPLALLLHAARPAIQLTQSPSSLSASVGDRVTITCRASENIYYNLAWYQQKPGKAPKLLIYTANSLEDVPSRFSGSGSGTDFTLTISSLQPEDFATYFCKQAYDVPPTFGGGTKLEIKGGGGSGGGGSGGGGSQVQLVQSGAEVKKPGASVKVSCKASGYTFTRYWIHWIRQAPGQGLEWMGYINPTVYTEFNQNFKDRVTMTRDTSTSTVYMELSSLRSEDTAVYYCARGGSNFFDYWQGTTVTVSS

SEQ ID NO: 474 - protein, 27 aa, synthetic construct
  REGION 1..27: note = CD28 transmembrane domain amino acid sequence
FWVLVVVGGVLACYSLLVTVAFIIFWV

SEQ ID NO: 475 - protein, 39 aa, synthetic construct
  REGION 1..39: note = CD28 hinge
IEVMYPPPYLDNEKSNGTIIHVKGKHLCPSPLFPGPSKP

SEQ ID NO: 476 - protein, 369 aa, synthetic construct
  REGION 1..369: note = Camel anti-DLL3 CAR sequence CAS63997
MALPVTALLLPLALLLHAARPQVRLVESGGGSVQAGGSLRLSCAGSFSGYGVSTMAWFRQAPGKEREGVAAITVGSGNTYYADSVKGRFTISRDNAKRTVFLQMNSLKPEDTAMYYCAVGYLSGGSWDVPGRYNYWGQGTQVTVSSTTTPAPRPPTPAPTIASQPLSLRPEACRPAAGGAVHTRGLDFACDIYIWAPLAGTCGVLLLSLVITLYCKRGRKKLLYIFKQPFMRPVQTTQEEDGCSCRFPEEEEGGCELRVKFSRSADAPAYKQGQNQLYNELNLGRREEYDVLDKRRGRDPEMGGKPRRKNPQEGLYNELQKDKMAEAYSEIGMKGERRRGKGHDGLYQGLSTATKDTYDALHMQALPPR

SEQ ID NO: 477 - protein, 369 aa, synthetic construct
  REGION 1..369: note = Camel anti-DLL3 CAR sequence CAS64380
MALPVTALLLPLALLLHAARPEVQLVESGGGSVQAGGSLTLSCEASGNTYSSNYMGWFRQAPGKEREEVAVIYTRGGHTYYVDSVRGRFTISQDNAKNTVYLQMNSLKPEDTAMYYCAASSRHRLGLNNPRDYDYWGQGTQVTVSSTTTPAPRPPTPAPTIASQPLSLRPEACRPAAGGAVHTRGLDFACDIYIWAPLAGTCGVLLLSLVITLYCKRGRKKLLYIFKQPFMRPVQTTQEEDGCSCRFPEEEEGGCELRVKFSRSADAPAYKQGQNQLYNELNLGRREEYDVLDKRRGRDPEMGGKPRRKNPQEGLYNELQKDKMAEAYSEIGMKGERRRGKGHDGLYQGLSTATKDTYDALHMQALPPR

SEQ ID NO: 478 - protein, 369 aa, synthetic construct
  REGION 1..369: note = Camel anti-DLL3 CAR sequence CAS64511
MALPVTALLLPLALLLHAARPQVQLVESGGGSVQAGGSLRLSCAASRATYSTNYISWFRQAPGKEREAVATITTGDGETAYADSVKGRFTISRDNAKNTVYLQMNSLKPEDTAMYYCAANLRIGGDWFDGRDFRAWGQGTQVTVSSTTTPAPRPPTPAPTIASQPLSLRPEACRPAAGGAVHTRGLDFACDIYIWAPLAGTCGVLLLSLVITLYCKRGRKKLLYIFKQPFMRPVQTTQEEDGCSCRFPEEEEGGCELRVKFSRSADAPAYKQGQNQLYNELNLGRREEYDVLDKRRGRDPEMGGKPRRKNPQEGLYNELQKDKMAEAYSEIGMKGERRRGKGHDGLYQGLSTATKDTYDALHMQALPPR

SEQ ID NO: 479 - protein, 361 aa, synthetic construct
  REGION 1..361: note = Camel anti-DLL3 CAR sequence CAS64617
MALPVTALLLPLALLLHAARPQVQLVESGGGSVQAGGSLRLSCAASGYTDRCSMAWYRQAPGKERELVSRISTSGFTNYAASVKGRFTISQDNAKNTVYLQMNSLNPGDTGMYYCAIIVGRTCSLNYWGNGILVTVSSTTTPAPRPPTPAPTIASQPLSLRPEACRPAAGGAVHTRGLDFACDIYIWAPLAGTCGVLLLSLVITLYCKRGRKKLLYIFKQPFMRPVQTTQEEDGCSCRFPEEEEGGCELRVKFSRSADAPAYKQGQNQLYNELNLGRREEYDVLDKRRGRDPEMGGKPRRKNPQEGLYNELQKDKMAEAYSEIGMKGERRRGKGHDGLYQGLSTATKDTYDALHMQALPPR

SEQ ID NO: 480 - protein, 376 aa, synthetic construct
  REGION 1..376: note = Camel anti-DLL3 CAR sequence CAS69443
MALPVTALLLPLALLLHAARPEVQLAESGGGSVQAGGSLRLSCSASGFTFDDSDMAWYRQAPGDGCDLVSTISSDGSTYYADSVKGRFTISQDNAKNTVYLQMHSLKPEDTAVYYCAADFLTGFYYSDSPHPAPCSASDFGYWGQGTQVTVSSTTTPAPRPPTPAPTIASQPLSLRPEACRPAAGGAVHTRGLDFACDIYIWAPLAGTCGVLLLSLVITLYCKRGRKKLLYIFKQPFMRPVQTTQEEDGCSCRFPEEEEGGCELRVKFSRSADAPAYKQGQNQLYNELNLGRREEYDVLDKRRGRDPEMGGKPRRKNPQEGLYNELQKDKMAEAYSEIGMKGERRRGKGHDGLYQGLSTATKDTYDALHMQALPPR

SEQ ID NO: 481 - protein, 369 aa, synthetic construct
  REGION 1..369: note = Camel anti-DLL3 CAR sequence CAS63931
MALPVTALLLPLALLLHAARPEVQLAESGGGSVQAGGSLRLSCAGSFSGYGVSTMAWFRQAPGKEREGVAAITVGSGNTYYADSVTGRFTISRDNAKRTVYLQMNSLKPEDTAMYYCAAGWLSGGSWHVPGRYNYWGQGTQVTVSSTTTPAPRPPTPAPTIASQPLSLRPEACRPAAGGAVHTRGLDFACDIYIWAPLAGTCGVLLLSLVITLYCKRGRKKLLYIFKQPFMRPVQTTQEEDGCSCRFPEEEEGGCELRVKFSRSADAPAYKQGQNQLYNELNLGRREEYDVLDKRRGRDPEMGGKPRRKNPQEGLYNELQKDKMAEAYSEIGMKGERRRGKGHDGLYQGLSTATKDTYDALHMQALPPR

SEQ ID NO: 482 - protein, 369 aa, synthetic construct
  REGION 1..369: note = Camel anti-DLL3 CAR sequence CAS64047
MALPVTALLLPLALLLHAARPQVHLVESGGGSVQAGGSLRLSCAASQYVYRWDLMGWFRQAPGKEREAVAAVYTGDGITYYADSVKGRFSISQDNAKNTVYLQMNSLKPEDTGMYFCAAGFVSGGRWNQSYRYKYWGQGTQVTVSSTTTPAPRPPTPAPTIASQPLSLRPEACRPAAGGAVHTRGLDFACDIYIWAPLAGTCGVLLLSLVITLYCKRGRKKLLYIFKQPFMRPVQTTQEEDGCSCRFPEEEEGGCELRVKFSRSADAPAYKQGQNQLYNELNLGRREEYDVLDKRRGRDPEMGGKPRRKNPQEGLYNELQKDKMAEAYSEIGMKGERRRGKGHDGLYQGLSTATKDTYDALHMQALPPR

SEQ ID NO: 483 - protein, 373 aa, synthetic construct
  REGION 1..373: note = Camel anti-DLL3 CAR sequence CAS64052
MALPVTALLLPLALLLHAARPQVHLMESGGGSVQAGGSLRLSCAASGYTYRSNFMGWFRQAPGKEREGIATIHSGVATTYYADSVKGRFTISQDNAKNTVYLQMNSLKPEDTAMYYCAAGGPPANADRWYPLRPPGYNYWGQGTQVTVSSTTTPAPRPPTPAPTIASQPLSLRPEACRPAAGGAVHTRGLDFACDIYIWAPLAGTCGVLLLSLVITLYCKRGRKKLLYIFKQPFMRPVQTTQEEDGCSCRFPEEEEGGCELRVKFSRSADAPAYKQGQNQLYNELNLGRREEYDVLDKRRGRDPEMGGKPRRKNPQEGLYNELQKDKMAEAYSEIGMKGERRRGKGHDGLYQGLSTATKDTYDALHMQALPPR

SEQ ID NO: 484 - protein, 371 aa, synthetic construct
  REGION 1..371: note = Camel anti-DLL3 CAR sequence CAS64062
MALPVTALLLPLALLLHAARPQVRLVESGGGSVQVGGSLRLSCAASRSPYSSSRCMGWFRQAPGKEREGVAALYTGGGSTSYADSVKGRFTISQDNAKNTVYLQMNSLKPEDTAMYYCAAVVPRGGSCRLDERGYYHWGQGTQVTVSSTTTPAPRPPTPAPTIASQPLSLRPEACRPAAGGAVHTRGLDFACDIYIWAPLAGTCGVLLLSLVITLYCKRGRKKLLYIFKQPFMRPVQTTQEEDGCSCRFPEEEEGGCELRVKFSRSADAPAYKQGQNQLYNELNLGRREEYDVLDKRRGRDPEMGGKPRRKNPQEGLYNELQKDKMAEAYSEIGMKGERRRGKGHDGLYQGLSTATKDTYDALHMQALPPR

SEQ ID NO: 485 - protein, 369 aa, synthetic construct
  REGION 1..369: note = Humanized anti-DLL3 CAR sequence CAS64380VH4
MALPVTALLLPLALLLHAARPEVQLVESGGGLVQPGGSLRLSCAASGNTYSSNYMGWFRQAPGKGLEEVAVIYTRGGHTYYVDSVRGRFTISRDNAKNSLYLQMNSLRAEDTAVYYCAASSRHRLGLNNPRDYDYWGQGTLVTVSSTTTPAPRPPTPAPTIASQPLSLRPEACRPAAGGAVHTRGLDFACDIYIWAPLAGTCGVLLLSLVITLYCKRGRKKLLYIFKQPFMRPVQTTQEEDGCSCRFPEEEEGGCELRVKFSRSADAPAYKQGQNQLYNELNLGRREEYDVLDKRRGRDPEMGGKPRRKNPQEGLYNELQKDKMAEAYSEIGMKGERRRGKGHDGLYQGLSTATKDTYDALHMQALPPR

SEQ ID NO: 486 - protein, 369 aa, synthetic construct
  REGION 1..369: note = Humanized anti-DLL3 CAR sequence CAS64380VH5
MALPVTALLLPLALLLHAARPEVQLVESGGGLVQPGGSLRLSCAASGNTYSSNYMGWFRQAPGKGLEEVAVIYTRGGHTYYVDSVRGRFTISQDNAKNSLYLQMNSLRAEDTAVYYCAASSRHRLGLNNPRDYDYWGQGTLVTVSSTTTPAPRPPTPAPTIASQPLSLRPEACRPAAGGAVHTRGLDFACDIYIWAPLAGTCGVLLLSLVITLYCKRGRKKLLYIFKQPFMRPVQTTQEEDGCSCRFPEEEEGGCELRVKFSRSADAPAYKQGQNQLYNELNLGRREEYDVLDKRRGRDPEMGGKPRRKNPQEGLYNELQKDKMAEAYSEIGMKGERRRGKGHDGLYQGLSTATKDTYDALHMQALPPR

SEQ ID NO: 487 - protein, 369 aa, synthetic construct
  REGION 1..369: note = Humanized anti-DLL3 CAR sequence CAS64380VH6
MALPVTALLLPLALLLHAARPEVQLVESGGGLVQPGGSLRLSCAASGNTYSSNYMGWFRQAPGKGLEEVAVIYTRGGHTYYVDSVRGRFTISQDNAKNSVYLQMNSLRAEDTAMYYCAASSRHRLGLNNPRDYDYWGQGTLVTVSSTTTPAPRPPTPAPTIASQPLSLRPEACRPAAGGAVHTRGLDFACDIYIWAPLAGTCGVLLLSLVITLYCKRGRKKLLYIFKQPFMRPVQTTQEEDGCSCRFPEEEEGGCELRVKFSRSADAPAYKQGQNQLYNELNLGRREEYDVLDKRRGRDPEMGGKPRRKNPQEGLYNELQKDKMAEAYSEIGMKGERRRGKGHDGLYQGLSTATKDTYDALHMQALPPR

SEQ ID NO: 488 - protein, 369 aa, synthetic construct
  REGION 1..369: note = Humanized anti-DLL3 CAR sequence CAS64380VH7
MALPVTALLLPLALLLHAARPEVQLVESGGGLVQPGGSLRLSCAASGNTYSSNYMGWFRQAPGKGREEVAVIYTRGGHTYYVDSVRGRFTISQDNAKNSVYLQMNSLRAEDTAMYYCAASSRHRLGLNNPRDYDYWGQGTLVTVSSTTTPAPRPPTPAPTIASQPLSLRPEACRPAAGGAVHTRGLDFACDIYIWAPLAGTCGVLLLSLVITLYCKRGRKKLLYIFKQPFMRPVQTTQEEDGCSCRFPEEEEGGCELRVKFSRSADAPAYKQGQNQLYNELNLGRREEYDVLDKRRGRDPEMGGKPRRKNPQEGLYNELQKDKMAEAYSEIGMKGERRRGKGHDGLYQGLSTATKDTYDALHMQALPPR

SEQ ID NO: 489 - protein, 369 aa, synthetic construct
  REGION 1..369: note = Humanized anti-DLL3 CAR sequence CAS64511VH4
MALPVTALLLPLALLLHAARPEVQLVESGGGLVQPGGSLRLSCAASRATYSTNYISWFRQAPGKGLEAVATITTGDGETAYADSVKGRFTISRDNAKNSLYLQMNSLRAEDTAVYYCAANLRIGGDWFDGRDFRAWGQGTLVTVSSTTTPAPRPPTPAPTIASQPLSLRPEACRPAAGGAVHTRGLDFACDIYIWAPLAGTCGVLLLSLVITLYCKRGRKKLLYIFKQPFMRPVQTTQEEDGCSCRFPEEEEGGCELRVKFSRSADAPAYKQGQNQLYNELNLGRREEYDVLDKRRGRDPEMGGKPRRKNPQEGLYNELQKDKMAEAYSEIGMKGERRRGKGHDGLYQGLSTATKDTYDALHMQALPPR

SEQ ID NO: 490 - protein, 369 aa, synthetic construct
  REGION 1..369: note = Humanized anti-DLL3 CAR sequence CAS64511VH5
MALPVTALLLPLALLLHAARPEVQLVESGGGLVQPGGSLRLSCAASRATYSTNYISWFRQAPGKGLEAVATITTGDGETAYADSVKGRFTISRDNAKNSVYLQMNSLRAEDTAMYYCAANLRIGGDWFDGRDFRAWGQGTLVTVSSTTTPAPRPPTPAPTIASQPLSLRPEACRPAAGGAVHTRGLDFACDIYIWAPLAGTCGVLLLSLVITLYCKRGRKKLLYIFKQPFMRPVQTTQEEDGCSCRFPEEEEGGCELRVKFSRSADAPAYKQGQNQLYNELNLGRREEYDVLDKRRGRDPEMGGKPRRKNPQEGLYNELQKDKMAEAYSEIGMKGERRRGKGHDGLYQGLSTATKDTYDALHMQALPPR

SEQ ID NO: 491 - protein, 369 aa, synthetic construct
  REGION 1..369: note = Humanized anti-DLL3 CAR sequence CAS64511VH6
MALPVTALLLPLALLLHAARPEVQLVESGGGLVQPGGSLRLSCAASRATYSTNYISWFRQAPGKGREAVATITTGDGETAYADSVKGRFTISRDNAKNSVYLQMNSLRAEDTAMYYCAANLRIGGDWFDGRDFRAWGQGTLVTVSSTTTPAPRPPTPAPTIASQPLSLRPEACRPAAGGAVHTRGLDFACDIYIWAPLAGTCGVLLLSLVITLYCKRGRKKLLYIFKQPFMRPVQTTQEEDGCSCRFPEEEEGGCELRVKFSRSADAPAYKQGQNQLYNELNLGRREEYDVLDKRRGRDPEMGGKPRRKNPQEGLYNELQKDKMAEAYSEIGMKGERRRGKGHDGLYQGLSTATKDTYDALHMQALPPR

SEQ ID NO: 492 - protein, 369 aa, synthetic construct
  REGION 1..369: note = Humanized anti-DLL3 CAR sequence CAS63997VH4
MALPVTALLLPLALLLHAARPQVQLVESGGGVVQPGGSLRLSCAASFSGYGVSTMAWFRQAPGKGLEGVAAITVGSGNTYYADSVKGRFTISRDNSKNTLYLQMNSLRAEDTAVYYCAVGYLSGGSWDVPGRYNYWGQGTLVTVSSTTTPAPRPPTPAPTIASQPLSLRPEACRPAAGGAVHTRGLDFACDIYIWAPLAGTCGVLLLSLVITLYCKRGRKKLLYIFKQPFMRPVQTTQEEDGCSCRFPEEEEGGCELRVKFSRSADAPAYKQGQNQLYNELNLGRREEYDVLDKRRGRDPEMGGKPRRKNPQEGLYNELQKDKMAEAYSEIGMKGERRRGKGHDGLYQGLSTATKDTYDALHMQALPPR

SEQ ID NO: 493 - protein, 369 aa, synthetic construct
  REGION 1..369: note = Humanized anti-DLL3 CAR sequence CAS63997VH5
MALPVTALLLPLALLLHAARPQVQLVESGGGVVQPGGSLRLSCAASFSGYGVSTMAWFRQAPGKGLEGVAAITVGSGNTYYADSVKGRFTISRDNSKNTVYLQMNSLRAEDTAMYYCAVGYLSGGSWDVPGRYNYWGQGTLVTVSSTTTPAPRPPTPAPTIASQPLSLRPEACRPAAGGAVHTRGLDFACDIYIWAPLAGTCGVLLLSLVITLYCKRGRKKLLYIFKQPFMRPVQTTQEEDGCSCRFPEEEEGGCELRVKFSRSADAPAYKQGQNQLYNELNLGRREEYDVLDKRRGRDPEMGGKPRRKNPQEGLYNELQKDKMAEAYSEIGMKGERRRGKGHDGLYQGLSTATKDTYDALHMQALPPR

SEQ ID NO: 494 - protein, 369 aa, synthetic construct
  REGION 1..369: note = Humanized anti-DLL3 CAR sequence CAS63997VH6
MALPVTALLLPLALLLHAARPQVQLVESGGGVVQPGGSLRLSCAASFSGYGVSTMAWFRQAPGKGREGVAAITVGSGNTYYADSVKGRFTISRDNSKNTVYLQMNSLRAEDTAMYYCAVGYLSGGSWDVPGRYNYWGQGTLVTVSSTTTPAPRPPTPAPTIASQPLSLRPEACRPAAGGAVHTRGLDFACDIYIWAPLAGTCGVLLLSLVITLYCKRGRKKLLYIFKQPFMRPVQTTQEEDGCSCRFPEEEEGGCELRVKFSRSADAPAYKQGQNQLYNELNLGRREEYDVLDKRRGRDPEMGGKPRRKNPQEGLYNELQKDKMAEAYSEIGMKGERRRGKGHDGLYQGLSTATKDTYDALHMQALPPR

SEQ ID NO: 495 - protein, 11 aa, synthetic construct
  REGION 1..11: note = Anti-DLL3 human scFv CDR1 sequence AS56704
RASQSVSSAVA

SEQ ID NO: 496 - protein, 7 aa, synthetic construct
  REGION 1..7: note = Anti-DLL3 human scFv CDR2 sequence AS56704
SASSLYS

SEQ ID NO: 497 - protein, 9 aa, synthetic construct
  REGION 1..9: note = Anti-DLL3 human scFv CDR3 sequence AS56704
QQASWSPIT

SEQ ID NO: 498 - protein, 10 aa, synthetic construct
  REGION 1..10: note = Anti-DLL3 human scFv VH CDR1 sequence AS56704
GFNISSSYMH

SEQ ID NO: 499 - protein, 17 aa, synthetic construct
  REGION 1..17: note = Anti-DLL3 human scFv VH CDR2 sequence AS56704
YIYPSYGYTSYADSVKG

SEQ ID NO: 500 - protein, 10 aa, synthetic construct
  REGION 1..10: note = Anti-DLL3 human scFv VH CDR3 sequence AS56704
GGYYYHGMDY

SEQ ID NO: 501 - protein, 11 aa, synthetic construct
  REGION 1..11: note = Anti-DLL3 human scFv VL CDR1 sequence AS56788
RASQSVSSAVA

SEQ ID NO: 502 - protein, 7 aa, synthetic construct
  REGION 1..7: note = Anti-DLL3 human scFv VL CDR2 sequence AS56788
SASSLYS

SEQ ID NO: 503 - protein, 10 aa, synthetic construct
  REGION 1..10: note = Anti-DLL3 human scFv VL CDR3 sequence AS56788
QQHYAPSLIT

SEQ ID NO: 504 - protein, 10 aa, synthetic construct
  REGION 1..10: note = Anti-DLL3 human scFv VH CDR1 sequence AS56788
GFNISSYSMH

SEQ ID NO: 505 - protein, 17 aa, synthetic construct
  REGION 1..17: note = Anti-DLL3 human scFv VH CDR2 sequence AS56788
YISSYYGYTYYADSVKG

SEQ ID NO: 506 - protein, 9 aa, synthetic construct
  REGION 1..9: note = Anti-DLL3 human scFv VH CDR3 sequence AS56788
YSYYYGMDY

SEQ ID NO: 507 - protein, 107 aa, synthetic construct
  REGION 1..107: note = Anti-DLL3 human scFv VL amino acid sequence AS56704
DIQMTQSPSSLSASVGDRVTITCRASQSVSSAVAWYQQKPGKAPKLLIYSASSLYSGVPSRFSGSRSGTDFTLTISSLQPEDFATYYCQQASWSPITFGQGTKVEIK

SEQ ID NO: 508 - protein, 119 aa, synthetic construct
  REGION 1..119: note = Anti-DLL3 human scFv VH amino acid sequence AS56704
EVQLVESGGGLVQPGGSLRLSCAASGFNISSSYMHWVRQAPGKGLEWVAYIYPSYGYTSYADSVKGRFTISADTSKNTAYLQMNSLRAEDTAVYYCARGGYYYHGMDYWGQGTLVTVSS

SEQ ID NO: 509 - protein, 108 aa, synthetic construct
  REGION 1..108: note = Anti-DLL3 human scFv VL amino acid sequence AS56788
DIQMTQSPSSLSASVGDRVTITCRASQSVSSAVAWYQQKPGKAPKLLIYSASSLYSGVPSRFSGSRSGTDFTLTISSLQPEDFATYYCQQHYAPSLITFGQGTKVEIK

SEQ ID NO: 510 - protein, 118 aa, synthetic construct
  REGION 1..118: note = Anti-DLL3 human scFv VH amino acid sequence AS56788
EVQLVESGGGLVQPGGSLRLSCAASGFNISSYSMHWVRQAPGKGLEWVAYISSYYGYTYYADSVKGRFTISADTSKNTAYLQMNSLRAEDTAVYYCARYSYYYGMDYWGQGTLVTVSS

SEQ ID NO: 511 - DNA, 321 bp, synthetic construct
  misc_feature 1..321: note = Nucleic Acid Sequence for VL domain of anti-DLL3 human scFv AS56704
  source 1..321: mol_type = other DNA
gacatccagatgacccagagcccgagcagcctgagcgcgagcgttggtgaccgtgttaccattacctgccgtgcgagccagagcgttagcagcgcggtggcgtggtaccagcaaaagccgggtaaagcgccgaagctgctgatctatagcgcgagcagcctgtatagcggcgttccgagccgtttcagcggtagccgtagcggcaccgactttaccctgaccattagcagcctgcagccggaagatttcgcaacttattactgtcagcaagcttcttggtctccgatcacgttcggacagggcaccaaagttgagattaaa

SEQ ID NO: 512 - DNA, 357 bp, synthetic construct
  misc_feature 1..357: note = Nucleic Acid Sequence for VH domain of anti-DLL3 human scFv AS56704
  source 1..357: mol_type = other DNA
gaggttcaactggtggagagcggtggtggtctggttcagccgggtggtagcctgcgtctgagctgcgcagcttctggcttcaacatctcttcttcttatatgcactgggtgcgtcaggcgccgggtaaaggcctggaatgggttgcatatatttatccttcttatggctatacttcttatgccgatagcgtcaagggccgtttcaccatcagcgcggataccagcaaaaacaccgcatacctgcaaatgaacagcctgcgtgcggaagataccgccgtctattattgtgctcgcggtggttactactaccatggtatggactactggggtcaaggcaccctggttaccgtgagcagc

SEQ ID NO: 513 - DNA, 324 bp, synthetic construct
  misc_feature 1..324: note = Nucleic Acid Sequence for VL domain of anti-DLL3 human scFv AS56788
  source 1..324: mol_type = other DNA
gacatccagatgacccagagcccgagcagcctgagcgcgagcgttggtgaccgtgttaccattacctgccgtgcgagccagagcgttagcagcgcggtggcgtggtaccagcaaaagccgggtaaagcgccgaagctgctgatctatagcgcgagcagcctgtatagcggcgttccgagccgtttcagcggtagccgtagcggcaccgactttaccctgaccattagcagcctgcagccggaagatttcgcaacttattactgtcagcaacattacgctccgtctctgatcacgttcggacagggcaccaaagttgagattaaa

SEQ ID NO: 514 - DNA, 354 bp, synthetic construct
  misc_feature 1..354: note = Nucleic Acid Sequence for VH domain of anti-DLL3 human scFv AS56788
  source 1..354: mol_type = other DNA
gaggttcaactggtggagagcggtggtggtctggttcagccgggtggtagcctgcgtctgagctgcgcagcttctggcttcaacatctcttcttattctatgcactgggtgcgtcaggcgccgggtaaaggcctggaatgggttgcatatatttcttcttattatggctatacttattatgccgatagcgtcaagggccgtttcaccatcagcgcggataccagcaaaaacaccgcatacctgcaaatgaacagcctgcgtgcggaagataccgccgtctattattgtgctcgctactcttactactacggtatggactactggggtcaaggcaccctggttaccgtgagcagc

SEQ ID NO: 515 - protein, 485 aa, synthetic construct
  REGION 1..485: note = Human anti-DLL3 scFv CAR sequences CAS56704
MALPVTALLLPLALLLHAARPDIQMTQSPSSLSASVGDRVTITCRASQSVSSAVAWYQQKPGKAPKLLIYSASSLYSGVPSRFSGSRSGTDFTLTISSLQPEDFATYYCQQASWSPITFGQGTKVEIKGGGGSGGGGSGGGGSEVQLVESGGGLVQPGGSLRLSCAASGFNISSSYMHWVRQAPGKGLEWVAYIYPSYGYTSYADSVKGRFTISADTSKNTAYLQMNSLRAEDTAVYYCARGGYYYHGMDYWGQGTLVTVSSTTTPAPRPPTPAPTIASQPLSLRPEACRPAAGGAVHTRGLDFACDIYIWAPLAGTCGVLLLSLVITLYCKRGRKKLLYIFKQPFMRPVQTTQEEDGCSCRFPEEEEGGCELRVKFSRSADAPAYKQGQNQLYNELNLGRREEYDVLDKRRGRDPEMGGKPRRKNPQEGLYNELQKDKMAEAYSEIGMKGERRRGKGHDGLYQGLSTATKDTYDALHMQALPPR

SEQ ID NO: 516 - protein, 485 aa, synthetic construct
  REGION 1..485: note = Human anti-DLL3 scFv CAR sequences CAS56788
MALPVTALLLPLALLLHAARPDIQMTQSPSSLSASVGDRVTITCRASQSVSSAVAWYQQKPGKAPKLLIYSASSLYSGVPSRFSGSRSGTDFTLTISSLQPEDFATYYCQQHYAPSLITFGQGTKVEIKGGGGSGGGGSGGGGSEVQLVESGGGLVQPGGSLRLSCAASGFNISSYSMHWVRQAPGKGLEWVAYISSYYGYTYYADSVKGRFTISADTSKNTAYLQMNSLRAEDTAVYYCARYSYYYGMDYWGQGTLVTVSSTTTPAPRPPTPAPTIASQPLSLRPEACRPAAGGAVHTRGLDFACDIYIWAPLAGTCGVLLLSLVITLYCKRGRKKLLYIFKQPFMRPVQTTQEEDGCSCRFPEEEEGGCELRVKFSRSADAPAYKQGQNQLYNELNLGRREEYDVLDKRRGRDPEMGGKPRRKNPQEGLYNELQKDKMAEAYSEIGMKGERRRGKGHDGLYQGLSTATKDTYDALHMQALPPR

SEQ ID NO: 517 - protein, 476 aa, synthetic construct
  REGION 1..476: note = 1H2.1 amino acid sequence
MALPVTALLLPLALLLHAARPQVQLQESGPGLVKPSETLSLTCTVSGDSISSYYWTWIRQPPGKGLEWIGYIYYSGTTNYNPSLKSRVTISVDTSKSQFSLKLSSVTAADTAVYYCASIAVRGFFFDYWGQGTLVTVSSGGGGSGGGGSGGGGSEIVLTQSPGTLSLSPGERATLSCRASQSVSSSYLAWYQQKPGQAPRLLIYGASTRATGIPDRFSGSGSGTDFTLTISRLEPEDFAVYYCQQYGTSPLTFGGGTKVEIKRAAALDNEKSNGTIIHVKGKHLCPSPLFPGPSKPFWVLVVVGGVLACYSLLVTVAFIIFWVRSKRSRLLHSDYMNMTPRRPGPTRKHYQPYAPPRDFAAYRSRVKFSRSADAPAYQQGQNQLYNELNLGRREEYDVLDKRRGRDPEMGGKPRRKNPQEGLYNELQKDKMAEAYSEIGMKGERRRGKGHDGLYQGLSTATKDTYDALHMQALPPR

SEQ ID NO: 518 - protein, 509 aa, synthetic construct
  REGION 1..509: note = T1 amino acid sequence
MALPVTALLLPLALLLHAARPEVQLVESGGGLVQPGGSLRLSCAASGNTYSSNYMGWFRQAPGKGLEEVAVIYTRGGHTYYVDSVRGRFTISQDNAKNSLYLQMNSLRAEDTAVYYCAASSRHRLGLNNPRDYDYWGQGTLVTVSSGGGGSGGGGSGGGGSEVQLVESGGGLVQPGGSLRLSCAASGNTYSSNYMGWFRQAPGKGLEEVAVIYTRGGHTYYVDSVRGRFTISQDNAKNSLYLQMNSLRAEDTAVYYCAASSRHRLGLNNPRDYDYWGQGTLVTVSSTTTPAPRPPTPAPTIASQPLSLRPEACRPAAGGAVHTRGLDFACDIYIWAPLAGTCGVLLLSLVITLYCKRGRKKLLYIFKQPFMRPVQTTQEEDGCSCRFPEEEEGGCELRVKFSRSADAPAYKQGQNQLYNELNLGRREEYDVLDKRRGRDPEMGGKPRRKNPQEGLYNELQKDKMAEAYSEIGMKGERRRGKGHDGLYQGLSTATKDTYDALHMQALPPR

SEQ ID NO: 519 - protein, 509 aa, synthetic construct
  REGION 1..509: note = T2 amino acid sequence
MALPVTALLLPLALLLHAARPQVQLVESGGGVVQPGGSLRLSCAASFSGYGVSTMAWFRQAPGKGLEGVAAITVGSGNTYYADSVKGRFTISRDNSKNTVYLQMNSLRAEDTAMYYCAVGYLSGGSWDVPGRYNYWGQGTLVTVSSGGGGSGGGGSGGGGSQVQLVESGGGVVQPGGSLRLSCAASFSGYGVSTMAWFRQAPGKGLEGVAAITVGSGNTYYADSVKGRFTISRDNSKNTVYLQMNSLRAEDTAMYYCAVGYLSGGSWDVPGRYNYWGQGTLVTVSSTTTPAPRPPTPAPTIASQPLSLRPEACRPAAGGAVHTRGLDFACDIYIWAPLAGTCGVLLLSLVITLYCKRGRKKLLYIFKQPFMRPVQTTQEEDGCSCRFPEEEEGGCELRVKFSRSADAPAYKQGQNQLYNELNLGRREEYDVLDKRRGRDPEMGGKPRRKNPQEGLYNELQKDKMAEAYSEIGMKGERRRGKGHDGLYQGLSTATKDTYDALHMQALPPR

SEQ ID NO: 520 - protein, 509 aa, synthetic construct
  REGION 1..509: note = T3 amino acid sequence
MALPVTALLLPLALLLHAARPQVQLVESGGGVVQPGGSLRLSCAASFSGYGVSTMAWFRQAPGKGLEGVAAITVGSGNTYYADSVKGRFTISRDNSKNTVYLQMNSLRAEDTAMYYCAVGYLSGGSWDVPGRYNYWGQGTLVTVSSGGGGSGGGGSGGGGSEVQLVESGGGLVQPGGSLRLSCAASGNTYSSNYMGWFRQAPGKGLEEVAVIYTRGGHTYYVDSVRGRFTISQDNAKNSLYLQMNSLRAEDTAVYYCAASSRHRLGLNNPRDYDYWGQGTLVTVSSTTTPAPRPPTPAPTIASQPLSLRPEACRPAAGGAVHTRGLDFACDIYIWAPLAGTCGVLLLSLVITLYCKRGRKKLLYIFKQPFMRPVQTTQEEDGCSCRFPEEEEGGCELRVKFSRSADAPAYKQGQNQLYNELNLGRREEYDVLDKRRGRDPEMGGKPRRKNPQEGLYNELQKDKMAEAYSEIGMKGERRRGKGHDGLYQGLSTATKDTYDALHMQALPPR

SEQ ID NO: 521 - protein, 775 aa, synthetic construct
  REGION 1..775: note = T3-PD-1DNR amino acid sequence
MALPVTALLLPLALLLHAARPQVQLVESGGGVVQPGGSLRLSCAASFSGYGVSTMAWFRQAPGKGLEGVAAITVGSGNTYYADSVKGRFTISRDNSKNTVYLQMNSLRAEDTAMYYCAVGYLSGGSWDVPGRYNYWGQGTLVTVSSGGGGSGGGGSGGGGSEVQLVESGGGLVQPGGSLRLSCAASGNTYSSNYMGWFRQAPGKGLEEVAVIYTRGGHTYYVDSVRGRFTISQDNAKNSLYLQMNSLRAEDTAVYYCAASSRHRLGLNNPRDYDYWGQGTLVTVSSTTTPAPRPPTPAPTIASQPLSLRPEACRPAAGGAVHTRGLDFACDIYIWAPLAGTCGVLLLSLVITLYCKRGRKKLLYIFKQPFMRPVQTTQEEDGCSCRFPEEEEGGCELRVKFSRSADAPAYKQGQNQLYNELNLGRREEYDVLDKRRGRDPEMGGKPRRKNPQEGLYNELQKDKMAEAYSEIGMKGERRRGKGHDGLYQGLSTATKDTYDALHMQALPPRGSGATNFSLLKQAGDVEENPGPMQIPQAPWPVVWAVLQLGWRPGWFLDSPDRPWNPPTFSPALLVVTEGDNATFTCSFSNTSESFVLNWYRMSPSNQTDKLAAFPEDRSQPGQDCRFRVTQLPNGRDFHMSVVRARRNDSGTYLCGAISLAPKAQIKESLRAELRVTERRAEVPTAHPSPSPRPAGQAAAPTTTPAPRPPTPAPTIASQPLSLRPEACRPAAGGAVHTRGLDFACDIYIWAPLAGTCGVLLLSLVITLYCNHRRIQ

SEQ ID NO: 522 - protein, 766 aa, synthetic construct
  REGION 1..766: note = T3-PD-1CSR amino acid sequence
MALPVTALLLPLALLLHAARPQVQLVESGGGVVQPGGSLRLSCAASFSGYGVSTMAWFRQAPGKGLEGVAAITVGSGNTYYADSVKGRFTISRDNSKNTVYLQMNSLRAEDTAMYYCAVGYLSGGSWDVPGRYNYWGQGTLVTVSSGGGGSGGGGSGGGGSEVQLVESGGGLVQPGGSLRLSCAASGNTYSSNYMGWFRQAPGKGLEEVAVIYTRGGHTYYVDSVRGRFTISQDNAKNSLYLQMNSLRAEDTAVYYCAASSRHRLGLNNPRDYDYWGQGTLVTVSSTTTPAPRPPTPAPTIASQPLSLRPEACRPAAGGAVHTRGLDFACDIYIWAPLAGTCGVLLLSLVITLYCKRGRKKLLYIFKQPFMRPVQTTQEEDGCSCRFPEEEEGGCELRVKFSRSADAPAYKQGQNQLYNELNLGRREEYDVLDKRRGRDPEMGGKPRRKNPQEGLYNELQKDKMAEAYSEIGMKGERRRGKGHDGLYQGLSTATKDTYDALHMQALPPRGSGATNFSLLKQAGDVEENPGPMQIPQAPWPVVWAVLQLGWRPGWFLDSPDRPWNPPTFSPALLVVTEGDNATFTCSFSNTSESFVLNWYRMSPSNQTDKLAAFPEDRSQPGQDCRFRVTQLPNGRDFHMSVVRARRNDSGTYLCGAISLAPKAQIKESLRAELRVTERRAEVPTAHCPSPLFPGPSKPFWVLVVVGGVLACYSLLVTVAFIIFWVRSKRSRLLHSDYMNMTPRRPGPTRKHYQPYAPPRDFAAYRS

SEQ ID NO: 523 - protein, 244 aa, synthetic construct
  REGION 1..244: note = PD-1DNR amino acid sequence
MQIPQAPWPVVWAVLQLGWRPGWFLDSPDRPWNPPTFSPALLVVTEGDNATFTCSFSNTSESFVLNWYRMSPSNQTDKLAAFPEDRSQPGQDCRFRVTQLPNGRDFHMSVVRARRNDSGTYLCGAISLAPKAQIKESLRAELRVTERRAEVPTAHPSPSPRPAGQAAAPTTTPAPRPPTPAPTIASQPLSLRPEACRPAAGGAVHTRGLDFACDIYIWAPLAGTCGVLLLSLVITLYCNHRRIQ

SEQ ID NO: 524 - protein, 235 aa, synthetic construct
  REGION 1..235: note = PD-1CSR amino acid sequence
MQIPQAPWPVVWAVLQLGWRPGWFLDSPDRPWNPPTFSPALLVVTEGDNATFTCSFSNTSESFVLNWYRMSPSNQTDKLAAFPEDRSQPGQDCRFRVTQLPNGRDFHMSVVRARRNDSGTYLCGAISLAPKAQIKESLRAELRVTERRAEVPTAHCPSPLFPGPSKPFWVLVVVGGVLACYSLLVTVAFIIFWVRSKRSRLLHSDYMNMTPRRPGPTRKHYQPYAPPRDFAAYRS

SEQ ID NO: 525 - protein, 730 aa, synthetic construct
  REGION 1..730: note = T3-P2A-TGF- -DNR amino acid sequence
MALPVTALLLPLALLLHAARPQVQLVESGGGVVQPGGSLRLSCAASFSGYGVSTMAWFRQAPGKGLEGVAAITVGSGNTYYADSVKGRFTISRDNSKNTVYLQMNSLRAEDTAMYYCAVGYLSGGSWDVPGRYNYWGQGTLVTVSSGGGGSGGGGSGGGGSEVQLVESGGGLVQPGGSLRLSCAASGNTYSSNYMGWFRQAPGKGLEEVAVIYTRGGHTYYVDSVRGRFTISQDNAKNSLYLQMNSLRAEDTAVYYCAASSRHRLGLNNPRDYDYWGQGTLVTVSSTTTPAPRPPTPAPTIASQPLSLRPEACRPAAGGAVHTRGLDFACDIYIWAPLAGTCGVLLLSLVITLYCKRGRKKLLYIFKQPFMRPVQTTQEEDGCSCRFPEEEEGGCELRVKFSRSADAPAYKQGQNQLYNELNLGRREEYDVLDKRRGRDPEMGGKPRRKNPQEGLYNELQKDKMAEAYSEIGMKGERRRGKGHDGLYQGLSTATKDTYDALHMQALPPRGSGATNFSLLKQAGDVEENPGPMGRGLLRGLWPLHIVLWTRIASTIPPHVQKSVNNDMIVTDNNGAVKFPQLCKFCDVRFSTCDNQKSCMSNCSITSICEKPQEVCVAVWRKNDENITLETVCHDPKLPYHDFILEDAASPKCIMKEKKKPGETFFMCSCSSDECNDNIIFSEEYNTSNPDLLLVIFQVTGISLLPPLGVAISVIIIFYCYRVNRQQKLSS

SEQ ID NO: 526 - protein, 730 aa, synthetic construct
  REGION 1..730: note = TGF- -DNR-P2A-T3 amino acid sequence
MGRGLLRGLWPLHIVLWTRIASTIPPHVQKSVNNDMIVTDNNGAVKFPQLCKFCDVRFSTCDNQKSCMSNCSITSICEKPQEVCVAVWRKNDENITLETVCHDPKLPYHDFILEDAASPKCIMKEKKKPGETFFMCSCSSDECNDNIIFSEEYNTSNPDLLLVIFQVTGISLLPPLGVAISVIIIFYCYRVNRQQKLSSGSGATNFSLLKQAGDVEENPGPMALPVTALLLPLALLLHAARPQVQLVESGGGVVQPGGSLRLSCAASFSGYGVSTMAWFRQAPGKGLEGVAAITVGSGNTYYADSVKGRFTISRDNSKNTVYLQMNSLRAEDTAMYYCAVGYLSGGSWDVPGRYNYWGQGTLVTVSSGGGGSGGGGSGGGGSEVQLVESGGGLVQPGGSLRLSCAASGNTYSSNYMGWFRQAPGKGLEEVAVIYTRGGHTYYVDSVRGRFTISQDNAKNSLYLQMNSLRAEDTAVYYCAASSRHRLGLNNPRDYDYWGQGTLVTVSSTTTPAPRPPTPAPTIASQPLSLRPEACRPAAGGAVHTRGLDFACDIYIWAPLAGTCGVLLLSLVITLYCKRGRKKLLYIFKQPFMRPVQTTQEEDGCSCRFPEEEEGGCELRVKFSRSADAPAYKQGQNQLYNELNLGRREEYDVLDKRRGRDPEMGGKPRRKNPQEGLYNELQKDKMAEAYSEIGMKGERRRGKGHDGLYQGLSTATKDTYDALHMQALPPR

SEQ ID NO: 527 - protein, 729 aa, synthetic construct
  REGION 1..729: note = T3-T2A-TGF- -DNR amino acid sequence
MALPVTALLLPLALLLHAARPQVQLVESGGGVVQPGGSLRLSCAASFSGYGVSTMAWFRQAPGKGLEGVAAITVGSGNTYYADSVKGRFTISRDNSKNTVYLQMNSLRAEDTAMYYCAVGYLSGGSWDVPGRYNYWGQGTLVTVSSGGGGSGGGGSGGGGSEVQLVESGGGLVQPGGSLRLSCAASGNTYSSNYMGWFRQAPGKGLEEVAVIYTRGGHTYYVDSVRGRFTISQDNAKNSLYLQMNSLRAEDTAVYYCAASSRHRLGLNNPRDYDYWGQGTLVTVSSTTTPAPRPPTPAPTIASQPLSLRPEACRPAAGGAVHTRGLDFACDIYIWAPLAGTCGVLLLSLVITLYCKRGRKKLLYIFKQPFMRPVQTTQEEDGCSCRFPEEEEGGCELRVKFSRSADAPAYKQGQNQLYNELNLGRREEYDVLDKRRGRDPEMGGKPRRKNPQEGLYNELQKDKMAEAYSEIGMKGERRRGKGHDGLYQGLSTATKDTYDALHMQALPPRGSGEGRGSLLTCGDVEENPGPMGRGLLRGLWPLHIVLWTRIASTIPPHVQKSVNNDMIVTDNNGAVKFPQLCKFCDVRFSTCDNQKSCMSNCSITSICEKPQEVCVAVWRKNDENITLETVCHDPKLPYHDFILEDAASPKCIMKEKKKPGETFFMCSCSSDECNDNIIFSEEYNTSNPDLLLVIFQVTGISLLPPLGVAISVIIIFYCYRVNRQQKLSS

SEQ ID NO: 528 - protein, 729 aa, synthetic construct
  REGION 1..729: note = TGF- -DNR-T2A-T3 amino acid sequence
MGRGLLRGLWPLHIVLWTRIASTIPPHVQKSVNNDMIVTDNNGAVKFPQLCKFCDVRFSTCDNQKSCMSNCSITSICEKPQEVCVAVWRKNDENITLETVCHDPKLPYHDFILEDAASPKCIMKEKKKPGETFFMCSCSSDECNDNIIFSEEYNTSNPDLLLVIFQVTGISLLPPLGVAISVIIIFYCYRVNRQQKLSSGSGEGRGSLLTCGDVEENPGPMALPVTALLLPLALLLHAARPQVQLVESGGGVVQPGGSLRLSCAASFSGYGVSTMAWFRQAPGKGLEGVAAITVGSGNTYYADSVKGRFTISRDNSKNTVYLQMNSLRAEDTAMYYCAVGYLSGGSWDVPGRYNYWGQGTLVTVSSGGGGSGGGGSGGGGSEVQLVESGGGLVQPGGSLRLSCAASGNTYSSNYMGWFRQAPGKGLEEVAVIYTRGGHTYYVDSVRGRFTISQDNAKNSLYLQMNSLRAEDTAVYYCAASSRHRLGLNNPRDYDYWGQGTLVTVSSTTTPAPRPPTPAPTIASQPLSLRPEACRPAAGGAVHTRGLDFACDIYIWAPLAGTCGVLLLSLVITLYCKRGRKKLLYIFKQPFMRPVQTTQEEDGCSCRFPEEEEGGCELRVKFSRSADAPAYKQGQNQLYNELNLGRREEYDVLDKRRGRDPEMGGKPRRKNPQEGLYNELQKDKMAEAYSEIGMKGERRRGKGHDGLYQGLSTATKDTYDALHMQALPPR

SEQ ID NO: 529 - protein, 199 aa, synthetic construct
  REGION 1..199: note = TGF- -DNR amino acid sequence
MGRGLLRGLWPLHIVLWTRIASTIPPHVQKSVNNDMIVTDNNGAVKFPQLCKFCDVRFSTCDNQKSCMSNCSITSICEKPQEVCVAVWRKNDENITLETVCHDPKLPYHDFILEDAASPKCIMKEKKKPGETFFMCSCSSDECNDNIIFSEEYNTSNPDLLLVIFQVTGISLLPPLGVAISVIIIFYCYRVNRQQKLSS